European Patent Specification EP 3 728 291 B1, published June 24, 2026. Title: EPSTEIN-BARR VIRUS ANTIGEN CONSTRUCTS. Applicant: GSK BIOLOGICALS S.A. The sequence listing filed with the application follows.

SEQUENCE LISTING (54 sequences)

SEQ ID NO: 1 - protein, 386 aa, Human herpesvirus 4
MEHDLERGPPGPRRPPRGPPLSSSLGLALLLLLLALLFWLYIVMSDWTGGALLVLYSFALMLIIIILIIFIFRRDLLCPLGALCILLLMITLLLIALWNLHGQALFLGIVLFIFGCLLVLGIWIYLLEMLWRLGATIWQLLAFFLAFFLDLILLIIALYLQQNWWTLLVDLLWLLLFLAILIWMYYHGQRHSDEHHHDDSLPHPQQATDDSGHESDSNSNEGRHHLLVSGAGDGPPLCSQNLGAPGGGPDNGPQDPDNTDDNGPQDPDNTDDNGPHDPLPQDPDNTDDNGPQDPDNTDDNGPHDPLPHSPSDSAGNDGGPPQLTEEVENKGGDQGPPLMTDGGGGHSHDSGHGGGDPHLPTLLLGSSGSGGDDDDPHGPVQLSYYD

SEQ ID NO: 2 - protein, 62 aa, Human herpesvirus 4
MSDWTGGALLVLYSFALMLIIIILIIFIFRRDLLCPLGALCILLLMITLLLIALWNLHGQAL

SEQ ID NO: 3 - protein, 85 aa, Human herpesvirus 4
FLGIVLFIFGCLLVLGIWIYLLEMLWRLGATIWQLLAFFLAFFLDLILLIIALYLQQNWWTLLVDLLWLLLFLAILIWMYYHGQR

SEQ ID NO: 4 - protein, 40 aa, Human herpesvirus 4
HSDEHHHDDSLPHPQQATDDSGHESDSNSNEGRHHLLVSG

SEQ ID NO: 5 - protein, 114 aa, Human herpesvirus 4
NGPHDPLPQDPDNTDDNGPQDPDNTDDNGPHDPLPHSPSDSAGNDGGPPQLTEEVENKGGDQGPPLMTDGGGGHSHDSGHGGGDPHLPTLLLGSSGSGGDDDDPHGPVQLSYYD

SEQ ID NO: 6 - protein, 497 aa, Human herpesvirus 4
MGSLEMVPMGAGPPSPGGDPDGYDGGNNSQYPSASGSSGNTPTPPNDEERESNEEPPPPYEDPYWGNGDRHSDYQPLGTQDQSLYLGLQHDGNDGLPPPPYSPRDDSSQHIYEEAGRGSMNPVCLPVIVAPYLFWLAAIAASCFTASVSTVVTATGLALSLLLLAAVASSYAAAQRKLLTPVTVLTAVVTFFAICLTWRIEDPPFNSLLFALLAAAGGLQGIYVLVMLVLLILAYRRRWRRLTVCGGIMFLACVLVLIVDAVLQLSPLLGAVTVVSMTLLLLAFVLWLSSPGGLGTLGAALLTLAAALALLASLILGTLNLTTMFLLMLLWTLVVLLICSSCSSCPLSKILLARLFLYALALLLLASALIAGGSILQTNFKSLSSTEFIPNLFCMLLLIVAGILFILAILTEWGSGNRTYGPVFMCLGGLLTMVAGAVWLTVMSNTLLSAWILTAGFLIFLIGFALFGVIRCCRYCCYYCLTLESEERPPTPYRNTV

SEQ ID NO: 7 - protein, 71 aa, Human herpesvirus 4
MNPVCLPVIVAPYLFWLAAIAASCFTASVSTVVTATGLALSLLLLAAVASSYAAAQRKLLTPVTVLTAVVT

SEQ ID NO: 8 - protein, 94 aa, Human herpesvirus 4
FFAICLTWRIEDPPFNSLLFALLAAAGGLQGIYVLVMLVLLILAYRRRWRRLTVCGGIMFLACVLVLIVDAVLQLSPLLGAVTVVSMTLLLLAF

SEQ ID NO: 9 - protein, 115 aa, Human herpesvirus 4
VLWLSSPGGLGTLGAALLTLAAALALLASLILGTLNLTTMFLLMLLWTLVVLLICSSCSSCPLSKILLARLFLYALALLLLASALIAGGSILQTNFKSLSSTEFIPNLFCMLLLI

SEQ ID NO: 10 - protein, 98 aa, Human herpesvirus 4
VAGILFILAILTEWGSGNRTYGPVFMCLGGLLTMVAGAVWLTVMSNTLLSAWILTAGFLIFLIGFALFGVIRCCRYCCYYCLTLESEERPPTPYRNTV

SEQ ID NO: 11 - protein, 641 aa, Human herpesvirus 4
MSDEGPGTGPGNGLGEKGDTSGPEGSGGSGPQRRGGDNHGRGRGRGRGRGGGRPGAPGGSGSGPRHRDGVRRPQKRPSCIGCKGTHGGTGAGAGAGGAGAGGAGAGGGAGAGGGAGGAGGAGGAGAGGGAGAGGGAGGAGGAGAGGGAGAGGGAGGAGAGGGAGGAGGAGAGGGAGAGGGAGGAGAGGGAGGAGGAGAGGGAGAGGAGGAGGAGAGGAGAGGGAGGAGGAGAGGAGAGGAGAGGAGAGGAGGAGAGGAGGAGAGGAGGAGAGGGAGGAGAGGGAGGAGAGGAGGAGAGGAGGAGAGGAGGAGAGGGAGAGGAGAGGGGRGRGGSGGRGRGGSGGRGRGGSGGRRGRGRERARGGSRERARGRGRGRGEKRPRSPSSQSSSSGSPPRRPPPGRRPFFHPVGEADYFEYHQEGGPDGEPDVPPGAIEQGPADDPGEGPSTGPRGQGDGGRRKKGGWFGKHRGQGGSNPKFENIAEGLRALLARSHVERTTDEGTWVAGVFVYGGSKTSLYNLRRGTALAIPQCRLTPLSRLPFGMAPGPGPQPGPLRESIVCYFMVFLQTHIFAEVLKDAIKDLVMTKPAPTCNIRVTVCSFDDGVDLPPWFPPMVEGAAAEGDDGDDGDEGGDGDEGEEGQE

SEQ ID NO: 12 - protein, 86 aa, Human herpesvirus 4
MSDEGPGTGPGNGLGEKGDTSGPEGSGGSGPQRRGGDNHGRGRGRGRGRGGGRPGAPGGSGSGPRHRDGVRRPQKRPSCIGCKGTH

SEQ ID NO: 13 - protein, 944 aa, Human herpesvirus 4
MDKDRPGPPALDDNMEEEVPSTSVVQEQVSAGDWENVLIELSDSSSEKEAEDAHLEPAQKGTKRKRVDHDAGGSAPARPMLPPQPDLPGREAILRRFPLDLRTLLQAIGAAATRIDTRAIDQFFGSQISNTEMYIMYAMAIRQAIRDRRRNPASRRDQAKWRLQTLAAGWPMGYQAYSSWMYSYTDHQTTPTFVHLQATLGCTGGRRCHVTFSAGTFKLPRCTPGDRQWLYVQSSVGNIVQSCNPRYSIFFDYMAIHRSLTKIWEEVLTPDQRVSFMEFLGFLQRTDLSYIKSFVSDALGTTSIQTPWIDDNPSTETAQAWNAGFLRGRAYGIDLLRTEGEHVEGATGETREESEDTESDGDDEDLPCIVSRGGPKVKRPPIFIRRLHRLLLMRAGKRTEQGKEVLEKARGSTYGTPRPPVPKPRPEVPQSDETATSHGSAQVPEPPTIHLAAQGMAYPLHEQHGMAPCPVAQAPPTPLPPVSPGDQLPGVFSDGRVACAPVPAPAGPIVRPWEPSLTQAAGQAFAPVRPQHMPVEPVPVPTVALERPVYPKPVRPAPPKIAMQGPGETSGIRRARERWRPAPWTPNPPRSPSQMSVRDRLARLRAEAQVKQASVEVQPPQLTQVSPQQPMEGPLVPEQQMFPGAPFSQVADVVRAPGVPAMQPQYFDLPLIQPISQGAPVAPLRASMGPVPPVPATQPQYFDIPLTEPINQGASAAHFLPQQPMEGPLVPEQWMFPGAALSQSVRPGVAQSQYFDLPLTQPINHGAPAAHFLHQPPMEGPWVPEQWMFQGAPPSQGTDVVQHQLDALGYTLHGLNHPGVPVSPAVNQYHLSQAAFGLPIDEDESGEGSDTSEPCEALDLSIHGRPCPQAPEWPVQEEGGQDATEVLDLSIHGRPRPRTPEWPVQGEGGQNVTGPETRRVVVSAVVHMCQDDEFPDLQDPPDEA

SEQ ID NO: 14 - protein, 66 aa, Human herpesvirus 4
IRDRRRNPASRRDQAKWRLQTLAAGWPMGYQAYSSWMYSYTDHQTTPTFVHLQATLGCTGGRRCHV

SEQ ID NO: 15 - protein, 55 aa, Human herpesvirus 4
TFSAGTFKLPRCTPGDRQWLYVQSSVGNIVQSCNPRYSIFFDYMAIHRSLTKIWE

SEQ ID NO: 16 - protein, 88 aa, Human herpesvirus 4
WIDDNPSTETAQAWNAGFLRGRAYGIDLLRTEGEHVEGATGETREESEDTESDGDDEDLPCIVSRGGPKVKRPPIFIRRLHRLLLMRA

SEQ ID NO: 17 - protein, 25 aa, Human herpesvirus 4
GKRTEQGKEVLEKARGSTYGTPRPP

SEQ ID NO: 18 - protein, 40 aa, Human herpesvirus 4
AQVPEPPTIHLAAQGMAYPLHEQHGMAPCPVAQAPPTPLP

SEQ ID NO: 19 - protein, 62 aa, Human herpesvirus 4
GRVACAPVPAPAGPIVRPWEPSLTQAAGQAFAPVRPQHMPVEPVPVPTVALERPVYPKPVRP

SEQ ID NO: 20 - protein, 51 aa, Human herpesvirus 4
RPAPWTPNPPRSPSQMSVRDRLARLRAEAQVKQASVEVQPPQLTQVSPQQP

SEQ ID NO: 21 - protein, 245 aa, Human herpesvirus 4
MMDPNSTSEDVKFTPDPYQVPFVQAFDQATRVYQDLGGPSQAPLPCVLWPVLPEPLPQGQLTAYHVSTAPTGSWFSAPQPAPENAYQAYAAPQLFPVSDITQNQQTNQAGGEAPQPGDNSTVQTAAAVVFACPGANQGQQLADIGVPQPAPVAAPARRTRKPQQPESLEECDSELEIKRYKNRVASRKCRAKFKQLLQHYREVAAAKSSENDRLRLLLKQMCPSLDVDSIIPRTPDVLHEDLLNF

SEQ ID NO: 22 - protein, 66 aa, Human herpesvirus 4
DLGGPSQAPLPCVLWPVLPEPLPQGQLTAYHVSTAPTGSWFSAPQPAPENAYQAYAAPQLFPVSDI

SEQ ID NO: 23 - protein, 51 aa, Human herpesvirus 4
RKPQQPESLEECDSELEIKRYKNRVASRKCRAKFKQLLQHYREVAAAKSSE

SEQ ID NO: 24 - protein, 1153 aa, Artificial Sequence
  source: /note="Description of Artificial Sequence: Synthetic polypeptide"
MRPAPWTPNPPRSPSQMSVRDRLARLRAEAQVKQASVEVQPPQLTQVSPQQPVAGILFILAILTEWGSGNRTYGPVFMCLGGLLTMVAGAVWLTVMSNTLLSAWILTAGFLIFLIGFALFGVIRCCRYCCYYCLTLESEERPPTPYRNTVIRDRRRNPASRRDQAKWRLQTLAAGWPMGYQAYSSWMYSYTDHQTTPTFVHLQATLGCTGGRRCHVFLGIVLFIFGCLLVLGIWIYLLEMLWRLGATIWQLLAFFLAFFLDLILLIIALYLQQNWWTLLVDLLWLLLFLAILIWMYYHGQRGRVACAPVPAPAGPIVRPWEPSLTQAAGQAFAPVRPQHMPVEPVPVPTVALERPVYPKPVRPVLWLSSPGGLGTLGAALLTLAAALALLASLILGTLNLTTMFLLMLLWTLVVLLICSSCSSCPLSKILLARLFLYALALLLLASALIAGGSILQTNFKSLSSTEFIPNLFCMLLLIHSDEHHHDDSLPHPQQATDDSGHESDSNSNEGRHHLLVSGAQVPEPPTIHLAAQGMAYPLHEQHGMAPCPVAQAPPTPLPFFAICLTWRIEDPPFNSLLFALLAAAGGLQGIYVLVMLVLLILAYRRRWRRLTVCGGIMFLACVLVLIVDAVLQLSPLLGAVTVVSMTLLLLAFNGPHDPLPQDPDNTDDNGPQDPDNTDDNGPHDPLPHSPSDSAGNDGGPPQLTEEVENKGGDQGPPLMTDGGGGHSHDSGHGGGDPHLPTLLLGSSGSGGDDDDPHGPVQLSYYDGKRTEQGKEVLEKARGSTYGTPRPPMSDWTGGALLVLYSFALMLIIIILIIFIFRRDLLCPLGALCILLLMITLLLIALWNLHGQALMSDEGPGTGPGNGLGEKGDTSGPEGSGGSGPQRRGGDNHGRGRGRGRGRGGGRPGAPGGSGSGPRHRDGVRRPQKRPSCIGCKGTHWIDDNPSTETAQAWNAGFLRGRAYGIDLLRTEGEHVEGATGETREESEDTESDGDDEDLPCIVSRGGPKVKRPPIFIRRLHRLLLMRAMNPVCLPVIVAPYLFWLAAIAASCFTASVSTVVTATGLALSLLLLAAVASSYAAAQRKLLTPVTVLTAVVTTFSAGTFKLPRCTPGDRQWLYVQSSVGNIVQSCNPRYSIFFDYMAIHRSLTKIWE

SEQ ID NO: 25 - DNA, 3459 bp, Artificial Sequence
  source: /note="Description of Artificial Sequence: Synthetic polynucleotide"
atgagacctgctccctggacacctaatcctcccaggtcccccagccagatgagcgtgagagacagactggctaggctgagagccgaggctcaggtcaagcaggccagcgtcgaggtgcaaccccctcagctcacccaggtgtccccccagcagcctgtggccggcattctgttcattctggccattctgaccgagtggggaagcggcaacagaacctacggccctgtcttcatgtgcctcggaggactgctgacaatggtggctggcgccgtgtggctcaccgtcatgtccaacaccctgctcagcgcctggattctgaccgccggattcctgatctttctgatcggattcgctctctttggcgtcatcaggtgttgcaggtactgttgctactactgcctgaccctcgagagcgaggaaagaccccccaccccctacaggaatacagtgattagggacagaaggaggaatcctgcctccaggagagaccaggccaaatggagactccaaacactcgccgctggatggcccatgggctaccaggcctatagctcctggatgtacagctacaccgaccatcagacaacacccaccttcgtgcatctgcaggctacactgggctgcaccggaggcagaaggtgtcacgtgtttctgggaatcgtgctgttcatctttggatgcctgctcgtgctgggcatctggatttatctcctggagatgctctggagactcggcgctacaatttggcagctgctcgccttttttctggccttctttctggacctgatcctcctgatcatcgccctgtacctccaacagaactggtggaccctcctggtggatctgctgtggctcctcctcttcctggccatcctgatctggatgtactaccatggccagagaggaagggtcgcttgcgctcctgtccctgctcctgctggccccatcgtgaggccttgggagccttccctcacacaggccgccggccaggcctttgctcccgtgaggccccagcacatgcctgtggaacccgtgcccgtccccacagtggctctggaaaggcctgtgtaccccaagcccgtgagacctgtcctctggctcagcagccctggaggactcggaacactcggagccgctctcctgacactggccgctgctctggctctgctggctagcctgatcctgggaaccctcaacctcaccaccatgtttctcctcatgctcctgtggaccctcgtggtgctgctcatctgttccagctgctccagctgccccctgagcaagatcctgctggccaggctgttcctgtacgccctcgccctcctgctgctggctagcgccctgatcgctggcggaagcatcctccagaccaatttcaagagcctctcctccaccgagttcatccccaacctgttctgtatgttactgctgatccatagcgacgagcaccatcatgacgactccctgccccatcctcagcaggccacagacgactccggccacgagagcgacagcaatagcaatgagggcaggcaccatctgctcgtgtccggagctcaagtccccgagcctcccaccatccatctcgccgcccagggaatggcttaccccctccacgagcagcacggcatggccccttgtcccgtcgctcaagccccccctacacctctgccctttttcgccatttgtctgacctggagaatcgaggacccccccttcaacagcctgctgttcgccctgctcgccgccgctggcggcctccagggcatttacgtcctcgtgatgctggtgctgctgatcctcgcttacaggagaagatggaggagactgacagtgtgcggcggcatcatgtttctcgcctgcgtcctggtcctgatcgtggacgccgtcctgcaactcagccccctcctgggagctgtgacagtggtctccatgaccctgctgctgctggccttcaacggaccccacgatcctctgccccaagatcctgacaataccgacgataacggcccccaagaccccgataacaccgacgacaatggccctcacgaccctctgccccatagcccttccgatagcgctggcaacgatggcggccctcctcagctgacagaggaggtggaaaataagggcggcgatcagggaccccccctgatgacagatggcggaggaggacacagccatgatagcggacatggcggaggcgatccccatctgcctaccctcctcctgggcagctccggttctggaggcgacgatgatgaccctcacggccctgtgcagctctcctactacgacggcaaaaggaccgaacaaggaaaagaggtcctggagaaggccaggggcagcacatacggaacccccaggcctcccatgtccgattggaccggaggagccctgctggtcctctacagcttcgccctgatgctgatcattatcatcctgatcatctttatcttcagaagggacctgctgtgccctctcggcgccctgtgcatcctgctgctcatgatcacactcctcctgatcgccctctggaacctgcacggacaagccctgatgtccgatgagggacctggaacaggacccggaaacggactgggcgagaagggagatacaagcggccccgaaggcagcggcggaagcggaccccaaagaaggggcggcgacaaccacggaagaggaagaggcaggggcagaggcagaggaggaggaagacctggagcccctggcggttctggaagcggacccaggcacagggacggagtgaggaggcctcaaaaaagacccagctgcatcggctgcaagggaacccactggattgatgataacccctccacagagaccgctcaggcctggaacgccggcttcctgaggggaagagcctatggcatcgatctgctgaggaccgagggcgaacacgtggagggagccaccggagagacaagggaggaaagcgaagacacagaaagcgatggcgacgacgaagacctgccctgcattgtgtccaggggcggacccaaggtgaagaggccccctatctttatcagaaggctccatagactgctcctgatgagggccatgaaccctgtgtgcctgcccgtgatcgtggccccctacctcttttggctggccgccattgccgctagctgcttcaccgcctccgtgtccacagtggtgacagccaccggcctcgccctgagcctgctgctcctcgctgccgtggcctccagctacgccgctgctcaaagaaagctcctgacccctgtcaccgtcctgacagccgtcgtgaccaccttttccgctggcaccttcaagctgcctaggtgcacacctggcgacaggcagtggctctacgtgcagagctccgtgggcaatattgtgcagagctgcaatcccaggtacagcatttttttcgactacatggccatccataggtccctcaccaagatctgggag

SEQ ID NO: 26 - protein, 1270 aa, Artificial Sequence
  source: /note="Description of Artificial Sequence: Synthetic polypeptide"
MRPAPWTPNPPRSPSQMSVRDRLARLRAEAQVKQASVEVQPPQLTQVSPQQPVAGILFILAILTEWGSGNRTYGPVFMCLGGLLTMVAGAVWLTVMSNTLLSAWILTAGFLIFLIGFALFGVIRCCRYCCYYCLTLESEERPPTPYRNTVRKPQQPESLEECDSELEIKRYKNRVASRKCRAKFKQLLQHYREVAAAKSSEIRDRRRNPASRRDQAKWRLQTLAAGWPMGYQAYSSWMYSYTDHQTTPTFVHLQATLGCTGGRRCHVFLGIVLFIFGCLLVLGIWIYLLEMLWRLGATIWQLLAFFLAFFLDLILLIIALYLQQNWWTLLVDLLWLLLFLAILIWMYYHGQRGRVACAPVPAPAGPIVRPWEPSLTQAAGQAFAPVRPQHMPVEPVPVPTVALERPVYPKPVRPVLWLSSPGGLGTLGAALLTLAAALALLASLILGTLNLTTMFLLMLLWTLVVLLICSSCSSCPLSKILLARLFLYALALLLLASALIAGGSILQTNFKSLSSTEFIPNLFCMLLLIHSDEHHHDDSLPHPQQATDDSGHESDSNSNEGRHHLLVSGAQVPEPPTIHLAAQGMAYPLHEQHGMAPCPVAQAPPTPLPFFAICLTWRIEDPPFNSLLFALLAAAGGLQGIYVLVMLVLLILAYRRRWRRLTVCGGIMFLACVLVLIVDAVLQLSPLLGAVTVVSMTLLLLAFNGPHDPLPQDPDNTDDNGPQDPDNTDDNGPHDPLPHSPSDSAGNDGGPPQLTEEVENKGGDQGPPLMTDGGGGHSHDSGHGGGDPHLPTLLLGSSGSGGDDDDPHGPVQLSYYDGKRTEQGKEVLEKARGSTYGTPRPPMSDWTGGALLVLYSFALMLIIIILIIFIFRRDLLCPLGALCILLLMITLLLIALWNLHGQALMSDEGPGTGPGNGLGEKGDTSGPEGSGGSGPQRRGGDNHGRGRGRGRGRGGGRPGAPGGSGSGPRHRDGVRRPQKRPSCIGCKGTHWIDDNPSTETAQAWNAGFLRGRAYGIDLLRTEGEHVEGATGETREESEDTESDGDDEDLPCIVSRGGPKVKRPPIFIRRLHRLLLMRAMNPVCLPVIVAPYLFWLAAIAASCFTASVSTVVTATGLALSLLLLAAVASSYAAAQRKLLTPVTVLTAVVTTFSAGTFKLPRCTPGDRQWLYVQSSVGNIVQSCNPRYSIFFDYMAIHRSLTKIWEDLGGPSQAPLPCVLWPVLPEPLPQGQLTAYHVSTAPTGSWFSAPQPAPENAYQAYAAPQLFPVSDI

SEQ ID NO: 27 - DNA, 3810 bp, Artificial Sequence
  source: /note="Description of Artificial Sequence: Synthetic polynucleotide"
atgagacctgctccctggacacctaatcctcccaggtcccccagccagatgagcgtgagagacagactggctaggctgagagccgaggctcaggtcaagcaggccagcgtcgaggtgcaaccccctcagctcacccaggtgtccccccagcagcctgtggccggcattctgttcattctggccattctgaccgagtggggaagcggcaacagaacctacggccctgtcttcatgtgcctcggaggactgctgacaatggtggctggcgccgtgtggctcaccgtcatgtccaacaccctgctcagcgcctggattctgaccgccggattcctgatctttctgatcggattcgctctctttggcgtcatcaggtgttgcaggtactgttgctactactgcctgaccctcgagagcgaggaaagaccccccaccccctacaggaatacagtgaggaaacctcagcagcccgagagcctcgaggagtgcgatagcgagctggagattaaaaggtataagaatagggtggcctccaggaagtgtagggctaaattcaaacagctcctgcaacactatagggaagtggccgccgccaagtccagcgagattagggacagaaggaggaatcctgcctccaggagagaccaggccaaatggagactccaaacactcgccgctggatggcccatgggctaccaggcctatagctcctggatgtacagctacaccgaccatcagacaacacccaccttcgtgcatctgcaggctacactgggctgcaccggaggcagaaggtgtcacgtgtttctgggaatcgtgctgttcatctttggatgcctgctcgtgctgggcatctggatttatctcctggagatgctctggagactcggcgctacaatttggcagctgctcgccttttttctggccttctttctggacctgatcctcctgatcatcgccctgtacctccaacagaactggtggaccctcctggtggatctgctgtggctcctcctcttcctggccatcctgatctggatgtactaccatggccagagaggaagggtcgcttgcgctcctgtccctgctcctgctggccccatcgtgaggccttgggagccttccctcacacaggccgccggccaggcctttgctcccgtgaggccccagcacatgcctgtggaacccgtgcccgtccccacagtggctctggaaaggcctgtgtaccccaagcccgtgagacctgtcctctggctcagcagccctggaggactcggaacactcggagccgctctcctgacactggccgctgctctggctctgctggctagcctgatcctgggaaccctcaacctcaccaccatgtttctcctcatgctcctgtggaccctcgtggtgctgctcatctgttccagctgctccagctgccccctgagcaagatcctgctggccaggctgttcctgtacgccctcgccctcctgctgctggctagcgccctgatcgctggcggaagcatcctccagaccaatttcaagagcctctcctccaccgagttcatccccaacctgttctgtatgttactgctgatccatagcgacgagcaccatcatgacgactccctgccccatcctcagcaggccacagacgactccggccacgagagcgacagcaatagcaatgagggcaggcaccatctgctcgtgtccggagctcaagtccccgagcctcccaccatccatctcgccgcccagggaatggcttaccccctccacgagcagcacggcatggccccttgtcccgtcgctcaagccccccctacacctctgccctttttcgccatttgtctgacctggagaatcgaggacccccccttcaacagcctgctgttcgccctgctcgccgccgctggcggcctccagggcatttacgtcctcgtgatgctggtgctgctgatcctcgcttacaggagaagatggaggagactgacagtgtgcggcggcatcatgtttctcgcctgcgtcctggtcctgatcgtggacgccgtcctgcaactcagccccctcctgggagctgtgacagtggtctccatgaccctgctgctgctggccttcaacggaccccacgatcctctgccccaagatcctgacaataccgacgataacggcccccaagaccccgataacaccgacgacaatggccctcacgaccctctgccccatagcccttccgatagcgctggcaacgatggcggccctcctcagctgacagaggaggtggaaaataagggcggcgatcagggaccccccctgatgacagatggcggaggaggacacagccatgatagcggacatggcggaggcgatccccatctgcctaccctcctcctgggcagctccggttctggaggcgacgatgatgaccctcacggccctgtgcagctctcctactacgacggcaaaaggaccgaacaaggaaaagaggtcctggagaaggccaggggcagcacatacggaacccccaggcctcccatgtccgattggaccggaggagccctgctggtcctctacagcttcgccctgatgctgatcattatcatcctgatcatctttatcttcagaagggacctgctgtgccctctcggcgccctgtgcatcctgctgctcatgatcacactcctcctgatcgccctctggaacctgcacggacaagccctgatgtccgatgagggacctggaacaggacccggaaacggactgggcgagaagggagatacaagcggccccgaaggcagcggcggaagcggaccccaaagaaggggcggcgacaaccacggaagaggaagaggcaggggcagaggcagaggaggaggaagacctggagcccctggcggttctggaagcggacccaggcacagggacggagtgaggaggcctcaaaaaagacccagctgcatcggctgcaagggaacccactggattgatgataacccctccacagagaccgctcaggcctggaacgccggcttcctgaggggaagagcctatggcatcgatctgctgaggaccgagggcgaacacgtggagggagccaccggagagacaagggaggaaagcgaagacacagaaagcgatggcgacgacgaagacctgccctgcattgtgtccaggggcggacccaaggtgaagaggccccctatctttatcagaaggctccatagactgctcctgatgagggccatgaaccctgtgtgcctgcccgtgatcgtggccccctacctcttttggctggccgccattgccgctagctgcttcaccgcctccgtgtccacagtggtgacagccaccggcctcgccctgagcctgctgctcctcgctgccgtggcctccagctacgccgctgctcaaagaaagctcctgacccctgtcaccgtcctgacagccgtcgtgaccaccttttccgctggcaccttcaagctgcctaggtgcacacctggcgacaggcagtggctctacgtgcagagctccgtgggcaatattgtgcagagctgcaatcccaggtacagcatttttttcgactacatggccatccataggtccctcaccaagatctgggaggatctgggaggcccttcccaggctcctctgccctgcgtgctgtggcctgtgctgcctgagcctctgccccaaggccagctgacagcctatcacgtgtccaccgctcctacaggttcttggttcagcgctccccagcccgctcccgaaaacgcttaccaggcttacgccgccccccagctgttccccgtctccgacatc

SEQ ID NO: 28 - protein, 355 aa, Callitrichine gammaherpesvirus 3
MAPRRRLSGPPWLTVLLLLSTLSVAALLILFLIFSAGATISTEASLLVLLLLFVTLLLPLLSSNGLQLPAALILIQCFLLAADYLAYLILPTISEDFLILIAILVIVILVGTITTLVGAIGGIRARRSFLFICIFFLFLSLFLTILALLLGFSWLLLVAILFWVLWLVILILLLLVYPIPHHPLPTSLRFRMKQRVSSDPTGSDRSPQGSHNSLNSPDEEDPKDDTKQPLCNMTQGGPPVNGQLLGQHAQCPPHYPCCHIQHPDGEDSDGDDGKSWGDAGEEDNGPNDPNTNNGNEGGEGDDYKSWRKPEEEDNGPNDPNTNNRIEDGDGDDGKSWRNPEEEDNRKQDRLGTKPF

SEQ ID NO: 29 - protein, 93 aa, Callitrichine gammaherpesvirus 3
MAPRRRLSGPPWLTVLLLLSTLSVAALLILFLIFSAGATISTEASLLVLLLLFVTLLLPLLSSNGLQLPAALILIQCFLLAADYLAYLILPTI

SEQ ID NO: 30 - protein, 198 aa, Callitrichine gammaherpesvirus 3
SEDFLILIAILVIVILVGTITTLVGAIGGIRARRSFLFICIFFLFLSLFLTILALLLGFSWLLLVAILFWVLWLVILILLLLVYPIPHHPLPTSLRFRMKQRVSSDPTGSDRSPQGSHNSLNSPDEEDPKDDTKQPLCNMTQGGPPVNGQLLGQHAQCPPHYPCCHIQHPDGEDSDGDDGKSWGDAGEEDNGPNDPNT

SEQ ID NO: 31 - protein, 64 aa, Callitrichine gammaherpesvirus 3
NNGNEGGEGDDYKSWRKPEEEDNGPNDPNTNNRIEDGDGDDGKSWRNPEEEDNRKQDRLGTKPF

SEQ ID NO: 32 - protein, 413 aa, Callitrichine gammaherpesvirus 3
MAGHWYESVIPGLFLCPLILPSLFWICSLLTFLVGHGANIVSAVLFLVLAWCLLIANWNVTREDFVSGRRSSMSSLSVAASTATAMFASFLTLSFDGLGLLLFGTALVIQTIYVLYLVVMEITVWIMMFRYLHFWITLLFLLSPIILSVACLIIQSSALLIEAVVVTTITVLAIFLWLPPQGAEADLGTALLILNTALCLVVLILTAIPTDAQILTVFCLFCQWTLFICLGIRMICNWRGKLTRIICLKFCLYGLISASLSFGWYAFLKEVTLPTTATVDPRQLPLFLFILSSVLVILAIMMEFQTSSSLFAALFVIIAGMLCVTVGVIFLLAGVKPLLSGMICASGITMLVLGVVLLVVCTRASTRESIYEDLRYPTRDANGEYENVGYPPRDGDAPHRLGEPVYDDVEQAT

SEQ ID NO: 33 - protein, 210 aa, Callitrichine gammaherpesvirus 3
MAGHWYESVIPGLFLCPLILPSLFWICSLLTFLVGHGANIVSAVLFLVLAWCLLIANWNVTREDFVSGRRSSMSSLSVAASTATAMFASFLTLSFDGLGLLLFGTALVIQTIYVLYLVVMEITVWIMMFRYLHFWITLLFLLSPIILSVACLIIQSSALLIEAVVVTTITVLAIFLWLPPQGAEADLGTALLILNTALCLVVLILTAIPT

SEQ ID NO: 34 - protein, 153 aa, Callitrichine gammaherpesvirus 3
DAQILTVFCLFCQWTLFICLGIRMICNWRGKLTRIICLKFCLYGLISASLSFGWYAFLKEVTLPTTATVDPRQLPLFLFILSSVLVILAIMMEFQTSSSLFAALFVIIAGMLCVTVGVIFLLAGVKPLLSGMICASGITMLVLGVVLLVVCTR

SEQ ID NO: 35 - protein, 50 aa, Callitrichine gammaherpesvirus 3
ASTRESIYEDLRYPTRDANGEYENVGYPPRDGDAPHRLGEPVYDDVEQAT

SEQ ID NO: 36 - protein, 327 aa, Callitrichine gammaherpesvirus 3
MPRGRSTGRKGRDTEKERSRSPLRAPGGSDGPSTRAGCGAGPCQLSSPIAGGSRGGRGGRGGRGGSRGRGASRGRGGRGGRGGRGGRGGRGGRGGRGSPGDDSPSPCHHRDEPPSRSPSPQPTVSEQSQQSPRQQSPQGTSQGSTRPQVPGGATTRKRGGVRGQPAKCHGKYTTTAEGLTALLNRRHSPRTSNEGRWMNGVMAVNLSKWPLYSLRRALALAANEVRISPLFRLPYGSAFGPGPQPGPILESSTWGFLVFTQTSLFADDIADAIRDYCTTHPGPTRNTQVVLMNFEGSGVPLPMFFPPGEETEEQREGDRASDSDESE

SEQ ID NO: 37 - protein, 51 aa, Callitrichine gammaherpesvirus 3
MPRGRSTGRKGRDTEKERSRSPLRAPGGSDGPSTRAGCGAGPCQLSSPIAG

SEQ ID NO: 38 - protein, 119 aa, Callitrichine gammaherpesvirus 3
SPSPCHHRDEPPSRSPSPQPTVSEQSQQSPRQQSPQGTSQGSTRPQVPGGATTRKRGGVRGQPAKCHGKYTTTAEGLTALLNRRHSPRTSNEGRWMNGVMAVNLSKWPLYSLRRALALA

SEQ ID NO: 39 - protein, 106 aa, Callitrichine gammaherpesvirus 3
ANEVRISPLFRLPYGSAFGPGPQPGPILESSTWGFLVFTQTSLFADDIADAIRDYCTTHPGPTRNTQVVLMNFEGSGVPLPMFFPPGEETEEQREGDRASDSDESE

SEQ ID NO: 40 - protein, 252 aa, Callitrichine gammaherpesvirus 3
MDLDGTGGGEGYSQMVPIATAPGSGHAATYQDLQAAPYIIWPLQTDCQPVATTFASPGQIQWYTSAVPQPTEHCSQFTNAPTVNQQQPISQPQPENPPAFTFTQPASIIPGVISASNLNVSASPIIPSDHVLPIITSVTSLAQPNNDEHAISASHHASDGSVNQQKENQPQTLEECKTDQERKRYRNRLASRRCRAKFRNQLEHFRTVAAAKTEENNRLRVLIRQMCPTLDVESIVPSTSAGYHEPLNHLTH

SEQ ID NO: 41 - protein, 146 aa, Callitrichine gammaherpesvirus 3
MDLDGTGGGEGYSQMVPIATAPGSGHAATYQDLQAAPYIIWPLQTDCQPVATTFASPGQIQWYTSAVPQPTEHCSQFTNAPTVNQQQPISQPQPENPPAFTFTQPASIIPGVISASNLNVSASPIIPSDHVLPIITSVTSLAQPNN

SEQ ID NO: 42 - protein, 106 aa, Callitrichine gammaherpesvirus 3
DEHAISASHHASDGSVNQQKENQPQTLEECKTDQERKRYRNRLASRRCRAKFRNQLEHFRTVAAAKTEENNRLRVLIRQMCPTLDVESIVPSTSAGYHEPLNHLTH

SEQ ID NO: 43 - protein, 216 aa, Callithrix jacchus
MDDQRDLISNNEQLPMLGQRPGAPESKCSRGAVYTVFSILVALLLAGQATTAYFLYQQQGRLDKLTVTSQNLQLENLRMKLPKPAKPLSQMRMATPLLMQALPMAGLPQKPMQNATKHGNMTEDHVMHLLLNADPLKVYPPLKGSLSENLKHLKNTMETMDWKVFESWLHHWLLFEMSKHSLEQKPTEAPPKESLELEDPSSGLGVTKQDLGPVAM

SEQ ID NO: 44 - protein, 1045 aa, Artificial Sequence
  source: /note="Description of Artificial Sequence: Synthetic polypeptide"
MSEDFLILIAILVIVILVGTITTLVGAIGGIRARRSFLFICIFFLFLSLFLTILALLLGFSWLLLVAILFWVLWLVILILLLLVYPIPHHPLPTSLRFRMKQRVSSDPTGSDRSPQGSHNSLNSPDEEDPKDDTKQPLCNMTQGGPPVNGQLLGQHAQCPPHYPCCHIQHPDGEDSDGDDGKSWGDAGEEDNGPNDPNTASTRESIYEDLRYPTRDANGEYENVGYPPRDGDAPHRLGEPVYDDVEQATANEVRISPLFRLPYGSAFGPGPQPGPILESSTWGFLVFTQTSLFADDIADAIRDYCTTHPGPTRNTQVVLMNFEGSGVPLPMFFPPGEETEEQREGDRASDSDESEDAQILTVFCLFCQWTLFICLGIRMICNWRGKLTRIICLKFCLYGLISASLSFGWYAFLKEVTLPTTATVDPRQLPLFLFILSSVLVILAIMMEFQTSSSLFAALFVIIAGMLCVTVGVIFLLAGVKPLLSGMICASGITMLVLGVVLLVVCTRSPSPCHHRDEPPSRSPSPQPTVSEQSQQSPRQQSPQGTSQGSTRPQVPGGATTRKRGGVRGQPAKCHGKYTTTAEGLTALLNRRHSPRTSNEGRWMNGVMAVNLSKWPLYSLRRALALAMAPRRRLSGPPWLTVLLLLSTLSVAALLILFLIFSAGATISTEASLLVLLLLFVTLLLPLLSSNGLQLPAALILIQCFLLAADYLAYLILPTIMPRGRSTGRKGRDTEKERSRSPLRAPGGSDGPSTRAGCGAGPCQLSSPIAGNNGNEGGEGDDYKSWRKPEEEDNGPNDPNTNNRIEDGDGDDGKSWRNPEEEDNRKQDRLGTKPFMAGHWYESVIPGLFLCPLILPSLFWICSLLTFLVGHGANIVSAVLFLVLAWCLLIANWNVTREDFVSGRRSSMSSLSVAASTATAMFASFLTLSFDGLGLLLFGTALVIQTIYVLYLVVMEITVWIMMFRYLHFWITLLFLLSPIILSVACLIIQSSALLIEAVVVTTITVLAIFLWLPPQGAEADLGTALLILNTALCLVVLILTAIPT

SEQ ID NO: 45 - DNA, 3135 bp, Artificial Sequence
  source: /note="Description of Artificial Sequence: Synthetic polynucleotide"
atgtccgaggactttctgattctgatcgccatcctggtgatcgtgattctcgtgggcacaatcacaaccctggtgggcgccatcggcggcattagggccaggaggagcttcctcttcatttgcatcttcttcctgttcctctccctcttcctgacaatcctcgccctgctgctgggcttcagctggctcctgctggtggccatcctgttctgggtgctctggctggtcatcctcattctgctgctgctggtgtaccctattcctcaccaccccctgcccacctccctcaggtttagaatgaagcagagggtgagcagcgaccccacaggttctgacagaagccctcagggcagccataatagcctgaactcccccgatgaggaggaccccaaggatgacaccaagcaacctctgtgcaacatgacccagggcggacctcccgtcaatggacagctcctcggacaacatgctcaatgcccccctcactatccctgctgccatattcagcatcccgacggagaggattccgatggagacgatggcaagtcctggggcgatgccggagaggaagacaatggccctaacgaccctaacaccgccagcaccagagagtccatttacgaggacctcagataccccacaagggacgccaatggcgagtatgagaacgtgggatacccccctagggacggagatgcccctcataggctcggagagcctgtgtatgacgatgtggagcaagccaccgctaacgaggtgagaatctcccctctgttcagactgccctacggaagcgctttcggacctggcccccagcctggacccattctggagagctccacatggggctttctggtcttcacacagacctccctgttcgccgacgacattgccgacgctattagggactactgcacaacccaccctggccccacaaggaacacccaggtggtcctcatgaacttcgagggcagcggagtgcccctgcctatgttttttccccctggagaggagacagaagagcagagagagggcgatagagctagcgactccgacgagtccgaagacgctcagatcctgaccgtgttctgcctgttttgccagtggacactctttatctgcctgggaatcaggatgatctgtaactggaggggcaaactcaccaggatcatctgcctgaagttctgcctctacggactgatttccgcctccctgtccttcggctggtacgcttttctgaaggaagtgaccctccccaccacagccaccgttgatcctaggcaactccccctgttcctcttcatcctgagctccgtgctggtgattctcgccatcatgatggagtttcaaacatcctccagcctcttcgctgctctgttcgtgattatcgccggaatgctgtgcgtcacagtgggcgtgatttttctgctggctggcgtcaagcctctcctgagcggcatgatctgcgcctccggcatcacaatgctcgtgctcggcgtcgtgctgctggtggtgtgcaccagaagccccagcccttgtcatcacagggatgaacccccctccagaagccccagccctcaacccaccgtctccgagcagtcccagcagtcccccaggcagcagagccctcaaggcacatcccagggttctacaagacctcaggtgcctggaggcgccaccaccagaaaaagaggcggcgtgagaggccaacctgccaagtgtcacggcaagtacaccacaaccgccgagggactgaccgctctcctgaataggaggcacagccccaggacatccaacgagggcaggtggatgaatggagtcatggctgtgaacctctccaaatggcccctgtacagcctgaggagagccctggccctcgccatggctcctagaaggaggctctccggccctccctggctgacagtgctgctgctgctgtccacactgagcgtggccgccctgctgattctcttcctgattttcagcgccggcgccaccattagcacagaagccagcctgctggtcctgctcctgctgtttgtgaccctgctgctgcctctcctgtcctccaacggactccagctccctgccgccctgattctgatccagtgtttcctcctggccgctgattatctcgcctacctgattctgcctaccattatgcccaggggcagaagcacaggaaggaagggcagggacacagagaaagagaggagcagatcccctctcagagctcctggcggttctgatggacccagcacaagggctggctgtggagccggaccctgtcagctgagcagccccatcgccggaaacaacggcaatgaaggcggcgagggcgacgactacaagagctggaggaagcccgaggaagaggacaacggccccaatgaccccaataccaacaacaggattgaggatggagacggcgacgacggaaaatcctggaggaatcctgaggaggaggataacagaaagcaggacaggctgggcaccaagcctttcatggccggccactggtatgagagcgtgattcccggcctgttcctctgccccctgatcctcccttccctgttctggatttgctccctgctgaccttcctggtgggccacggagccaatattgtgagcgccgtcctgttcctcgtgctggcttggtgtctcctcattgccaactggaacgtgacaagagaggacttcgtgtccggcaggagaagctccatgagcagcctgtccgtggccgcttccaccgccacagccatgttcgccagcttcctcaccctgagctttgatggcctgggcctgctgctgtttggcaccgccctggtgatccagacaatttacgtgctgtatctggtggtcatggagatcaccgtgtggatcatgatgtttaggtatctccacttttggatcaccctgctgttcctgctgagccccattattctctccgtcgcctgtctcatcatccaatcctccgccctgctgatcgaggctgtggtcgtcaccaccatcacagtcctggccatttttctgtggctccctcctcaaggcgctgaggccgatctcggcaccgccctgctgattctgaataccgccctgtgcctggtcgtgctgatcctgaccgctatccctaca

SEQ ID NO: 46 - protein, 1270 aa, Artificial Sequence; identical to SEQ ID NO: 26
  source: /note="Description of Artificial Sequence: Synthetic polypeptide"

SEQ ID NO: 47 - DNA, 3810 bp, Artificial Sequence; identical to SEQ ID NO: 27
  source: /note="Description of Artificial Sequence: Synthetic polynucleotide"

SEQ ID NO: 48 - protein, 1512 aa, Artificial Sequence
  source: /note="Description of Artificial Sequence: Synthetic polypeptide"
MDDQRDLISNNEQLPMLGQRPGAPESKCSRGAVYTVFSILVALLLAGQATTAYFLYQQQGRLDKLTVTSQNLQLENLRMKLPKPAKPLSQMRMATPLLMQALPMAGLPQKPMQNATKHGNMTEDHVMHLLLNADPLKVYPPLKGSLSENLKHLKNTMETMDWKVFESWLHHWLLFEMSKHSLEQKPTEAPPKESLELEDPSSGLGVTKQDLGPVAMSEDFLILIAILVIVILVGTITTLVGAIGGIRARRSFLFICIFFLFLSLFLTILALLLGFSWLLLVAILFWVLWLVILILLLLVYPIPHHPLPTSLRFRMKQRVSSDPTGSDRSPQGSHNSLNSPDEEDPKDDTKQPLCNMTQGGPPVNGQLLGQHAQCPPHYPCCHIQHPDGEDSDGDDGKSWGDAGEEDNGPNDPNTASTRESIYEDLRYPTRDANGEYENVGYPPRDGDAPHRLGEPVYDDVEQATANEVRISPLFRLPYGSAFGPGPQPGPILESSTWGFLVFTQTSLFADDIADAIRDYCTTHPGPTRNTQVVLMNFEGSGVPLPMFFPPGEETEEQREGDRASDSDESEDAQILTVFCLFCQWTLFICLGIRMICNWRGKLTRIICLKFCLYGLISASLSFGWYAFLKEVTLPTTATVDPRQLPLFLFILSSVLVILAIMMEFQTSSSLFAALFVIIAGMLCVTVGVIFLLAGVKPLLSGMICASGITMLVLGVVLLVVCTRDEHAISASHHASDGSVNQQKENQPQTLEECKTDQERKRYRNRLASRRCRAKFRNQLEHFRTVAAAKTEENNRLRVLIRQMCPTLDVESIVPSTSAGYHEPLNHLTHSPSPCHHRDEPPSRSPSPQPTVSEQSQQSPRQQSPQGTSQGSTRPQVPGGATTRKRGGVRGQPAKCHGKYTTTAEGLTALLNRRHSPRTSNEGRWMNGVMAVNLSKWPLYSLRRALALAMAPRRRLSGPPWLTVLLLLSTLSVAALLILFLIFSAGATISTEASLLVLLLLFVTLLLPLLSSNGLQLPAALILIQCFLLAADYLAYLILPTIMPRGRSTGRKGRDTEKERSRSPLRAPGGSDGPSTRAGCGAGPCQLSSPIAGNNGNEGGEGDDYKSWRKPEEEDNGPNDPNTNNRIEDGDGDDGKSWRNPEEEDNRKQDRLGTKPFMDLDGTGGGEGYSQMVPIATAPGSGHAATYQDLQAAPYIIWPLQTDCQPVATTFASPGQIQWYTSAVPQPTEHCSQFTNAPTVNQQQPISQPQPENPPAFTFTQPASIIPGVISASNLNVSASPIIPSDHVLPIITSVTSLAQPNNMAGHWYESVIPGLFLCPLILPSLFWICSLLTFLVGHGANIVSAVLFLVLAWCLLIANWNVTREDFVSGRRSSMSSLSVAASTATAMFASFLTLSFDGLGLLLFGTALVIQTIYVLYLVVMEITVWIMMFRYLHFWITLLFLLSPIILSVACLIIQSSALLIEAVVVTTITVLAIFLWLPPQGAEADLGTALLILNTALCLVVLILTAIPT

SEQ ID NO: 49 - DNA, 4536 bp, Artificial Sequence
  source: /note="Description of Artificial Sequence: Synthetic polynucleotide"
atggacgaccagcgggacctgatcagcaacaacgagcagctgcccatgctgggccagaggcctggcgcccctgagagcaagtgtagcagaggcgccgtgtacaccgtgttcagcatcctggtggccctgctgctggccggacaggccaccaccgcctactttctgtatcagcagcagggacggctggacaagctgaccgtgaccagccagaacctgcagctggaaaacctgcggatgaagctgcccaagcccgccaagcccctgagccagatgagaatggccacccccctgctgatgcaggccctgcctatggccggcctgccccagaaacccatgcagaacgccaccaagcacggcaacatgaccgaggaccacgtgatgcatctgctgctgaacgccgaccccctgaaggtgtaccccccactgaagggcagcctgagcgagaacctgaagcacctgaagaacaccatggaaaccatggactggaaggtgttcgagagctggctgcaccactggctgctgttcgagatgagcaagcacagcctggaacagaagcccaccgaggcccctcccaaagagagcctggaactggaagatcccagcagcggcctgggcgtgaccaagcaggatctgggccccgtggctatgtccgaggactttctgattctgatcgccatcctggtgatcgtgattctcgtgggcacaatcacaaccctggtgggcgccatcggcggcattagggccaggaggagcttcctcttcatttgcatcttcttcctgttcctctccctcttcctgacaatcctcgccctgctgctgggcttcagctggctcctgctggtggccatcctgttctgggtgctctggctggtcatcctcattctgctgctgctggtgtaccctattcctcaccaccccctgcccacctccctcaggtttagaatgaagcagagggtgagcagcgaccccacaggttctgacagaagccctcagggcagccataatagcctgaactcccccgatgaggaggaccccaaggatgacaccaagcaacctctgtgcaacatgacccagggcggacctcccgtcaatggacagctcctcggacaacatgctcaatgcccccctcactatccctgctgccatattcagcatcccgacggagaggattccgatggagacgatggcaagtcctggggcgatgccggagaggaagacaatggccctaacgaccctaacaccgccagcaccagagagtccatttacgaggacctcagataccccacaagggacgccaatggcgagtatgagaacgtgggatacccccctagggacggagatgcccctcataggctcggagagcctgtgtatgacgatgtggagcaagccaccgctaacgaggtgagaatctcccctctgttcagactgccctacggaagcgctttcggacctggcccccagcctggacccattctggagagctccacatggggctttctggtcttcacacagacctccctgttcgccgacgacattgccgacgctattagggactactgcacaacccaccctggccccacaaggaacacccaggtggtcctcatgaacttcgagggcagcggagtgcccctgcctatgttttttccccctggagaggagacagaagagcagagagagggcgatagagctagcgactccgacgagtccgaagacgctcagatcctgaccgtgttctgcctgttttgccagtggacactctttatctgcctgggaatcaggatgatctgtaactggaggggcaaactcaccaggatcatctgcctgaagttctgcctctacggactgatttccgcctccctgtccttcggctggtacgcttttctgaaggaagtgaccctccccaccacagccaccgttgatcctaggcaactccccctgttcctcttcatcctgagctccgtgctggtgattctcgccatcatgatggagtttcaaacatcctccagcctcttcgctgctctgttcgtgattatcgccggaatgctgtgcgtcacagtgggcgtgatttttctgctggctggcgtcaagcctctcctgagcggcatgatctgcgcctccggcatcacaatgctcgtgctcggcgtcgtgctgctggtggtgtgcaccagagatgagcacgctatttccgccagccaccatgctagcgatggctccgtgaatcagcagaaggaaaatcagccccagaccctggaggaatgcaagacagatcaggagaggaagaggtacaggaacaggctggcctccaggaggtgtagagctaagttcaggaaccagctggaacattttaggacagtcgccgctgctaagacagaggagaacaacaggctcagggtgctcatcaggcagatgtgtcctacactggacgtggaatccatcgtcccctccacctccgccggctaccacgagcctctgaatcacctgacccacagccccagcccttgtcatcacagggatgaacccccctccagaagccccagccctcaacccaccgtctccgagcagtcccagcagtcccccaggcagcagagccctcaaggcacatcccagggttctacaagacctcaggtgcctggaggcgccaccaccagaaaaagaggcggcgtgagaggccaacctgccaagtgtcacggcaagtacaccacaaccgccgagggactgaccgctctcctgaataggaggcacagccccaggacatccaacgagggcaggtggatgaatggagtcatggctgtgaacctctccaaatggcccctgtacagcctgaggagagccctggccctcgccatggctcctagaaggaggctctccggccctccctggctgacagtgctgctgctgctgtccacactgagcgtggccgccctgctgattctcttcctgattttcagcgccggcgccaccattagcacagaagccagcctgctggtcctgctcctgctgtttgtgaccctgctgctgcctctcctgtcctccaacggactccagctccctgccgccctgattctgatccagtgtttcctcctggccgctgattatctcgcctacctgattctgcctaccattatgcccaggggcagaagcacaggaaggaagggcagggacacagagaaagagaggagcagatcccctctcagagctcctggcggttctgatggacccagcacaagggctggctgtggagccggaccctgtcagctgagcagccccatcgccggaaacaacggcaatgaaggcggcgagggcgacgactacaagagctggaggaagcccgaggaagaggacaacggccccaatgaccccaataccaacaacaggattgaggatggagacggcgacgacggaaaatcctggaggaatcctgaggaggaggataacagaaagcaggacaggctgggcaccaagcctttcatggacctcgacggaaccggcggaggcgagggctacagccagatggtccctatcgccaccgcccccggaagcggccacgccgctacctatcaggatctccaggccgccccttacatcatctggcctctccagaccgattgccagcctgtggctaccaccttcgcctcccccggacagatccagtggtatacaagcgccgtcccccagcccacagagcattgctcccagtttacaaacgctcccaccgtcaaccagcagcagcctattagccaaccccagcccgaaaatccccctgctttcacctttacccagcccgcttccatcattcccggcgtcattagcgcctccaacctgaacgtgagcgcttcccctatcatccctagcgaccatgtcctccccatcattacctccgtgaccagcctcgcccaacctaataacatggccggccactggtatgagagcgtgattcccggcctgttcctctgccccctgatcctcccttccctgttctggatttgctccctgctgaccttcctggtgggccacggagccaatattgtgagcgccgtcctgttcctcgtgctggcttggtgtctcctcattgccaactggaacgtgacaagagaggacttcgtgtccggcaggagaagctccatgagcagcctgtccgtggccgcttccaccgccacagccatgttcgccagcttcctcaccctgagctttgatggcctgggcctgctgctgtttggcaccgccctggtgatccagacaatttacgtgctgtatctggtggtcatggagatcaccgtgtggatcatgatgtttaggtatctccacttttggatcaccctgctgttcctgctgagccccattattctctccgtcgcctgtctcatcatccaatcctccgccctgctgatcgaggctgtggtcgtcaccaccatcacagtcctggccatttttctgtggctccctcctcaaggcgctgaggccgatctcggcaccgccctgctgattctgaataccgccctgtgcctggtcgtgctgatcctgaccgctatccctaca

SEQ ID NO: 50 - DNA, 44035 bp, Artificial Sequence
  source: /note="Description of Artificial Sequence: Synthetic polynucleotide"
  modified_base (15712)..(15712): a, c, t, g, unknown or other
catcatcaataatataccttattttggattgaagccaatatgataatgagatgggcggcgcggggcggggcgcggggcgggaggcgggtttgggggcgggccggcgggcggggcggtgtggcggaagtggactttgtaagtgtggcggatgtgacttgctagtgccgggcgcggtaaaagtgacgttttccgtgcgcgacaacgcccccgggaagtgacatttttcccgcggtttttaccggatgttgtagtgaatttgggcgtaaccaagtaagatttggccattttcgcgggaaaactgaaacggggaagtgaaatctgattaattttgcgttagtcataccgcgtaatatttgtctagggccgagggactttggccgattacgtggaggactcgcccaggtgttttttgaggtgaatttccgcgttccgggtcaaagtctgcgttttattattataggatatcccattgcatacgttgtatccatatcataatatgtacatttatattggctcatgtccaacattaccgccatgttgacattgattattgactagttattaatagtaatcaattacggggtcattagttcatagcccatatatggagttccgcgttacataacttacggtaaatggcccgcctggctgaccgcccaacgacccccgcccattgacgtcaataatgacgtatgttcccatagtaacgccaatagggactttccattgacgtcaatgggtggagtatttacggtaaactgcccacttggcagtacatcaagtgtatcatatgccaagtacgccccctattgacgtcaatgacggtaaatggcccgcctggcattatgcccagtacatgaccttatgggactttcctacttggcagtacatctacgtattagtcatcgctattaccatggtgatgcggttttggcagtacatcaatgggcgtggatagcggtttgactcacggggatttccaagtctccaccccattgacgtcaatgggagtttgttttggcaccaaaatcaacgggactttccaaaatgtcgtaacaactccgccccattgacgcaaatgggcggtaggcgtgtacggtgggaggtctatataagcagagctctccctatcagtgatagagatctccctatcagtgatagagatcgtcgacgagctcgtttagtgaaccgtcagatcgcctggagacgccatccacgctgttttgacctccatagaagacaccgggaccgatccagcctccgcggccgggaacggtgcattggaacgcggattccccgtgccaagagtgagatcttccgtttatctaggtaccagatatcgccaccatgagacctgctccctggacacctaatcctcccaggtcccccagccagatgagcgtgagagacagactggctaggctgagagccgaggctcaggtcaagcaggccagcgtcgaggtgcaaccccctcagctcacccaggtgtccccccagcagcctgtggccggcattctgttcattctggccattctgaccgagtggggaagcggcaacagaacctacggccctgtcttcatgtgcctcggaggactgctgacaatggtggctggcgccgtgtggctcaccgtcatgtccaacaccctgctcagcgcctggattctgaccgccggattcctgatctttctgatcggattcgctctctttggcgtcatcaggtgttgcaggtactgttgctactactgcctgaccctcgagagcgaggaaagaccccccaccccctacaggaatacagtgattagggacagaaggaggaatcctgcctccaggagagaccaggccaaatggagactccaaacactcgccgctggatggcccatgggctaccaggcctatagctcctggatgtacagctacaccgaccatcagacaacacccaccttcgtgcatctgcaggctacactgggctgcaccggaggcagaaggtgtcacgtgtttctgggaatcgtgctgttcatctttggatgcctgctcgtgctgggcatctggatttatctcctggagatgctctggagactcggcgctacaatttggcagctgctcgccttttttctggccttctttctggacctgatcctcctgatcatcgccctgtacctccaacagaactggtggaccctcctggtggatctgctgtggctcctcctcttcctggccatcctgatctggatgtactaccatggccagagaggaagggtcgcttgcgctcctgtccctgctcctgctggccccatcgtgaggccttgggagccttccctcacacaggccgccggccaggcctttgctcccgtgaggccccagcacatgcctgtggaacccgtgcccgtccccacagtggctctggaaaggcctgtgtaccccaagcccgtgagacctgtcctctggctcagcagccctggaggactcggaacactcggagccgctctcctgacactggccgctgctctggctctgctggctagcctgatcctgggaaccctcaacctcaccaccatgtttctcctcatgctcctgtggaccctcgtggtgctgctcatctgttccagctgctccagctgccccctgagcaagatcctgctggccaggctgttcctgtacgccctcgccctcctgctgctggctagcgccctgatcgctggcggaagcatcctccagaccaatttcaagagcctctcctccaccgagttcatccccaacctgttctgtatgttactgctgatccatagcgacgagcaccatcatgacgactccctgccccatcctcagcaggccacagacgactccggccacgagagcgacagcaatagcaatgagggcaggcaccatctgctcgtgtccggagctcaagtccccgagcctcccaccatccatctcgccgcccagggaatggcttaccccctccacgagcagcacggcatggccccttgtcccgtcgctcaagccccccctacacctctgccctttttcgccatttgtctgacctggagaatcgaggacccccccttcaacagcctgctgttcgccctgctcgccgccgctggcggcctccagggcatttacgtcctcgtgatgctggtgctgctgatcctcgcttacaggagaagatggaggagactgacagtgtgcggcggcatcatgtttctcgcctgcgtcctggtcctgatcgtggacgccgtcctgcaactcagccccctcctgggagctgtgacagtggtctccatgaccctgctgctgctggccttcaacggaccccacgatcctctgccccaagatcctgacaataccgacgataacggcccccaagaccccgataacaccgacgacaatggccctcacgaccctctgccccatagcccttccgatagcgctggcaacgatggcggccctcctcagctgacagaggaggtggaaaataagggcggcgatcagggaccccccctgatgacagatggcggaggaggacacagccatgatagcggacatggcggaggcgatccccatctgcctaccctcctcctgggcagctccggttctggaggcgacgatgatgaccctcacggccctgtgcagctctcctactacgacggcaaaaggaccgaacaaggaaaagaggtcctggagaaggccaggggcagcacatacggaacccccaggcctcccatgtccgattggaccggaggagccctgctggtcctctacagcttcgccctgatgctgatcattatcatcctgatcatctttatcttcagaagggacctgctgtgccctctcggcgccctgtgcatcctgctgctcatgatcacactcctcctgatcgccctctggaacctgcacggacaagccctgatgtccgatgagggacctggaacaggacccggaaacggactgggcgagaagggagatacaagcggccccgaaggcagcggcggaagcggaccccaaagaaggggcggcgacaaccacggaagaggaagaggcaggggcagaggcagaggaggaggaagacctggagcccctggcggttctggaagcggacccaggcacagggacggagtgaggaggcctcaaaaaagacccagctgcatcggctgcaagggaacccactggattgatgataacccctccacagagaccgctcaggcctggaacgccggcttcctgaggggaagagcctatggcatcgatctgctgaggaccgagggcgaacacgtggagggagccaccggagagacaagggaggaaagcgaagacacagaaagcgatggcgacgacgaagacctgccctgcattgtgtccaggggcggacccaaggtgaagaggccccctatctttatcagaaggctccatagactgctcctgatgagggccatgaaccctgtgtgcctgcccgtgatcgtggccccctacctcttttggctggccgccattgccgctagctgcttcaccgcctccgtgtccacagtggtgacagccaccggcctcgccctgagcctgctgctcctcgctgccgtggcctccagctacgccgctgctcaaagaaagctcctgacccctgtcaccgtcctgacagccgtcgtgaccaccttttccgctggcaccttcaagctgcctaggtgcacacctggcgacaggcagtggctctacgtgcagagctccgtgggcaatattgtgcagagctgcaatcccaggtacagcatttttttcgactacatggccatccataggtccctcaccaagatctgggagtgatgatgagcggccgcgatctgctgtgccttctagttgccagccatctgttgtttgcccctcccccgtgccttccttgaccctggaaggtgccactcccactgtcctttcctaataaaatgaggaaattgcatcgcattgtctgagtaggtgtcattctattctggggggtggggtggggcaggacagcaagggggaggattgggaagacaatagcaggcatgctggggatgcggtgggctctatggccgatcagcgatcgctgaggtgggtgagtgggcgtggcctggggtggtcatgaaaatatataagttgggggtcttagggtctctttatttgtgttgcagagaccgccggagccatgagcgggagcagcagcagcagcagtagcagcagcgccttggatggcagcatcgtgagcccttatttgacgacgcggatgccccactgggccggggtgcgtcagaatgtgatgggctccagcatcgacggccgacccgtcctgcccgcaaattccgccacgctgacctatgcgaccgtcgcggggacgccgttggacgccaccgccgccgccgccgccaccgcagccgcctcggccgtgcgcagcctggccacggactttgcattcctgggaccactggcgacaggggctacttctcgggccgctgctgccgccgttcgcgatgacaagctgaccgccctgctggcgcagttggatgcgcttactcgggaactgggtgacctttctcagcaggtcatggccctgcgccagcaggtctcctccctgcaagctggcgggaatgcttctcccacaaatgccgtttaagataaataaaaccagactctgtttggattaaagaaaagtagcaagtgcattgctctctttatttcataattttccgcgcgcgataggccctagaccagcgttctcggtcgttgagggtgcggtgtatcttctccaggacgtggtagaggtggctctggacgttgagatacatgggcatgagcccgtcccgggggtggaggtagcaccactgcagagcttcatgctccggggtggtgttgtagatgatccagtcgtagcaggagcgctgggcatggtgcctaaaaatgtccttcagcagcaggccgatggccagggggaggcccttggtgtaagtgtttacaaaacggttaagttgggaagggtgcattcggggagagatgatgtgcatcttggactgtatttttagattggcgatgtttccgcccagatcccttctgggattcatgttgtgcaggaccaccagtacagtgtatccggtgcacttggggaatttgtcatgcagcttagagggaaaagcgtggaagaacttggagacgcctttgtggcctcccagattttccatgcattcgtccatgatgatggcaatgggcccgcgggaggcagcttgggcaaagatatttctggggtcgctgacgtcgtagttgtgttccagggtgaggtcgtcataggccatttttacaaagcgcgggcggagggtgcccgactgggggatgatggtcccctctggccctggggcgtagttgccctcgcagatctgcatttcccaggccttaatctcggaggggggaatcatatccacctgcggggcgatgaagaaaacggtttccggagccggggagattaactgggatgagagcaggtttctaagcagctgtgattttccacaaccggtgggcccataaataacacctataaccggttgcagctggtagtttagagagctgcagctgccgtcgtcccggaggaggggggccacctcgttgagcatgtccctgacgcgcatgttctccccgaccagatccgccagaaggcgctcgccgcccagggacagcagctcttgcaaggaagcaaagtttttcagcggcttgaggccgtccgccgtgggcatgtttttcagggtctggctcagcagctccaggcggtcccagagctcggtgacgtgctctacggcatctctatccagcatatctcctcgtttcgcgggttggggcgactttcgctgtagggcaccaagcggtggtcgtccagcggggccagagtcatgtccttccatgggcgcagggtcctcgtcagggtggtctgggtcacggtgaaggggtgcgctccgggctgagcgcttgccaaggtgcgcttgaggctggttctgctggtgctgaagcgctgccggtcttcgccctgcgcgtcggccaggtagcatttgaccatggtgtcatagtccagcccctccgcggcgtgtcccttggcgcgcagcttgcccttggaggtggcgccgcacgaggggcagagcaggctcttgagcgcgtagagcttgggggcgaggaagaccgattcgggggagtaggcgtccgcgccgcagaccccgcacacggtctcgcactccaccagccaggtgagctcggggcgcgccgggtcaaaaaccaggtttcccccatgctttttgatgcgtttcttacctcgggtctccatgaggtggtgtccccgctcggtgacgaagaggctgtccgtgtctccgtagaccgacttgaggggtcttttctccaggggggtccctcggtcttcctcgtagaggaactcggaccactctgagacgaaggcccgcgtccaggccaggacgaaggaggctatgtgggaggggtagcggtcgttgtccactagggggtccaccttctccaaggtgtgaagacacatgtcgccttcctcggcgtccaggaaggtgattggcttgtaggtgtaggccacgtgaccgggggttcctgacgggggggtataaaagggggtgggggcgcgctcgtcgtcactctcttccgcatcgctgtctgcgagggccagctgctggggtgagtattccctctcgaaggcgggcatgacctccgcgctgaggttgtcagtttccaaaaacgaggaggatttgatgttcacctgtcccgaggtgatacctttgagggtacccgcgtccatctggtcagaaaacacgatctttttattgtccagcttggtggcgaacgacccgtagagggcgttggagagcagcttggcgatggagcgcagggtctggttcttgtccctgtcggcgcgctccttggccgcgatgttgagctgcacgtactcgcgcgcgacgcagcgccactcggggaagacggtggtgcgctcgtcgggcaccaggcgcacgcgccagccgcggttgtgcagggtgaccaggtccacgctggtggcgacctcgccgcgcaggcgctcgttggtccagcagagacggccgcccttgcgcgagcagaaggggggcagggggtcgagctgggtctcgtccggggggtccgcgtccacggtgaaaaccccggggcgcaggcgcgcgtcgaagtagtctatcttgcaaccttgcatgtccagcgcctgctgccagtcgcgggcggcgagcgcgcgctcgtaggggttgagcggcgggccccagggcatggggtgggtgagtgcggaggcgtacatgccgcagatgtcatagacgtagaggggctcccgcaggaccccgatgtaggtggggtagcagcggccgccgcggatgctggcgcgcacgtagtcatacagctcgtgcgagggggcgaggaggtcggggcccaggttggtgcgggcggggcgctccgcgcggaagacgatctgcctgaagatggcatgcgagttggaagagatggtggggcgctggaagacgttgaagctggcgtcctgcaggccgacggcgtcgcgcacgaaggaggcgtaggagtcgcgcagcttgtgtaccagctcggcggtgacctgcacgtcgagcgcgcagtagtcgagggtctcgcggatgatgtcatatttagcctgccccttctttttccacagctcgcggttgaggacaaactcttcgcggtctttccagtactcttggatcgggaaaccgtccggttccgaacggtaagagcctagcatgtagaactggttgacggcctggtaggcgcagcagcccttctccacggggagggcgtaggcctgcgcggccttgcggagcgaggtgtgggtcagggcgaaggtgtccctgaccatgactttgaggtactggtgcttgaagtcggagtcgtcgcagccgccccgctcccagagcgagaagtcggtgcgcttcttggagcgggggttgggcagagcgaaggtgacatcgttgaagaggattttgcccgcgcggggcatgaagttgcgggtgatgcggaagggccccggcacttcagagcggttgttgatgacctgggcggcgagcacgatctcgtcgaagccgttgatgttgtggcccacgatgtagagttccaggaagcggggccggccctttacggtgggcagcttctttagctcttcgtaggtgagctcctcgggcgaggcgaggccgtgctcggccagggcccagtccgcgaggtgcgggttgtctctgaggaaggacttccagaggtcgcgggccaggagggtctgcaggcggtctctgaaggtcctgaactggcggcccacggccattttttcgggggtgatgcagtagaaggtgagggggtcttgctgccagcggtcccagtcgagctgcagggcgaggtcgcgcgcggcggtgaccaggcgctcgtcgcccccgaatttcatgaccagcatgaagggcacgagctgctttccgaaggcccccatccaagtgtaggtctctacatcgtaggtgacaaagaggcgctccgtgcgaggatgcgagccgatcgggaagaactggatctcccgccaccagttggaggagtggctgttgatgtggtggaagtagaagtcccgtcgccgggccgaacactcgtgctggcttttgtaaaagcgagcgcagtactggcagcgctgcacgggctgtacctcatgcacgagatgcacctttcgcccgcgcacgaggaagccgaggggaaatctgagccccccgcctggctcgcggcatggctggttctcttctactttggatgcgtgtccgtctccgtctggctcctcgaggggtgttacggtggagcggaccaccacgccgcgcgagccgcaggtccagatatcggcgcgcggcggtcggagtttgatgacgacatcgcgcagctgggagctgtccatggtctggagctcccgcggcggcggcaggtcagccgggagttcttgcaggttcacctcgcagagtcgggccagggcgcggggcaggtctaggtggtacctgatctctaggggcgtgttggtggcggcgtcgatggcttgcaggagcccgcagccccggggggcgacgacggtgccccgcggggtggtggtggtggtggcggtgcagctcagaagcggtgccgcgggcgggcccccggaggtagggggggctccggtcccgcgggcaggggcggcagcggcacgtcggcgtggagcgcgggcaggagttggtgctgtgcccggaggttgctggcgaaggcgacgacgcggcggttgatctcctggatctggcgcctctgcgtgaagacgacgggcccggtgagcttgaacctgaaagagagttcgacagaatcaatctcggtgtcattgaccgcggcctggcgcaggatctcctgcacgtctcccgagttgtcttggtaggcgatctcggccatgaactgctcgatctcttcctcctggaggtctccgcgtccggcgcgttccacggtggccgccaggtcgttggagatgcgccccatgagctgcgagaaggcgttgagtccgccctcgttccagactcggctgtagaccacgcccccctggtcatcgcgggcgcgcatgaccacctgcgcgaggttgagctccacgtgccgcgcgaagacggcgtagttgcgcagacgctggaagaggtagttgagggtggtggcggtgtgctcggccacgaagaagttcatgacccagcggcgcaacgtggattcgttgatgtcccccaaggcctccagccgttccatggcctcgtagaagtccacggcgaagttgaaaaactgggagttgcgcgccgacacggtcaactcctcctccagaagacggatgagctcggcgacggtgtcgcgcacctcgcgctcgaaggctatggggatctcttcctccgctagcatcaccacctcctcctcttcctcctcttctggcacttccatgatggcttcctcctcttcggggggtggcggcggcggcggtgggggagggggcgctctgcgccggcggcggcgcaccgggaggcggtccacgaagcgcgcgatcatctccccgcggcggcggcgcatggtctcggtgacggcgcggccgttctcccgggggcgcagttggaagacgccgccggacatctggtgctggggcgggtggccgtgaggcagcgagacggcgctgacgatgcatctcaacaattgctgcgtaggtacgccgccgagggacctgagggagtccatatccaccggatccgaaaacctttcgaggaaggcgtctaaccagtcgcagtcgcaaggtaggctgagcaccgtggcgggcggcggggggtggggggagtgtctggcggaggtgctgctgatgatgtaattgaagtaggcggacttgacacggcggatggtcgacaggagcaccatgtccttgggtccggcctgctggatgcggaggcggtcggctatgccccaggcttcgttctggcatcggcgcaggtccttgtagtagtcttgcatgagcctttccaccggcacctcttctccttcctcttctgcttcttccatgtctgcttcggccctggggcggcgccgcgcccccctgccccccatgcgcgtgaccccgaaccccctgagcggttggagcagggccaggtcggcgacgacgcgctcggccaggatggcctgctgcacctgcgtgagggtggtttggaagtcatccaagtccacgaagcggtggtaggcgcccgtgttgatggtgtaggtgcagttggccatgacggaccagttgacggtctggtggcccggttgcgacatctcggtgtacctgagtcgcgagtaggcgcgggagtcgaagacgtagtcgttgcaagtccgcaccaggtactggtagcccaccaggaagtgcggcggcggctggcggtagaggggccagcgcagggtggcgggggctccgggggccaggtcttccagcatgaggcggtggtaggcgtagatgtacctggacatccaggtgatacccgcggcggtggtggaggcgcgcgggaagtcgcgcacccggttccagatgttgcgcaggggcagaaagtgctccatggtaggcgtgctctgtccagtcagacgcgcgcagtcgttgatactctagaccagggaaaacgaaagccggtcagcgggcactcttccgtggtctggtgaatagatcgcaagggtatcatggcggagggcctcggttcgagccccgggtccgggccggacggtccgccatgatccacgcggttaccgcccgcgtgtcgaacccaggtgtgcgacgtcagacaacggtggagtgttccttttggcgtttttctggccgggcgccggcgccgcgtaagagactaagccgcgaaagcgaaagcagtaagtggctcgctccccgtagccggagggatccttgctaagggttgcgttgcggcgaaccccggttcgaatcccgtactcgggccggccggacccgcggctaaggtgttggattggcctccccctcgtataaagaccccgcttgcggattgactccggacacggggacgagccccttttatttttgctttccccagatgcatccggtgctgcggcagatgcgccccccgccccagcagcagcaacaacaccagcaagagcggcagcaacagcagcgggagtcatgcagggccccctcacccaccctcggcgggccggccacctcggcgtccgcggccgtgtctggcgcctgcggcggcggcggggggccggctgacgaccccgaggagcccccgcggcgcagggccagacactacctggacctggaggagggcgagggcctggcgcggctgggggcgccgtctcccgagcgccacccgcgggtgcagctgaagcgcgactcgcgcgaggcgtacgtgcctcggcagaacctgttcagggaccgcgcgggcgaggagcccgaggagatgcgggacaggaggttcagcgcagggcgggagctgcggcaggggctgaaccgcgagcggctgctgcgcgaggaggactttgagcccgacgcgcggacggggatcagccccgcgcgcgcgcacgtggcggccgccgacctggtgacggcgtacgagcagacggtgaaccaggagatcaacttccaaaagagtttcaacaaccacgtgcgcacgctggtggcgcgcgaggaggtgaccatcgggctgatgcacctgtgggactttgtaagcgcgctggtgcagaaccccaacagcaagcctctgacggcgcagctgttcctgatagtgcagcacagcagggacaacgaggcgtttagggacgcgctgctgaacatcaccgagcccgagggtcggtggctgctggacctgattaacatcctgcagagcatagtggtgcaggagcgcagcctgagcctggccgacaaggtggcggccatcaactactcgatgctgagcctgggcaagttttacgcgcgcaagatctaccagacgccgtacgtgcccatagacaaggaggtgaagatcgacggtttttacatgcgcatggcgctgaaggtgctcaccctgagcgacgacctgggcgtgtaccgcaacgagcgcatccacaaggccgtgagcgtgagccggcggcgcgagctgagcgaccgcgagctgatgcacagcctgcagcgggcgctggcgggcgccggcagcggcgacagggaggcggagtcctacttcgatgcgggggcggacctgcgctgggcgcccagccggcgggccctggaggccgcgggggtccgcgaggactatgacgaggacggcgaggaggatgaggagtacgagctagaggagggcgagtacctggactaaaccgcgggtggtgtttccggtagatgcaagacccgaacgtggtggacccggcgctgcgggcggctctgcagagccagccgtccggccttaactcctcagacgactggcgacaggtcatggaccgcatcatgtcgctgacggcgcgtaacccggacgcgttccggcagcagccgcaggccaacaggctctccgccatcctggaggcggtggtgcctgcgcgctcgaaccccacgcacgagaaggtgctggccatagtgaacgcgctggccgagaacagggccatccgcccggacgaggccgggctggtgtacgacgcgctgctgcagcgcgtggcccgctacaacagcggcaacgtgcagaccaacctggaccggctggtgggggacgtgcgcgaggcggtggcgcagcgcgagcgcgcggatcggcagggcaacctgggctccatggtggcgctgaatgccttcctgagcacgcagccggccaacgtgccgcgggggcaggaagactacaccaactttgtgagcgcgctgcggctgatggtgaccgagaccccccagagcgaggtgtaccagtcgggcccggactacttcttccagaccagcagacagggcctgcagacggtgaacctgagccaggctttcaagaacctgcgggggctgtggggcgtgaaggcgcccaccggcgaccgggcgacggtgtccagcctgctgacgcccaactcgcgcctgctgctgctgctgatcgcgccgttcacggacagcggcagcgtgtcccgggacacctacctggggcacctgctgaccctgtaccgcgaggccatcgggcaggcgcaggtggacgagcacaccttccaggagatcaccagcgtgagccgcgcgctggggcaggaggacacgagcagcctggaggcgactctgaactacctgctgaccaaccggcggcagaagattccctcgctgcacagcctgacctccgaggaggagcgcatcttgcgctacgtgcagcagagcgtgagcctgaacctgatgcgcgacggggtgacgcccagcgtggcgctggacatgaccgcgcgcaacatggaaccgggcatgtacgccgcgcaccggccttacatcaaccgcctgatggactacctgcatcgcgcggcggccgtgaaccccgagtactttaccaacgccatcctgaacccgcactggctcccgccgcccgggttctacagcgggggcttcgaggtcccggagaccaacgatggcttcctgtgggacgacatggacgacagcgtgttctccccgcggccgcaggcgctggcggaagcgtccctgctgcgtcccaagaaggaggaggaggaggaggcgagtcgccgccgcggcagcagcggcgtggcttctctgtccgagctgggggcggcagccgccgcgcgccccgggtccctgggcggcagcccctttccgagcctggtggggtctctgcacagcgagcgcaccacccgccctcggctgctgggcgaggacgagtacctgaataactccctgctgcagccggtgcgggagaaaaacctgcctcccgccttccccaacaacgggatagagagcctggtggacaagatgagcagatggaagacctatgcgcaggagcacagggacgcgcctgcgctccggccgcccacgcggcgccagcgccacgaccggcagcgggggctggtgtgggatgacgaggactccgcggacgatagcagcgtgctggacctgggagggagcggcaacccgttcgcgcacctgcgcccccgcctggggaggatgttttaaaaaaaaaaaaaaaangcaagaagcatgatgcaaaaattaaataaaactcaccaaggccatggcgaccgagcgttggtttcttgtgttcccttcagtatgcggcgcgcggcgatgtaccaggagggacctcctccctcttacgagagcgtggtgggcgcggcggcggcggcgccctcttctccctttgcgtcgcagctgctggagccgccgtacgtgcctccgcgctacctgcggcctacgggggggagaaacagcatccgttactcggagctggcgcccctgttcgacaccacccgggtgtacctggtggacaacaagtcggcggacgtggcctccctgaactaccagaacgaccacagcaattttttgaccacggtcatccagaacaatgactacagcccgagcgaggccagcacccagaccatcaatctggatgaccggtcgcactggggcggcgacctgaaaaccatcctgcacaccaacatgcccaacgtgaacgagttcatgttcaccaataagttcaaggcgcgggtgatggtgtcgcgctcgcacaccaaggaagaccgggtggagctgaagtacgagtgggtggagttcgagctgccagagggcaactactccgagaccatgaccattgacctgatgaacaacgcgatcgtggagcactatctgaaagtgggcaggcagaacggggtcctggagagcgacatcggggtcaagttcgacaccaggaacttccgcctggggctggaccccgtgaccgggctggttatgcccggggtgtacaccaacgaggccttccatcccgacatcatcctgctgcccggctgcggggtggacttcacttacagccgcctgagcaacctcctgggcatccgcaagcggcagcccttccaggagggcttcaggatcacctacgaggacctggaggggggcaacatccccgcgctcctcgatgtggaggcctaccaggatagcttgaaggaaaatgaggcgggacaggaggataccgcccccgccgcctccgccgccgccgagcagggcgaggatgctgctgacaccgcggccgcggacggggcagaggccgaccccgctatggtggtggaggctcccgagcaggaggaggacatgaatgacagtgcggtgcgcggagacaccttcgtcacccggggggaggaaaagcaagcggaggccgaggccgcggccgaggaaaagcaactggcggcagcagcggcggcggcggcgttggccgcggcggaggctgagtctgaggggaccaagcccgccaaggagcccgtgattaagcccctgaccgaagatagcaagaagcgcagttacaacctgctcaaggacagcaccaacaccgcgtaccgcagctggtacctggcctacaactacggcgacccgtcgacgggggtgcgctcctggaccctgctgtgcacgccggacgtgacctgcggctcggagcaggtgtactggtcgctgcccgacatgatgcaagaccccgtgaccttccgctccacgcggcaggtcagcaacttcccggtggtgggcgccgagctgctgcccgtgcactccaagagcttctacaacgaccaggccgtctactcccagctcatccgccagttcacctctctgacccacgtgttcaatcgctttcctgagaaccagattctggcgcgcccgcccgcccccaccatcaccaccgtcagtgaaaacgttcctgctctcacagatcacgggacgctaccgctgcgcaacagcatcggaggagtccagcgagtgaccgttactgacgccagacgccgcacctgcccctacgtttacaaggccttgggcatagtctcgccgcgcgtcctttccagccgcactttttgagcaacaccaccatcatgtccatcctgatctcacccagcaataactccggctggggactgctgcgcgcgcccagcaagatgttcggaggggcgaggaagcgttccgagcagcaccccgtgcgcgtgcgcgggcacttccgcgccccctggggagcgcacaaacgcggccgcgcggggcgcaccaccgtggacgacgccatcgactcggtggtggagcaggcgcgcaactacaggcccgcggtctctaccgtggacgcggccatccagaccgtggtgcggggcgcgcggcggtacgccaagctgaagagccgccggaagcgcgtggcccgccgccaccgccgccgacccggggccgccgccaaacgcgccgccgcggccctgcttcgccgggccaagcgcacgggccgccgcgccgccatgagggccgcgcgccgcttggccgccggcatcaccgccgccaccatggccccccgtacccgaagacgcgcggccgccgccgccgccgccgccatcagtgacatggccagcaggcgccggggcaacgtgtactgggtgcgcgactcggtgaccggcacgcgcgtgcccgtgcgcttccgccccccgcggacttgagatgatgtgaaaaaacaacactgagtctcctgctgttgtgtgtatcccagcggcggcggcgcgcgcagcgtcatgtccaagcgcaaaatcaaagaagagatgctccaggtcgtcgcgccggagatctatgggcccccgaagaaggaagagcaggattcgaagccccgcaagataaagcgggtcaaaaagaaaaagaaagatgatgacgatgccgatggggaggtggagttcctgcgcgccacggcgcccaggcgcccggtgcagtggaagggccggcgcgtaaagcgcgtcctgcgccccggcaccgcggtggtcttcacgcccggcgagcgctccacccggactttcaagcgcgtctatgacgaggtgtacggcgacgaagacctgctggagcaggccaacgagcgcttcggagagtttgcttacgggaagcgtcagcgggcgctggggaaggaggacctgctggcgctgccgctggaccagggcaaccccacccccagtctgaagcccgtgaccctgcagcaggtgctgccgagcagcgcaccctccgaggcgaagcggggtctgaagcgcgagggcggcgacctggcgcccaccgtgcagctcatggtgcccaagcggcagaggctggaggatgtgctggagaaaatgaaagtagaccccggtctgcagccggacatcagggtccgccccatcaagcaggtggcgccgggcctcggcgtgcagaccgtggacgtggtcatccccaccggcaactcccccgccgccgccaccactaccgctgcctccacggacatggagacacagaccgatcccgccgcagccgcagccgcagccgccgccgcgacctcctcggcggaggtgcagacggacccctggctgccgccggcgatgtcagctccccgcgcgcgtcgcgggcgcaggaagtacggcgccgccaacgcgctcctgcccgagtacgccttgcatccttccatcgcgcccacccccggctaccgaggctatacctaccgcccgcgaagagccaagggttccacccgccgtccccgccgacgcgccgccgccaccacccgccgccgccgccgcagacgccagcccgcactggctccagtctccgtgaggaaagtggcgcgcgacggacacaccctggtgctgcccagggcgcgctaccaccccagcatcgtttaaaagcctgttgtggttcttgcagatatggccctcacttgccgcctccgtttcccggtgccgggataccgaggaggaagatcgcgccgcaggaggggtctggccggccgcggcctgagcggaggcagccgccgcgcgcaccggcggcgacgcgccaccagccgacgcatgcgcggcggggtgctgcccctgttaatccccctgatcgccgcggcgatcggcgccgtgcccgggatcgcctccgtggccttgcaagcgtcccagaggcattgacagacttgcaaacttgcaaatatggaaaaaaaaaccccaataaaaaagtctagactctcacgctcgcttggtcctgtgactattttgtagaatggaagacatcaactttgcgtcgctggccccgcgtcacggctcgcgcccgttcctgggacactggaacgatatcggcaccagcaacatgagcggtggcgccttcagttggggctctctgtggagcggcattaaaagtatcgggtctgccgttaaaaattacggctcccgggcctggaacagcagcacgggccagatgttgagagacaagttgaaagagcagaacttccagcagaaggtggtggagggcctggcctccggcatcaacggggtggtggacctggccaaccaggccgtgcagaataagatcaacagcagactggacccccggccgccggtggaggaggtgccgccggcgctggagacggtgtcccccgatgggcgtggcgagaagcgcccgcggcccgatagggaagagaccactctggtcacgcagaccgatgagccgcccccgtatgaggaggccctgaagcaaggtctgcccaccacgcggcccatcgcgcccatggccaccggggtggtgggccgccacacccccgccacgctggacttgcctccgcccgccgatgtgccgcagcagcagaaggcggcacagccgggcccgcccgcgaccgcctcccgttcctccgccggtcctctgcgccgcgcggccagcggcccccgcgggggggtcgcgaggcacggcaactggcagagcacgctgaacagcatcgtgggtctgggggtgcggtccgtgaagcgccgccgatgctactgaatagcttagctaacgtgttgtatgtgtgtatgcgccctatgtcgccgccagaggagctgctgagtcgccgccgttcgcgcgcccaccaccaccgccactccgcccctcaagatggcgaccccatcgatgatgccgcagtggtcgtacatgcacatctcgggccaggacgcctcggagtacctgagccccgggctggtgcagttcgcccgcgccaccgagagctacttcagcctgagtaacaagtttaggaaccccacggtggcgcccacgcacgatgtgaccaccgaccggtctcagcgcctgacgctgcggttcattcccgtggaccgcgaggacaccgcgtactcgtacaaggcgcggttcaccctggccgtgggcgacaaccgcgtgctggacatggcctccacctactttgacatccgcggggtgctggaccggggtcccactttcaagccctactctggcaccgcctacaactccctggcccccaagggcgctcccaactcctgcgagtgggagcaagaggaaactcaggcagttgaagaagcagcagaagaggaagaagaagatgctgacggtcaagctgaggaagagcaagcagctaccaaaaagactcatgtatatgctcaggctcccctttctggcgaaaaaattagtaaagatggtctgcaaataggaacggacgctacagctacagaacaaaaacctatttatgcagaccctacattccagcccgaaccccaaatcggggagtcccagtggaatgaggcagatgctacagtcgccggcggtagagtgctaaagaaatctactcccatgaaaccatgctatggttcctatgcaagacccacaaatgctaatggaggtcagggtgtactaacggcaaatgcccagggacagctagaatctcaggttgaaatgcaattcttttcaacttctgaaaacgcccgtaacgaggctaacaacattcagcccaaattggtgctgtatagtgaggatgtgcacatggagaccccggatacgcacctttcttacaagcccgcaaaaagcgatgacaattcaaaaatcatgctgggtcagcagtccatgcccaacagacctaattacatcggcttcagagacaactttatcggcctcatgtattacaatagcactggcaacatgggagtgcttgcaggtcaggcctctcagttgaatgcagtggtggacttgcaagacagaaacacagaactgtcctaccagctcttgcttgattccatgggtgacagaaccagatacttttccatgtggaatcaggcagtggacagttatgacccagatgttagaattattgaaaatcatggaactgaagacgagctccccaactattgtttccctctgggtggcataggggtaactgacacttaccaggctgttaaaaccaacaatggcaataacgggggccaggtgacttggacaaaagatgaaacttttgcagatcgcaatgaaataggggtgggaaacaatttcgctatggagatcaacctcagtgccaacctgtggagaaacttcctgtactccaacgtggcgctgtacctaccagacaagcttaagtacaacccctccaatgtggacatctctgacaaccccaacacctacgattacatgaacaagcgagtggtggccccggggctggtggactgctacatcaacctgggcgcgcgctggtcgctggactacatggacaacgtcaaccccttcaaccaccaccgcaatgcgggcctgcgctaccgctccatgctcctgggcaacgggcgctacgtgcccttccacatccaggtgccccagaagttctttgccatcaagaacctcctcctcctgccgggctcctacacctacgagtggaacttcaggaaggatgtcaacatggtcctccagagctctctgggtaacgatctcagggtggacggggccagcatcaagttcgagagcatctgcctctacgccaccttcttccccatggcccacaacacggcctccacgctcgaggccatgctcaggaacgacaccaacgaccagtccttcaatgactacctctccgccgccaacatgctctaccccatacccgccaacgccaccaacgtccccatctccatcccctcgcgcaactgggcggccttccgcggctgggccttcacccgcctcaagaccaaggagaccccctccctgggctcgggattcgacccctactacacctactcgggctccattccctacctggacggcaccttctacctcaaccacactttcaagaaggtctcggtcaccttcgactcctcggtcagctggccgggcaacgaccgtctgctcacccccaacgagttcgagatcaagcgctcggtcgacggggagggctacaacgtggcccagtgcaacatgaccaaggactggttcctggtccagatgctggccaactacaacatcggctaccagggcttctacatcccagagagctacaaggacaggatgtactccttcttcaggaacttccagcccatgagccggcaggtggtggaccagaccaagtacaaggactaccaggaggtgggcatcatccaccagcacaacaactcgggcttcgtgggctacctcgcccccaccatgcgcgagggacaggcctaccccgccaacttcccctatccgctcataggcaagaccgcggtcgacagcatcacccagaaaaagttcctctgcgaccgcaccctctggcgcatccccttctccagcaacttcatgtccatgggtgcgctctcggacctgggccagaacttgctctacgccaactccgcccacgccctcgacatgaccttcgaggtcgaccccatggacgagcccacccttctctatgttctgttcgaagtctttgacgtggtccgggtccaccagccgcaccgcggcgtcatcgagaccgtgtacctgcgtacgcccttctcggccggcaacgccaccacctaaagaagcaagccgcagtcatcgccgcctgcatgccgtcgggttccaccgagcaagagctcagggccatcgtcagagacctgggatgcgggccctattttttgggcaccttcgacaagcgcttccctggctttgtctccccacacaagctggcctgcgccatcgtcaacacggccggccgcgagaccgggggcgtgcactggctggccttcgcctggaacccgcgctccaaaacatgcttcctctttgaccccttcggcttttcggaccagcggctcaagcaaatctacgagttcgagtacgagggcttgctgcgtcgcagcgccatcgcctcctcgcccgaccgctgcgtcaccctcgaaaagtccacccagaccgtgcaggggcccgactcggccgcctgcggtctcttctgctgcatgtttctgcacgcctttgtgcactggcctcagagtcccatggaccgcaaccccaccatgaacttgctgacgggggtgcccaactccatgctccagagcccccaggtcgagcccaccctgcgccgcaaccaggagcagctctacagcttcctggagcgccactcgccttacttccgccgccacagcgcacagatcaggagggccacctccttctgccacttgcaagagatgcaagaagggtaataacgatgtacacactttttttctcaataaatggcatctttttatttatacaagctctctggggtattcatttcccaccaccacccgccgttgtcgccatctggctctatttagaaatcgaaagggttctgccgggagtcgccgtgcgccacgggcagggacacgttgcgatactggtagcgggtgccccacttgaactcgggcaccaccaggcgaggcagctcggggaagttttcgctccacaggctgcgggtcagcaccagcgcgttcatcaggtcgggcgccgagatcttgaagtcgcagttggggccgccgccctgcgcgcgcgagttgcggtacaccgggttgcagcactggaacaccaacagcgccgggtgcttcacgctggccagcacgctgcggtcggagatcagctcggcgtccaggtcctccgcgttgctcagcgcgaacggggtcatcttgggcacttgccgccccaggaagggcgcgtgccccggtttcgagttgcagtcgcagcgcagcgggatcagcaggtgcccgtgcccggactcggcgttggggtacagcgcgcgcatgaaggcctgcatctggcggaaggccatctgggccttggcgccctccgagaagaacatgccgcaggacttgcccgagaactggtttgcggggcagctggcgtcgtgcaggcagcagcgcgcgtcggtgttggcgatctgcaccacgttgcgcccccaccggttcttcacgatcttggccttggacgattgctccttcagcgcgcgctgcccgttctcgctggtcacatccatctcgatcacatgttccttgttcaccatgctgctgccgtgcagacacttcagctcgccctccgtctcggtgcagcggtgctgccacagcgcgcagcccgtgggctcgaaagacttgtaggtcacctccgcgaaggactgcaggtacccctgcaaaaagcggcccatcatggtcacgaaggtcttgttgctgctgaaggtcagctgcagcccgcggtgctcctcgttcagccaggtcttgcacacggccgccagcgcctccacctggtcgggcagcatcttgaagttcaccttcagctcattctccacgtggtacttgtccatcagcgtgcgcgccgcctccatgcccttctcccaggccgacaccagcggcaggctcacggggttcttcaccatcaccgtggccgccgcctccgccgcgctttcgctttccgccccgctgttctcttcctcttcctcctcttcctcgccgccgcccactcgcagcccccgcaccacggggtcgtcttcctgcaggcgctgcaccttgcgcttgccgttgcgcccctgcttgatgcgcacgggcgggttgctgaagcccaccatcaccagcgcggcctcttcttgctcgtcctcgctgtccagaatgacctccggggagggggggttggtcatcctcagtaccgaggcacgcttctttttcttcctgggggcgttcgccagctccgcggctgcggccgctgccgaggtcgaaggccgagggctgggcgtgcgcggcaccagcgcgtcctgcgagccgtcctcgtcctcctcggactcgagacggaggcgggcccgcttcttcgggggcgcgcggggcggcggaggcggcggcggcgacggagacggggacgagacatcgtccagggtgggtggacggcgggccgcgccgcgtccgcgctcgggggtggtctcgcgctggtcctcttcccgactggccatctcccactgctccttctcctataggcagaaagagatcatggagtctctcatgcgagtcgagaaggaggaggacagcctaaccgccccctctgagccctccaccaccgccgccaccaccgccaatgccgccgcggacgacgcgcccaccgagaccaccgccagtaccaccctccccagcgacgcacccccgctcgagaatgaagtgctgatcgagcaggacccgggttttgtgagcggagaggaggatgaggtggatgagaaggagaaggaggaggtcgccgcctcagtgccaaaagaggataaaaagcaagaccaggacgacgcagataaggatgagacagcagtcgggcgggggaacggaagccatgatgctgatgacggctacctagacgtgggagacgacgtgctgcttaagcacctgcaccgccagtgcgtcatcgtctgcgacgcgctgcaggagcgctgcgaagtgcccctggacgtggcggaggtcagccgcgcctacgagcggcacctcttcgcgccgcacgtgccccccaagcgccgggagaacggcacctgcgagcccaacccgcgtctcaacttctacccggtcttcgcggtacccgaggtgctggccacctaccacatctttttccaaaactgcaagatccccctctcctgccgcgccaaccgcacccgcgccgacaaaaccctgaccctgcggcagggcgcccacatacctgatatcgcctctctggaggaagtgcccaagatcttcgagggtctcggtcgcgacgagaaacgggcggcgaacgctctgcacggagacagcgaaaacgagagtcactcgggggtgctggtggagctcgagggcgacaacgcgcgcctggccgtactcaagcgcagcatagaggtcacccactttgcctacccggcgctcaacctgccccccaaggtcatgagtgtggtcatgggcgagctcatcatgcgccgcgcccagcccctggccgcggatgcaaacttgcaagagtcctccgaggaaggcctgcccgcggtcagcgacgagcagctggcgcgctggctggagacccgcgaccccgcgcagctggaggagcggcgcaagctcatgatggccgcggtgctggtcaccgtggagctcgagtgtctgcagcgcttcttcgcggaccccgagatgcagcgcaagctcgaggagaccctgcactacaccttccgccagggctacgtgcgccaggcctgcaagatctccaacgtggagctctgcaacctggtctcctacctgggcatcctgcacgagaaccgcctcgggcagaacgtcctgcactccaccctcaaaggggaggcgcgccgcgactacatccgcgactgcgcctacctcttcctctgctacacctggcagacggccatgggggtctggcagcagtgcctggaggagcgcaacctcaaggagctggaaaagctcctcaagcgcaccctcagggacctctggacgggcttcaacgagcgctcggtggccgccgcgctggcggacatcatctttcccgagcgcctgctcaagaccctgcagcagggcctgcccgacttcaccagccagagcatgctgcagaacttcaggactttcatcctggagcgctcgggcatcctgccggccacttgctgcgcgctgcccagcgacttcgtgcccatcaagtacagggagtgcccgccgccgctctggggccactgctacctcttccagctggccaactacctcgcctaccactcggacctcatggaagacgtgagcggcgagggcctgctcgagtgccactgccgctgcaacctctgcacgccccaccgctctctagtctgcaacccgcagctgctcagcgagagtcagattatcggtaccttcgagctgcagggtccctcgcctgacgagaagtccgcggctccagggctgaaactcactccggggctgtggacttccgcctacctacgcaaatttgtacctgaggactaccacgcccacgagatcaggttctacgaagaccaatcccgcccgcccaaggcggagctcaccgcctgcgtcatcacccaggggcacatcctgggccaattgcaagccatcaacaaagcccgccgagagttcttgctgaaaaagggtcggggggtgtacctggacccccagtccggcgaggagctaaacccgctacccccgccgccgccccagcagcgggaccttgcttcccaggatggcacccagaaagaagcagcagccgccgccgccgccgcagccatacatgcttctggaggaagaggaggaggactgggacagtcaggcagaggaggtttcggacgaggagcaggaggagatgatggaagactgggaggaggacagcagcctagacgaggaagcttcagaggccgaagaggtggcagacgcaacaccatcgccctcggtcgcagccccctcgccggggcccctgaaatcctccgaacccagcaccagcgctataacctccgctcctccggcgccggcgccacccgcccgcagacccaaccgtagatgggacaccacaggaaccggggtcggtaagtccaagtgcccgccgccgccaccgcagcagcagcagcagcagcgccagggctaccgctcgtggcgcgggcacaagaacgccatagtcgcctgcttgcaagactgcgggggcaacatctctttcgcccgccgcttcctgctattccaccacggggtcgcctttccccgcaatgtcctgcattactaccgtcatctctacagcccctactgcagcggcgacccagaggcggcagcggcagccacagcggcgaccaccacctaggaagatatcctccgcgggcaagacagcggcagcagcggccaggagacccgcggcagcagcggcgggagcggtgggcgcactgcgcctctcgcccaacgaacccctctcgacccgggagctcagacacaggatcttccccactttgtatgccatcttccaacagagcagaggccaggagcaggagctgaaaataaaaaacagatctctgcgctccctcacccgcagctgtctgtatcacaaaagcgaagatcagcttcggcgcacgctggaggacgcggaggcactcttcagcaaatactgcgcgctcactcttaaagactagctccgcgcccttctcgaatttaggcgggagaaaactacgtcatcgccggccgccgcccagcccgcccagccgagatgagcaaagagattcccacgccatacatgtggagctaccagccgcagatgggactcgcggcgggagcggcccaggactactccacccgcatgaactacatgagcgcgggaccccacatgatctcacaggtcaacgggatccgcgcccagcgaaaccaaatactgctggaacaggcggccatcaccgccacgccccgccataatctcaacccccgaaattggcccgccgccctcgtgtaccaggaaaccccctccgccaccaccgtactacttccgcgtgacgcccaggccgaagtccagatgactaactcaggggcgcagctcgcgggcggctttcgtcacggggcgcggccgctccgaccaggtataagacacctgatgatcagaggccgaggtatccagctcaacgacgagtcggtgagctcttcgctcggtctccgtccggacggaactttccagctcgccggatccggccgctcttcgttcacgccccgccaggcgtacctgactctgcagacctcgtcctcggagccccgctccggcggcatcggaaccctccagttcgtggaggagttcgtgccctcggtctacttcaaccccttctcgggacctcccggacgctaccccgaccagttcattccgaactttgacgcggtgaaggactcggcggacggctacgactgaatgtcaggtgtcgaggcagagcagcttcgcctgagacacctcgagcactgccgccgccacaagtgcttcgcccgcggttctggtgagttctgctactttcagctacccgaggagcataccgaggggccggcgcacggcgtccgcctgaccacccagggcgaggttacctgttccctcatccgggagtttaccctccgtcccctgctagtggagcgggagcggggtccctgtgtcctaactatcgcctgcaactgccctaaccctggattacatcaagatctttgctgtcatctctgtgctgagtttaataaacgctgagatcagaatctactggggctcctgtcgccatcctgtgaacgccaccgtcttcacccaccccgaccaggcccaggcgaacctcacctgcggtctgcatcggagggccaagaagtacctcacctggtacttcaacggcaccccctttgtggtttacaacagcttcgacggggacggagtctccctgaaagaccagctctccggtctcagctactccatccacaagaacaccaccctccaactcttccctccctacctgccgggaacctacgagtgcgtcaccggccgctgcacccacctcacccgcctgatcgtaaaccagagctttccgggaacagataactccctcttccccagaacaggaggtgagctcaggaaactccccggggaccagggcggagacgtaccttcgacccttgtggggttaggattttttattaccgggttgctggctcttttaatcaaagtttccttgagatttgttctttccttctacgtgtatgaacacctcaacctccaataactctaccctttcttcggaatcaggtgacttctctgaaatcgggcttggtgtgctgcttactctgttgatttttttccttatcatactcagccttctgtgcctcaggctcgccgcctgctgcgcacacatctatatctactgctggttgctcaagtgcaggggtcgccacccaagatgaacaggtacatggtcctatcgatcctaggcctgctggccctggcggcctgcagcgccgccaaaaaagagattacctttgaggagcccgcttgcaatgtaactttcaagcccgagggtgaccaatgcaccaccctcgtcaaatgcgttaccaatcatgagaggctgcgcatcgactacaaaaacaaaactggccagtttgcggtctatagtgtgtttacgcccggagacccctctaactactctgtcaccgtcttccagggcggacagtctaagatattcaattacactttccctttttatgagttatgcgatgcggtcatgtacatgtcaaaacagtacaacctgtggcctccctctccccaggcgtgtgtggaaaatactgggtcttactgctgtatggctttcgcaatcactacgctcgctctaatctgcacggtgctatacataaaattcaggcagaggcgaatctttatcgatgaaaagaaaatgccttgatcgctaacaccggctttctatctgcagaatgaatgcaatcacctccctactaatcaccaccaccctccttgcgattgcccatgggttgacacgaatcgaagtgccagtggggtccaatgtcaccatggtgggccccgccggcaattccaccctcatgtgggaaaaatttgtccgcaatcaatgggttcatttctgctctaaccgaatcagtatcaagcccagagccatctgcgatgggcaaaatctaactctgatcaatgtgcaaatgatggatgctgggtactattacgggcagcggggagaaatcattaattactggcgaccccacaaggactacatgctgcatgtagtcgaggcacttcccactaccacccccactaccacctctcccaccaccaccaccactactactactactactactactactactactaccactaccgctgcccgccatacccgcaaaagcaccatgattagcacaaagccccctcgtgctcactcccacgccggcgggcccatcggtgcgacctcagaaaccaccgagctttgcttctgccaatgcactaacgccagcgctcatgaactgttcgacctggagaatgaggatgtccagcagagctccgcttgcctgacccaggaggctgtggagcccgttgccctgaagcagatcggtgattcaataattgactcttcttcttttgccactcccgaataccctcccgattctactttccacatcacgggtaccaaagaccctaacctctctttctacctgatgctgctgctctgtatctctgtggtctcttccgcgctgatgttactggggatgttctgctgcctgatctgccgcagaaagagaaaagctcgctctcagggccaaccactgatgcccttcccctaccccccggattttgcagataacaagatatgagctcgctgctgacactaaccgctttactagcctgcgctctaacccttgtcgcttgcgactcgagattccacaatgtcacagctgtggcaggagaaaatgttactttcaactccacggccgatacccagtggtcgtggagtggctcaggtagctacttaactatctgcaatagctccacttcccccggcatatccccaaccaagtaccaatgcaatgccagcctgttcaccctcatcaacgcttccaccctggacaatggactctatgtaggctatgtaccctttggtgggcaaggaaagacccacgcttacaacctggaagttcgccagcccagaaccactacccaagcttctcccaccaccaccaccaccaccaccatcaccagcagcagcagcagcagcagccacagcagcagcagcagattattgactttggttttggccagctcatctgccgctacccaggccatctacagctctgtgcccgaaaccactcagatccaccgcccagaaacgaccaccgccaccaccctacacacctccagcgatcagatgccgaccaacatcacccccttggctcttcaaatgggacttacaagccccactccaaaaccagtggatgcggccgaggtctccgccctcgtcaatgactgggcggggctgggaatgtggtggttcgccataggcatgatggcgctctgcctgcttctgctctggctcatctgctgcctccaccgcaggcgagccagaccccccatctatagacccatcattgtcctgaaccccgataatgatgggatccatagattggatggcctgaaaaacctacttttttcttttacagtatgataaattgagacatgcctcgcattttcttgtacatgttccttctcccaccttttctggggtgttctacgctggccgctgtgtctcacctggaggtagactgcctctcacccttcactgtctacctgctttacggattggtcaccctcactctcatctgcagcctaatcacagtaatcatcgccttcatccagtgcattgattacatctgtgtgcgcctcgcatacttcagacaccacccgcagtaccgagacaggaacattgcccaacttctaagactgctctaatcatgcataagactgtgatctgccttctgatcctctgcatcctgcccaccctcacctcctgccagtacaccacaaaatctccgcgcaaaagacatgcctcctgccgcttcacccaactgtggaatatacccaaatgctacaacgaaaagagcgagctctccgaagcttggctgtatggggtcatctgtgtcttagttttctgcagcactgtctttgccctcataatctacccctactttgatttgggatggaacgcgatcgatgccatgaattaccccacctttcccgcacccgagataattccactgcgacaagttgtacccgttgtcgttaatcaacgccccccatcccctacgcccactgaaatcagctactttaacctaacaggcggagatgactgacgccctagatctagaaatggacggcatcagtaccgagcagcgtctcctagagaggcgcaggcaggcggctgagcaagagcgcctcaatcaggagctccgagatctcgttaacctgcaccagtgcaaaagaggcatcttttgtctggtaaagcaggccaaagtcacctacgagaagaccggcaacagccaccgcctcagttacaaattgcccacccagcgccagaagctggtgctcatggtgggtgagaatcccatcaccgtcacccagcactcggtagagaccgaggggtgtctgcactccccctgtcggggtccagaagacctctgcaccctggtaaagaccctgtgcggtctcagagatttagtcccctttaactaatcaaacactggaatcaataaaaagaatcacttacttaaaatcagacagcaggtctctgtccagtttattcagcagcacctccttcccctcctcccaactctggtactccaaacgccttctggcggcaaacttcctccacaccctgaagggaatgtcagattcttgctcctgtccctccgcacccactatcttcatgttgttgcagatgaagcgcaccaaaacgtctgacgagagcttcaaccccgtgtacccctatgacacggaaagcggccctccctccgtccctttcctcacccctcccttcgtgtctcccgatggattccaagaaagtccccccggggtcctgtctctgaacctggccgagcccctggtcacttcccacggcatgctcgccctgaaaatgggaagtggcctctccctggacgacgctggcaacctcacctctcaagatatcaccaccgctagccctcccctcaaaaaaaccaagaccaacctcagcctagaaacctcatcccccctaactgtgagcacctcaggcgccctcaccgtagcagccgccgctcccctggcggtggccggcacctccctcaccatgcaatcagaggcccccctgacagtacaggatgcaaaactcaccctggccaccaaaggccccctgaccgtgtctgaaggcaaactggccttgcaaacatcggccccgctgacggccgctgacagcagcaccctcacagtcagtgccacaccaccccttagcacaagcaatggcagcttgggtattgacatgcaagcccccatttacaccaccaatggaaaactaggacttaactttggcgctcccctgcatgtggtagacagcctaaatgcactgactgtagttactggccaaggtcttacgataaacggaacagccctacaaactagagtctcaggtgccctcaactatgacacatcaggaaacctagaattgagagctgcagggggtatgcgagttgatgcaaatggtcaacttatccttgatgtagcttacccatttgatgcacaaaacaatctcagccttaggcttggacagggacccctgtttgttaactctgcccacaacttggatgttaactacaacagaggcctctacctgttcacatctggaaataccaaaaagctagaagttaatatcaaaacagccaagggtctcatttatgatgacactgctatagcaatcaatgcgggtgatgggctacagtttgactcaggctcagatacaaatccattaaaaactaaacttggattaggactggattatgactccagcagagccataattgctaaactgggaactggcctaagctttgacaacacaggtgccatcacagtaggcaacaaaaatgatgacaagcttaccttgtggaccacaccagacccatcccctaactgtagaatctattcagagaaagatgctaaattcacacttgttttgactaaatgcggcagtcaggtgttggccagcgtttctgttttatctgtaaaaggtagccttgcgcccatcagtggcacagtaactagtgctcagattgtcctcagatttgatgaaaatggagttctactaagcaattcttcccttgaccctcaatactggaactacagaaaaggtgaccttacagagggcactgcatataccaacgcagtgggatttatgcccaacctcacagcatacccaaaaacacagagccaaactgctaaaagcaacattgtaagtcaggtttacttgaatggggacaaatccaaacccatgaccctcaccattaccctcaatggaactaatgaaacaggagatgccacagtaagcacttactccatgtcattctcatggaactggaatggaagtaattacattaatgaaacgttccaaaccaactccttcaccttctcctacatcgcccaagaataaaaagcatgacgctgttgatttgattcaatgtgtttctgttttattttcaagcacaacaaaatcattcaagtcattcttccatcttagcttaatagacacagtagcttaatagacccagtagtgcaaagccccattctagcttataactagtggagaagtactcgcctacatgggggtagagtcataatcgtgcatcaggatagggcggtggtgctgcagcagcgcgcgaataaactgctgccgccgccgctccgtcctgcaggaatacaacatggcagtggtctcctcagcgatgattcgcaccgcccgcagcataaggcgccttgtcctccgggcacagcagcgcaccctgatctcacttaaatcagcacagtaactgcagcacagcaccacaatattgttcaaaatcccacagtgcaaggcgctgtatccaaagctcatggcggggaccacagaacccacgtggccatcataccacaagcgcaggtagattaagtggcgacccctcataaacacgctggacataaacattacctcttttggcatgttgtaattcaccacctcccggtaccatataaacctctgattaaacatggcgccatccaccaccatcctaaaccagctggccaaaacctgcccgccggctatacactgcagggaaccgggactggaacaatgacagtggagagcccaggactcgtaaccatggatcatcatgctcgtcatgatatcaatgttggcacaacacaggcacacgtgcatacacttcctcaggattacaagctcctcccgcgttagaaccatatcccagggaacaacccattcctgaatcagcgtaaatcccacactgcagggaagacctcgcacgtaactcacgttgtgcattgtcaaagtgttacattcgggcagcagcggatgatcctccagtatggtagcgcgggtttctgtctcaaaaggaggtagacgatccctactgtacggagtgcgccgagacaaccgagatcgtgttggtcgtagtgtcatgccaaatggaacgccggacgtagtcatatttcctgaagtcttagatctctcaacgcagcaccagcaccaacacttcgcagtgtaaaaggccaagtgccgagagagtatatataggaataaaaagtgacgtaaacgggcaaagtccaaaaaacgcccagaaaaaccgcacgcgaacctacgccccgaaacgaaagccaaaaaacactagacactcccttccggcgtcaacttccgctttcccacgctacgtcacttgccccagtcaaacaaactacatatcccgaacttccaagtcgccacgcccaaaacaccgcctacacctccccgcccgccggcccgcccccaaacccgcctcccgccccgcgccccgccccgcgccgcccatctcattatcatattggcttcaatccaaaataaggtatattattgatgatggtttaaacggatcctctagagtcgacctgcaggcatgcaagcttgagtataacccccttgcggccgcccgggccgtcgaccaattctcatgtttgacagcttatcatcgaatttctgccattcatccgcttattatcacttattcaggcgtagcaaccaggcgtttaagggcaccaataactgccttaaaaaaattacgccccgccctgccactcatcgcagtactgttgtaattcattaagcattctgccgacatggaagccatcacaaacggcatgatgaacctgaatcgccagcggcatcagcaccttgtcgccttgcgtataatatttgcccatggtgaaaacgggggcgaagaagttgtccatattggccacgtttaaatcaaaactggtgaaactcacccagggattggctgagacgaaaaacatattctcaataaaccctttagggaaataggccaggttttcaccgtaacacgccacatcttgcgaatatatgtgtagaaactgccggaaatcgtcgtggtattcactccagagcgatgaaaacgtttcagtttgctcatggaaaacggtgtaacaagggtgaacactatcccatatcaccagctcaccgtctttcattgccatacggaattccggatgagcattcatcaggcgggcaagaatgtgaataaaggccggataaaacttgtgcttatttttctttacggtctttaaaaaggccgtaatatccagctgaacggtctggttataggtacattgagcaactgactgaaatgcctcaaaatgttctttacgatgccattgggatatatcaacggtggtatatccagtgatttttttctccattttagcttccttagctcctgaaaatctcgataactcaaaaaatacgcccggtagtgatcttatttcattatggtgaaagttggaacctcttacgtgccgatcaacgtctcattttcgccaaaagttggcccagggcttcccggtatcaacagggacaccaggatttatttattctgcgaagtgatcttccgtcacaggtatttattcgcgataagctcatggagcggcgtaaccgtcgcacaggaaggacagagaaagcgcggatctgggaagtgacggacagaacggtcaggacctggattggggaggcggttgccgccgctgctgctgacggtgtgacgttctctgttccggtcacaccacatacgttccgccattcctatgcgatgcacatgctgtatgccggtataccgctgaaagttctgcaaagcctgatgggacataagtccatcagttcaacggaagtctacacgaaggtttttgcgctggatgtggctgcccggcaccgggtgcagtttgcgatgccggagtctgatgcggttgcgatgctgaaacaattatcctgagaataaatgccttggcctttatatggaaatgtggaactgagtggatatgctgtttttgtctgttaaacagagaagctggctgttatccactgagaagcgaacgaaacagtcgggaaaatctcccattatcgtagagatccgcattattaatctcaggagcctgtgtagcgtttataggaagtagtgttctgtcatgatgcctgcaagcggtaacgaaaacgatttgaatatgccttcaggaacaatagaaatcttcgtgcggtgttacgttgaagtggagcggattatgtcagcaatggacagaacaacctaatgaacacagaaccatgatgtggtctgtccttttacagccagtagtgctcgccgcagtcgagcgacagggcgaagccctcgagtgagcgaggaagcaccagggaacagcacttatatattctgcttacacacgatgcctgaaaaaacttcccttggggttatccacttatccacggggatatttttataattattttttttatagtttttagatcttcttttttagagcgccttgtaggcctttatccatgctggttctagagaaggtgttgtgacaaattgccctttcagtgtgacaaatcaccctcaaatgacagtcctgtctgtgacaaattgcccttaaccctgtgacaaattgccctcagaagaagctgttttttcacaaagttatccctgcttattgactcttttttatttagtgtgacaatctaaaaacttgtcacacttcacatggatctgtcatggcggaaacagcggttatcaatcacaagaaacgtaaaaatagcccgcgaatcgtccagtcaaacgacctcactgaggcggcatatagtctctcccgggatcaaaaacgtatgctgtatctgttcgttgaccagatcagaaaatctgatggcaccctacaggaacatgacggtatctgcgagatccatgttgctaaatatgctgaaatattcggattgacctctgcggaagccagtaaggatatacggcaggcattgaagagtttcgcggggaaggaagtggttttttatcgccctgaagaggatgccggcgatgaaaaaggctatgaatcttttccttggtttatcaaacgtgcgcacagtccatccagagggctttacagtgtacatatcaacccatatctcattcccttctttatcgggttacagaaccggtttacgcagtttcggcttagtgaaacaaaagaaatcaccaatccgtatgccatgcgtttatacgaatccctgtgtcagtatcgtaagccggatggctcaggcatcgtctctctgaaaatcgactggatcatagagcgttaccagctgcctcaaagttaccagcgtatgcctgacttccgccgccgcttcctgcaggtctgtgttaatgagatcaacagcagaactccaatgcgcctctcatacattgagaaaaagaaaggccgccagacgactcatatcgtattttccttccgcgatatcacttccatgacgacaggatagtctgagggttatctgtcacagatttgagggtggttcgtcacatttgttctgacctactgagggtaatttgtcacagttttgctgtttccttcagcctgcatggattttctcatactttttgaactgtaatttttaaggaagccaaatttgagggcagtttgtcacagttgatttccttctctttcccttcgtcatgtgacctgatatcgggggttagttcgtcatcattgatgagggttgattatcacagtttattactctgaattggctatccgcgtgtgtacctctacctggagtttttcccacggtggatatttcttcttgcgctgagcgtaagagctatctgacagaacagttcttctttgcttcctcgccagttcgctcgctatgctcggttacacggctgcggcgagcgctagtgataataagtgactgaggtatgtgctcttcttatctccttttgtagtgttgctcttattttaaacaactttgcggttttttgatgactttgcgattttgttgttgctttgcagtaaattgcaagatttaataaaaaaacgcaaagcaatgattaaaggatgttcagaatgaaactcatggaaacacttaaccagtgcataaacgctggtcatgaaatgacgaaggctatcgccattgcacagtttaatgatgacagcccggaagcgaggaaaataacccggcgctggagaataggtgaagcagcggatttagttggggtttcttctcaggctatcagagatgccgagaaagcagggcgactaccgcacccggatatggaaattcgaggacgggttgagcaacgtgttggttatacaattgaacaaattaatcatatgcgtgatgtgtttggtacgcgattgcgacgtgctgaagacgtatttccaccggtgatcggggttgctgcccataaaggtggcgtttacaaaacctcagtttctgttcatcttgctcaggatctggctctgaaggggctacgtgttttgctcgtggaaggtaacgacccccagggaacagcctcaatgtatcacggatgggtaccagatcttcatattcatgcagaagacactctcctgcctttctatcttggggaaaaggacgatgtcacttatgcaataaagcccacttgctggccggggcttgacattattccttcctgtctggctctgcaccgtattgaaactgagttaatgggcaaatttgatgaaggtaaactgcccaccgatccacacctgatgctccgactggccattgaaactgttgctcatgactatgatgtcatagttattgacagcgcgcctaacctgggtatcggcacgattaatgtcgtatgtgctgctgatgtgctgattgttcccacgcctgctgagttgtttgactacacctccgcactgcagtttttcgatatgcttcgtgatctgctcaagaacgttgatcttaaagggttcgagcctgatgtacgtattttgcttaccaaatacagcaatagtaatggctctcagtccccgtggatggaggagcaaattcgggatgcctggggaagcatggttctaaaaaatgttgtacgtgaaacggatgaagttggtaaaggtcagatccggatgagaactgtttttgaacaggccattgatcaacgctcttcaactggtgcctggagaaatgctctttctatttgggaacctgtctgcaatgaaattttcgatcgtctgattaaaccacgctgggagattagataatgaagcgtgcgcctgttattccaaaacatacgctcaatactcaaccggttgaagatacttcgttatcgacaccagctgccccgatggtggattcgttaattgcgcgcgtaggagtaatggctcgcggtaatgccattactttgcctgtatgtggtcgggatgtgaagtttactcttgaagtgctccggggtgatagtgttgagaagacctctcgggtatggtcaggtaatgaacgtgaccaggagctgcttactgaggacgcactggatgatctcatcccttcttttctactgactggtcaacagacaccggcgttcggtcgaagagtatctggtgtcatagaaattgccgatgggagtcgccgtcgtaaagctgctgcacttaccgaaagtgattatcgtgttctggttggcgagctggatgatgagcagatggctgcattatccagattgggtaacgattatcgcccaacaagtgcttatgaacgtggtcagcgttatgcaagccgattgcagaatgaatttgctggaaatatttctgcgctggctgatgcggaaaatatttcacgtaagattattacccgctgtatcaacaccgccaaattgcctaaatcagttgttgctcttttttctcaccccggtgaactatctgcccggtcaggtgatgcacttcaaaaagcctttacagataaagaggaattacttaagcagcaggcatctaaccttcatgagcagaaaaaagctggggtgatatttgaagctgaagaagttatcactcttttaacttctgtgcttaaaacgtcatctgcatcaagaactagtttaagctcacgacatcagtttgctcctggagcgacagtattgtataagggcgataaaatggtgcttaacctggacaggtctcgtgttccaactgagtgtatagagaaaattgaggccattcttaaggaacttgaaaagccagcaccctgatgcgaccacgttttagtctacgtttatctgtctttacttaatgtcctttgttacaggccagaaagcataactggcctgaatattctctctgggcccactgttccacttgtatcgtcggtctgataatcagactgggaccacggtcccactcgtatcgtcggtctgattattagtctgggaccacggtcccactcgtatcgtcggtctgattattagtctgggaccacggtcccactcgtatcgtcggtctgataatcagactgggaccacggtcccactcgtatcgtcggtctgattattagtctgggaccatggtcccactcgtatcgtcggtctgattattagtctgggaccacggtcccactcgtatcgtcggtctgattattagtctggaaccacggtcccactcgtatcgtcggtctgattattagtctgggaccacggtcccactcgtatcgtcggtctgattattagtctgggaccacgatcccactcgtgttgtcggtctgattatcggtctgggaccacggtcccacttgtattgtcgatcagactatcagcgtgagactacgattccatcaatgcctgtcaagggcaagtattgacatgtcgtcgtaacctgtagaacggagtaacctcggtgtgcggttgtatgcctgctgtggattgctgctgtgtcctgcttatccacaacattttgcgcacggttatgtggacaaaatacctggttacccaggccgtgccggcacgctcggtacccggggatcctcgtttaaac

SEQ ID NO: 51 - DNA, 41464 bp, Artificial Sequence
  source: /note="Description of Artificial Sequence: Synthetic polynucleotide"
  modified_base (16063)..(16063): a, c, t, g, unknown or other
catcatcaataatataccttattttggattgaagccaatatgataatgagatgggcggcgcggggcggggcgcggggcgggaggcgggtttgggggcgggccggcgggcggggcggtgtggcggaagtggactttgtaagtgtggcggatgtgacttgctagtgccgggcgcggtaaaagtgacgttttccgtgcgcgacaacgcccccgggaagtgacatttttcccgcggtttttaccggatgttgtagtgaatttgggcgtaaccaagtaagatttggccattttcgcgggaaaactgaaacggggaagtgaaatctgattaattttgcgttagtcataccgcgtaatatttgtctagggccgagggactttggccgattacgtggaggactcgcccaggtgttttttgaggtgaatttccgcgttccgggtcaaagtctgcgttttattattataggatatcccattgcatacgttgtatccatatcataatatgtacatttatattggctcatgtccaacattaccgccatgttgacattgattattgactagttattaatagtaatcaattacggggtcattagttcatagcccatatatggagttccgcgttacataacttacggtaaatggcccgcctggctgaccgcccaacgacccccgcccattgacgtcaataatgacgtatgttcccatagtaacgccaatagggactttccattgacgtcaatgggtggagtatttacggtaaactgcccacttggcagtacatcaagtgtatcatatgccaagtacgccccctattgacgtcaatgacggtaaatggcccgcctggcattatgcccagtacatgaccttatgggactttcctacttggcagtacatctacgtattagtcatcgctattaccatggtgatgcggttttggcagtacatcaatgggcgtggatagcggtttgactcacggggatttccaagtctccaccccattgacgtcaatgggagtttgttttggcaccaaaatcaacgggactttccaaaatgtcgtaacaactccgccccattgacgcaaatgggcggtaggcgtgtacggtgggaggtctatataagcagagctctccctatcagtgatagagatctccctatcagtgatagagatcgtcgacgagctcgtttagtgaaccgtcagatcgcctggagacgccatccacgctgttttgacctccatagaagacaccgggaccgatccagcctccgcggccgggaacggtgcattggaacgcggattccccgtgccaagagtgagatcttccgtttatctaggtaccagatatcgccaccatgagacctgctccctggacacctaatcctcccaggtcccccagccagatgagcgtgagagacagactggctaggctgagagccgaggctcaggtcaagcaggccagcgtcgaggtgcaaccccctcagctcacccaggtgtccccccagcagcctgtggccggcattctgttcattctggccattctgaccgagtggggaagcggcaacagaacctacggccctgtcttcatgtgcctcggaggactgctgacaatggtggctggcgccgtgtggctcaccgtcatgtccaacaccctgctcagcgcctggattctgaccgccggattcctgatctttctgatcggattcgctctctttggcgtcatcaggtgttgcaggtactgttgctactactgcctgaccctcgagagcgaggaaagaccccccaccccctacaggaatacagtgaggaaacctcagcagcccgagagcctcgaggagtgcgatagcgagctggagattaaaaggtataagaatagggtggcctccaggaagtgtagggctaaattcaaacagctcctgcaacactatagggaagtggccgccgccaagtccagcgagattagggacagaaggaggaatcctgcctccaggagagaccaggccaaatggagactccaaacactcgccgctggatggcccatgggctaccaggcctatagctcctggatgtacagctacaccgaccatcagacaacacccaccttcgtgcatctgcaggctacactgggctgcaccggaggcagaaggtgtcacgtgtttctgggaatcgtgctgttcatctttggatgcctgctcgtgctgggcatctggatttatctcctggagatgctctggagactcggcgctacaatttggcagctgctcgccttttttctggccttctttctggacctgatcctcctgatcatcgccctgtacctccaacagaactggtggaccctcctggtggatctgctgtggctcctcctcttcctggccatcctgatctggatgtactaccatggccagagaggaagggtcgcttgcgctcctgtccctgctcctgctggccccatcgtgaggccttgggagccttccctcacacaggccgccggccaggcctttgctcccgtgaggccccagcacatgcctgtggaacccgtgcccgtccccacagtggctctggaaaggcctgtgtaccccaagcccgtgagacctgtcctctggctcagcagccctggaggactcggaacactcggagccgctctcctgacactggccgctgctctggctctgctggctagcctgatcctgggaaccctcaacctcaccaccatgtttctcctcatgctcctgtggaccctcgtggtgctgctcatctgttccagctgctccagctgccccctgagcaagatcctgctggccaggctgttcctgtacgccctcgccctcctgctgctggctagcgccctgatcgctggcggaagcatcctccagaccaatttcaagagcctctcctccaccgagttcatccccaacctgttctgtatgttactgctgatccatagcgacgagcaccatcatgacgactccctgccccatcctcagcaggccacagacgactccggccacgagagcgacagcaatagcaatgagggcaggcaccatctgctcgtgtccggagctcaagtccccgagcctcccaccatccatctcgccgcccagggaatggcttaccccctccacgagcagcacggcatggccccttgtcccgtcgctcaagccccccctacacctctgccctttttcgccatttgtctgacctggagaatcgaggacccccccttcaacagcctgctgttcgccctgctcgccgccgctggcggcctccagggcatttacgtcctcgtgatgctggtgctgctgatcctcgcttacaggagaagatggaggagactgacagtgtgcggcggcatcatgtttctcgcctgcgtcctggtcctgatcgtggacgccgtcctgcaactcagccccctcctgggagctgtgacagtggtctccatgaccctgctgctgctggccttcaacggaccccacgatcctctgccccaagatcctgacaataccgacgataacggcccccaagaccccgataacaccgacgacaatggccctcacgaccctctgccccatagcccttccgatagcgctggcaacgatggcggccctcctcagctgacagaggaggtggaaaataagggcggcgatcagggaccccccctgatgacagatggcggaggaggacacagccatgatagcggacatggcggaggcgatccccatctgcctaccctcctcctgggcagctccggttctggaggcgacgatgatgaccctcacggccctgtgcagctctcctactacgacggcaaaaggaccgaacaaggaaaagaggtcctggagaaggccaggggcagcacatacggaacccccaggcctcccatgtccgattggaccggaggagccctgctggtcctctacagcttcgccctgatgctgatcattatcatcctgatcatctttatcttcagaagggacctgctgtgccctctcggcgccctgtgcatcctgctgctcatgatcacactcctcctgatcgccctctggaacctgcacggacaagccctgatgtccgatgagggacctggaacaggacccggaaacggactgggcgagaagggagatacaagcggccccgaaggcagcggcggaagcggaccccaaagaaggggcggcgacaaccacggaagaggaagaggcaggggcagaggcagaggaggaggaagacctggagcccctggcggttctggaagcggacccaggcacagggacggagtgaggaggcctcaaaaaagacccagctgcatcggctgcaagggaacccactggattgatgataacccctccacagagaccgctcaggcctggaacgccggcttcctgaggggaagagcctatggcatcgatctgctgaggaccgagggcgaacacgtggagggagccaccggagagacaagggaggaaagcgaagacacagaaagcgatggcgacgacgaagacctgccctgcattgtgtccaggggcggacccaaggtgaagaggccccctatctttatcagaaggctccatagactgctcctgatgagggccatgaaccctgtgtgcctgcccgtgatcgtggccccctacctcttttggctggccgccattgccgctagctgcttcaccgcctccgtgtccacagtggtgacagccaccggcctcgccctgagcctgctgctcctcgctgccgtggcctccagctacgccgctgctcaaagaaagctcctgacccctgtcaccgtcctgacagccgtcgtgaccaccttttccgctggcaccttcaagctgcctaggtgcacacctggcgacaggcagtggctctacgtgcagagctccgtgggcaatattgtgcagagctgcaatcccaggtacagcatttttttcgactacatggccatccataggtccctcaccaagatctgggaggatctgggaggcccttcccaggctcctctgccctgcgtgctgtggcctgtgctgcctgagcctctgccccaaggccagctgacagcctatcacgtgtccaccgctcctacaggttcttggttcagcgctccccagcccgctcccgaaaacgcttaccaggcttacgccgccccccagctgttccccgtctccgacatctgatgatgagcggccgcgatctgctgtgccttctagttgccagccatctgttgtttgcccctcccccgtgccttccttgaccctggaaggtgccactcccactgtcctttcctaataaaatgaggaaattgcatcgcattgtctgagtaggtgtcattctattctggggggtggggtggggcaggacagcaagggggaggattgggaagacaatagcaggcatgctggggatgcggtgggctctatggccgatcagcgatcgctgaggtgggtgagtgggcgtggcctggggtggtcatgaaaatatataagttgggggtcttagggtctctttatttgtgttgcagagaccgccggagccatgagcgggagcagcagcagcagcagtagcagcagcgccttggatggcagcatcgtgagcccttatttgacgacgcggatgccccactgggccggggtgcgtcagaatgtgatgggctccagcatcgacggccgacccgtcctgcccgcaaattccgccacgctgacctatgcgaccgtcgcggggacgccgttggacgccaccgccgccgccgccgccaccgcagccgcctcggccgtgcgcagcctggccacggactttgcattcctgggaccactggcgacaggggctacttctcgggccgctgctgccgccgttcgcgatgacaagctgaccgccctgctggcgcagttggatgcgcttactcgggaactgggtgacctttctcagcaggtcatggccctgcgccagcaggtctcctccctgcaagctggcgggaatgcttctcccacaaatgccgtttaagataaataaaaccagactctgtttggattaaagaaaagtagcaagtgcattgctctctttatttcataattttccgcgcgcgataggccctagaccagcgttctcggtcgttgagggtgcggtgtatcttctccaggacgtggtagaggtggctctggacgttgagatacatgggcatgagcccgtcccgggggtggaggtagcaccactgcagagcttcatgctccggggtggtgttgtagatgatccagtcgtagcaggagcgctgggcatggtgcctaaaaatgtccttcagcagcaggccgatggccagggggaggcccttggtgtaagtgtttacaaaacggttaagttgggaagggtgcattcggggagagatgatgtgcatcttggactgtatttttagattggcgatgtttccgcccagatcccttctgggattcatgttgtgcaggaccaccagtacagtgtatccggtgcacttggggaatttgtcatgcagcttagagggaaaagcgtggaagaacttggagacgcctttgtggcctcccagattttccatgcattcgtccatgatgatggcaatgggcccgcgggaggcagcttgggcaaagatatttctggggtcgctgacgtcgtagttgtgttccagggtgaggtcgtcataggccatttttacaaagcgcgggcggagggtgcccgactgggggatgatggtcccctctggccctggggcgtagttgccctcgcagatctgcatttcccaggccttaatctcggaggggggaatcatatccacctgcggggcgatgaagaaaacggtttccggagccggggagattaactgggatgagagcaggtttctaagcagctgtgattttccacaaccggtgggcccataaataacacctataaccggttgcagctggtagtttagagagctgcagctgccgtcgtcccggaggaggggggccacctcgttgagcatgtccctgacgcgcatgttctccccgaccagatccgccagaaggcgctcgccgcccagggacagcagctcttgcaaggaagcaaagtttttcagcggcttgaggccgtccgccgtgggcatgtttttcagggtctggctcagcagctccaggcggtcccagagctcggtgacgtgctctacggcatctctatccagcatatctcctcgtttcgcgggttggggcgactttcgctgtagggcaccaagcggtggtcgtccagcggggccagagtcatgtccttccatgggcgcagggtcctcgtcagggtggtctgggtcacggtgaaggggtgcgctccgggctgagcgcttgccaaggtgcgcttgaggctggttctgctggtgctgaagcgctgccggtcttcgccctgcgcgtcggccaggtagcatttgaccatggtgtcatagtccagcccctccgcggcgtgtcccttggcgcgcagcttgcccttggaggtggcgccgcacgaggggcagagcaggctcttgagcgcgtagagcttgggggcgaggaagaccgattcgggggagtaggcgtccgcgccgcagaccccgcacacggtctcgcactccaccagccaggtgagctcggggcgcgccgggtcaaaaaccaggtttcccccatgctttttgatgcgtttcttacctcgggtctccatgaggtggtgtccccgctcggtgacgaagaggctgtccgtgtctccgtagaccgacttgaggggtcttttctccaggggggtccctcggtcttcctcgtagaggaactcggaccactctgagacgaaggcccgcgtccaggccaggacgaaggaggctatgtgggaggggtagcggtcgttgtccactagggggtccaccttctccaaggtgtgaagacacatgtcgccttcctcggcgtccaggaaggtgattggcttgtaggtgtaggccacgtgaccgggggttcctgacgggggggtataaaagggggtgggggcgcgctcgtcgtcactctcttccgcatcgctgtctgcgagggccagctgctggggtgagtattccctctcgaaggcgggcatgacctccgcgctgaggttgtcagtttccaaaaacgaggaggatttgatgttcacctgtcccgaggtgatacctttgagggtacccgcgtccatctggtcagaaaacacgatctttttattgtccagcttggtggcgaacgacccgtagagggcgttggagagcagcttggcgatggagcgcagggtctggttcttgtccctgtcggcgcgctccttggccgcgatgttgagctgcacgtactcgcgcgcgacgcagcgccactcggggaagacggtggtgcgctcgtcgggcaccaggcgcacgcgccagccgcggttgtgcagggtgaccaggtccacgctggtggcgacctcgccgcgcaggcgctcgttggtccagcagagacggccgcccttgcgcgagcagaaggggggcagggggtcgagctgggtctcgtccggggggtccgcgtccacggtgaaaaccccggggcgcaggcgcgcgtcgaagtagtctatcttgcaaccttgcatgtccagcgcctgctgccagtcgcgggcggcgagcgcgcgctcgtaggggttgagcggcgggccccagggcatggggtgggtgagtgcggaggcgtacatgccgcagatgtcatagacgtagaggggctcccgcaggaccccgatgtaggtggggtagcagcggccgccgcggatgctggcgcgcacgtagtcatacagctcgtgcgagggggcgaggaggtcggggcccaggttggtgcgggcggggcgctccgcgcggaagacgatctgcctgaagatggcatgcgagttggaagagatggtggggcgctggaagacgttgaagctggcgtcctgcaggccgacggcgtcgcgcacgaaggaggcgtaggagtcgcgcagcttgtgtaccagctcggcggtgacctgcacgtcgagcgcgcagtagtcgagggtctcgcggatgatgtcatatttagcctgccccttctttttccacagctcgcggttgaggacaaactcttcgcggtctttccagtactcttggatcgggaaaccgtccggttccgaacggtaagagcctagcatgtagaactggttgacggcctggtaggcgcagcagcccttctccacggggagggcgtaggcctgcgcggccttgcggagcgaggtgtgggtcagggcgaaggtgtccctgaccatgactttgaggtactggtgcttgaagtcggagtcgtcgcagccgccccgctcccagagcgagaagtcggtgcgcttcttggagcgggggttgggcagagcgaaggtgacatcgttgaagaggattttgcccgcgcggggcatgaagttgcgggtgatgcggaagggccccggcacttcagagcggttgttgatgacctgggcggcgagcacgatctcgtcgaagccgttgatgttgtggcccacgatgtagagttccaggaagcggggccggccctttacggtgggcagcttctttagctcttcgtaggtgagctcctcgggcgaggcgaggccgtgctcggccagggcccagtccgcgaggtgcgggttgtctctgaggaaggacttccagaggtcgcgggccaggagggtctgcaggcggtctctgaaggtcctgaactggcggcccacggccattttttcgggggtgatgcagtagaaggtgagggggtcttgctgccagcggtcccagtcgagctgcagggcgaggtcgcgcgcggcggtgaccaggcgctcgtcgcccccgaatttcatgaccagcatgaagggcacgagctgctttccgaaggcccccatccaagtgtaggtctctacatcgtaggtgacaaagaggcgctccgtgcgaggatgcgagccgatcgggaagaactggatctcccgccaccagttggaggagtggctgttgatgtggtggaagtagaagtcccgtcgccgggccgaacactcgtgctggcttttgtaaaagcgagcgcagtactggcagcgctgcacgggctgtacctcatgcacgagatgcacctttcgcccgcgcacgaggaagccgaggggaaatctgagccccccgcctggctcgcggcatggctggttctcttctactttggatgcgtgtccgtctccgtctggctcctcgaggggtgttacggtggagcggaccaccacgccgcgcgagccgcaggtccagatatcggcgcgcggcggtcggagtttgatgacgacatcgcgcagctgggagctgtccatggtctggagctcccgcggcggcggcaggtcagccgggagttcttgcaggttcacctcgcagagtcgggccagggcgcggggcaggtctaggtggtacctgatctctaggggcgtgttggtggcggcgtcgatggcttgcaggagcccgcagccccggggggcgacgacggtgccccgcggggtggtggtggtggtggcggtgcagctcagaagcggtgccgcgggcgggcccccggaggtagggggggctccggtcccgcgggcaggggcggcagcggcacgtcggcgtggagcgcgggcaggagttggtgctgtgcccggaggttgctggcgaaggcgacgacgcggcggttgatctcctggatctggcgcctctgcgtgaagacgacgggcccggtgagcttgaacctgaaagagagttcgacagaatcaatctcggtgtcattgaccgcggcctggcgcaggatctcctgcacgtctcccgagttgtcttggtaggcgatctcggccatgaactgctcgatctcttcctcctggaggtctccgcgtccggcgcgttccacggtggccgccaggtcgttggagatgcgccccatgagctgcgagaaggcgttgagtccgccctcgttccagactcggctgtagaccacgcccccctggtcatcgcgggcgcgcatgaccacctgcgcgaggttgagctccacgtgccgcgcgaagacggcgtagttgcgcagacgctggaagaggtagttgagggtggtggcggtgtgctcggccacgaagaagttcatgacccagcggcgcaacgtggattcgttgatgtcccccaaggcctccagccgttccatggcctcgtagaagtccacggcgaagttgaaaaactgggagttgcgcgccgacacggtcaactcctcctccagaagacggatgagctcggcgacggtgtcgcgcacctcgcgctcgaaggctatggggatctcttcctccgctagcatcaccacctcctcctcttcctcctcttctggcacttccatgatggcttcctcctcttcggggggtggcggcggcggcggtgggggagggggcgctctgcgccggcggcggcgcaccgggaggcggtccacgaagcgcgcgatcatctccccgcggcggcggcgcatggtctcggtgacggcgcggccgttctcccgggggcgcagttggaagacgccgccggacatctggtgctggggcgggtggccgtgaggcagcgagacggcgctgacgatgcatctcaacaattgctgcgtaggtacgccgccgagggacctgagggagtccatatccaccggatccgaaaacctttcgaggaaggcgtctaaccagtcgcagtcgcaaggtaggctgagcaccgtggcgggcggcggggggtggggggagtgtctggcggaggtgctgctgatgatgtaattgaagtaggcggacttgacacggcggatggtcgacaggagcaccatgtccttgggtccggcctgctggatgcggaggcggtcggctatgccccaggcttcgttctggcatcggcgcaggtccttgtagtagtcttgcatgagcctttccaccggcacctcttctccttcctcttctgcttcttccatgtctgcttcggccctggggcggcgccgcgcccccctgccccccatgcgcgtgaccccgaaccccctgagcggttggagcagggccaggtcggcgacgacgcgctcggccaggatggcctgctgcacctgcgtgagggtggtttggaagtcatccaagtccacgaagcggtggtaggcgcccgtgttgatggtgtaggtgcagttggccatgacggaccagttgacggtctggtggcccggttgcgacatctcggtgtacctgagtcgcgagtaggcgcgggagtcgaagacgtagtcgttgcaagtccgcaccaggtactggtagcccaccaggaagtgcggcggcggctggcggtagaggggccagcgcagggtggcgggggctccgggggccaggtcttccagcatgaggcggtggtaggcgtagatgtacctggacatccaggtgatacccgcggcggtggtggaggcgcgcgggaagtcgcgcacccggttccagatgttgcgcaggggcagaaagtgctccatggtaggcgtgctctgtccagtcagacgcgcgcagtcgttgatactctagaccagggaaaacgaaagccggtcagcgggcactcttccgtggtctggtgaatagatcgcaagggtatcatggcggagggcctcggttcgagccccgggtccgggccggacggtccgccatgatccacgcggttaccgcccgcgtgtcgaacccaggtgtgcgacgtcagacaacggtggagtgttccttttggcgtttttctggccgggcgccggcgccgcgtaagagactaagccgcgaaagcgaaagcagtaagtggctcgctccccgtagccggagggatccttgctaagggttgcgttgcggcgaaccccggttcgaatcccgtactcgggccggccggacccgcggctaaggtgttggattggcctccccctcgtataaagaccccgcttgcggattgactccggacacggggacgagccccttttatttttgctttccccagatgcatccggtgctgcggcagatgcgccccccgccccagcagcagcaacaacaccagcaagagcggcagcaacagcagcgggagtcatgcagggccccctcacccaccctcggcgggccggccacctcggcgtccgcggccgtgtctggcgcctgcggcggcggcggggggccggctgacgaccccgaggagcccccgcggcgcagggccagacactacctggacctggaggagggcgagggcctggcgcggctgggggcgccgtctcccgagcgccacccgcgggtgcagctgaagcgcgactcgcgcgaggcgtacgtgcctcggcagaacctgttcagggaccgcgcgggcgaggagcccgaggagatgcgggacaggaggttcagcgcagggcgggagctgcggcaggggctgaaccgcgagcggctgctgcgcgaggaggactttgagcccgacgcgcggacggggatcagccccgcgcgcgcgcacgtggcggccgccgacctggtgacggcgtacgagcagacggtgaaccaggagatcaacttccaaaagagtttcaacaaccacgtgcgcacgctggtggcgcgcgaggaggtgaccatcgggctgatgcacctgtgggactttgtaagcgcgctggtgcagaaccccaacagcaagcctctgacggcgcagctgttcctgatagtgcagcacagcagggacaacgaggcgtttagggacgcgctgctgaacatcaccgagcccgagggtcggtggctgctggacctgattaacatcctgcagagcatagtggtgcaggagcgcagcctgagcctggccgacaaggtggcggccatcaactactcgatgctgagcctgggcaagttttacgcgcgcaagatctaccagacgccgtacgtgcccatagacaaggaggtgaagatcgacggtttttacatgcgcatggcgctgaaggtgctcaccctgagcgacgacctgggcgtgtaccgcaacgagcgcatccacaaggccgtgagcgtgagccggcggcgcgagctgagcgaccgcgagctgatgcacagcctgcagcgggcgctggcgggcgccggcagcggcgacagggaggcggagtcctacttcgatgcgggggcggacctgcgctgggcgcccagccggcgggccctggaggccgcgggggtccgcgaggactatgacgaggacggcgaggaggatgaggagtacgagctagaggagggcgagtacctggactaaaccgcgggtggtgtttccggtagatgcaagacccgaacgtggtggacccggcgctgcgggcggctctgcagagccagccgtccggccttaactcctcagacgactggcgacaggtcatggaccgcatcatgtcgctgacggcgcgtaacccggacgcgttccggcagcagccgcaggccaacaggctctccgccatcctggaggcggtggtgcctgcgcgctcgaaccccacgcacgagaaggtgctggccatagtgaacgcgctggccgagaacagggccatccgcccggacgaggccgggctggtgtacgacgcgctgctgcagcgcgtggcccgctacaacagcggcaacgtgcagaccaacctggaccggctggtgggggacgtgcgcgaggcggtggcgcagcgcgagcgcgcggatcggcagggcaacctgggctccatggtggcgctgaatgccttcctgagcacgcagccggccaacgtgccgcgggggcaggaagactacaccaactttgtgagcgcgctgcggctgatggtgaccgagaccccccagagcgaggtgtaccagtcgggcccggactacttcttccagaccagcagacagggcctgcagacggtgaacctgagccaggctttcaagaacctgcgggggctgtggggcgtgaaggcgcccaccggcgaccgggcgacggtgtccagcctgctgacgcccaactcgcgcctgctgctgctgctgatcgcgccgttcacggacagcggcagcgtgtcccgggacacctacctggggcacctgctgaccctgtaccgcgaggccatcgggcaggcgcaggtggacgagcacaccttccaggagatcaccagcgtgagccgcgcgctggggcaggaggacacgagcagcctggaggcgactctgaactacctgctgaccaaccggcggcagaagattccctcgctgcacagcctgacctccgaggaggagcgcatcttgcgctacgtgcagcagagcgtgagcctgaacctgatgcgcgacggggtgacgcccagcgtggcgctggacatgaccgcgcgcaacatggaaccgggcatgtacgccgcgcaccggccttacatcaaccgcctgatggactacctgcatcgcgcggcggccgtgaaccccgagtactttaccaacgccatcctgaacccgcactggctcccgccgcccgggttctacagcgggggcttcgaggtcccggagaccaacgatggcttcctgtgggacgacatggacgacagcgtgttctccccgcggccgcaggcgctggcggaagcgtccctgctgcgtcccaagaaggaggaggaggaggaggcgagtcgccgccgcggcagcagcggcgtggcttctctgtccgagctgggggcggcagccgccgcgcgccccgggtccctgggcggcagcccctttccgagcctggtggggtctctgcacagcgagcgcaccacccgccctcggctgctgggcgaggacgagtacctgaataactccctgctgcagccggtgcgggagaaaaacctgcctcccgccttccccaacaacgggatagagagcctggtggacaagatgagcagatggaagacctatgcgcaggagcacagggacgcgcctgcgctccggccgcccacgcggcgccagcgccacgaccggcagcgggggctggtgtgggatgacgaggactccgcggacgatagcagcgtgctggacctgggagggagcggcaacccgttcgcgcacctgcgcccccgcctggggaggatgttttaaaaaaaaaaaaaaaangcaagaagcatgatgcaaaaattaaataaaactcaccaaggccatggcgaccgagcgttggtttcttgtgttcccttcagtatgcggcgcgcggcgatgtaccaggagggacctcctccctcttacgagagcgtggtgggcgcggcggcggcggcgccctcttctccctttgcgtcgcagctgctggagccgccgtacgtgcctccgcgctacctgcggcctacgggggggagaaacagcatccgttactcggagctggcgcccctgttcgacaccacccgggtgtacctggtggacaacaagtcggcggacgtggcctccctgaactaccagaacgaccacagcaattttttgaccacggtcatccagaacaatgactacagcccgagcgaggccagcacccagaccatcaatctggatgaccggtcgcactggggcggcgacctgaaaaccatcctgcacaccaacatgcccaacgtgaacgagttcatgttcaccaataagttcaaggcgcgggtgatggtgtcgcgctcgcacaccaaggaagaccgggtggagctgaagtacgagtgggtggagttcgagctgccagagggcaactactccgagaccatgaccattgacctgatgaacaacgcgatcgtggagcactatctgaaagtgggcaggcagaacggggtcctggagagcgacatcggggtcaagttcgacaccaggaacttccgcctggggctggaccccgtgaccgggctggttatgcccggggtgtacaccaacgaggccttccatcccgacatcatcctgctgcccggctgcggggtggacttcacttacagccgcctgagcaacctcctgggcatccgcaagcggcagcccttccaggagggcttcaggatcacctacgaggacctggaggggggcaacatccccgcgctcctcgatgtggaggcctaccaggatagcttgaaggaaaatgaggcgggacaggaggataccgcccccgccgcctccgccgccgccgagcagggcgaggatgctgctgacaccgcggccgcggacggggcagaggccgaccccgctatggtggtggaggctcccgagcaggaggaggacatgaatgacagtgcggtgcgcggagacaccttcgtcacccggggggaggaaaagcaagcggaggccgaggccgcggccgaggaaaagcaactggcggcagcagcggcggcggcggcgttggccgcggcggaggctgagtctgaggggaccaagcccgccaaggagcccgtgattaagcccctgaccgaagatagcaagaagcgcagttacaacctgctcaaggacagcaccaacaccgcgtaccgcagctggtacctggcctacaactacggcgacccgtcgacgggggtgcgctcctggaccctgctgtgcacgccggacgtgacctgcggctcggagcaggtgtactggtcgctgcccgacatgatgcaagaccccgtgaccttccgctccacgcggcaggtcagcaacttcccggtggtgggcgccgagctgctgcccgtgcactccaagagcttctacaacgaccaggccgtctactcccagctcatccgccagttcacctctctgacccacgtgttcaatcgctttcctgagaaccagattctggcgcgcccgcccgcccccaccatcaccaccgtcagtgaaaacgttcctgctctcacagatcacgggacgctaccgctgcgcaacagcatcggaggagtccagcgagtgaccgttactgacgccagacgccgcacctgcccctacgtttacaaggccttgggcatagtctcgccgcgcgtcctttccagccgcactttttgagcaacaccaccatcatgtccatcctgatctcacccagcaataactccggctggggactgctgcgcgcgcccagcaagatgttcggaggggcgaggaagcgttccgagcagcaccccgtgcgcgtgcgcgggcacttccgcgccccctggggagcgcacaaacgcggccgcgcggggcgcaccaccgtggacgacgccatcgactcggtggtggagcaggcgcgcaactacaggcccgcggtctctaccgtggacgcggccatccagaccgtggtgcggggcgcgcggcggtacgccaagctgaagagccgccggaagcgcgtggcccgccgccaccgccgccgacccggggccgccgccaaacgcgccgccgcggccctgcttcgccgggccaagcgcacgggccgccgcgccgccatgagggccgcgcgccgcttggccgccggcatcaccgccgccaccatggccccccgtacccgaagacgcgcggccgccgccgccgccgccgccatcagtgacatggccagcaggcgccggggcaacgtgtactgggtgcgcgactcggtgaccggcacgcgcgtgcccgtgcgcttccgccccccgcggacttgagatgatgtgaaaaaacaacactgagtctcctgctgttgtgtgtatcccagcggcggcggcgcgcgcagcgtcatgtccaagcgcaaaatcaaagaagagatgctccaggtcgtcgcgccggagatctatgggcccccgaagaaggaagagcaggattcgaagccccgcaagataaagcgggtcaaaaagaaaaagaaagatgatgacgatgccgatggggaggtggagttcctgcgcgccacggcgcccaggcgcccggtgcagtggaagggccggcgcgtaaagcgcgtcctgcgccccggcaccgcggtggtcttcacgcccggcgagcgctccacccggactttcaagcgcgtctatgacgaggtgtacggcgacgaagacctgctggagcaggccaacgagcgcttcggagagtttgcttacgggaagcgtcagcgggcgctggggaaggaggacctgctggcgctgccgctggaccagggcaaccccacccccagtctgaagcccgtgaccctgcagcaggtgctgccgagcagcgcaccctccgaggcgaagcggggtctgaagcgcgagggcggcgacctggcgcccaccgtgcagctcatggtgcccaagcggcagaggctggaggatgtgctggagaaaatgaaagtagaccccggtctgcagccggacatcagggtccgccccatcaagcaggtggcgccgggcctcggcgtgcagaccgtggacgtggtcatccccaccggcaactcccccgccgccgccaccactaccgctgcctccacggacatggagacacagaccgatcccgccgcagccgcagccgcagccgccgccgcgacctcctcggcggaggtgcagacggacccctggctgccgccggcgatgtcagctccccgcgcgcgtcgcgggcgcaggaagtacggcgccgccaacgcgctcctgcccgagtacgccttgcatccttccatcgcgcccacccccggctaccgaggctatacctaccgcccgcgaagagccaagggttccacccgccgtccccgccgacgcgccgccgccaccacccgccgccgccgccgcagacgccagcccgcactggctccagtctccgtgaggaaagtggcgcgcgacggacacaccctggtgctgcccagggcgcgctaccaccccagcatcgtttaaaagcctgttgtggttcttgcagatatggccctcacttgccgcctccgtttcccggtgccgggataccgaggaggaagatcgcgccgcaggaggggtctggccggccgcggcctgagcggaggcagccgccgcgcgcaccggcggcgacgcgccaccagccgacgcatgcgcggcggggtgctgcccctgttaatccccctgatcgccgcggcgatcggcgccgtgcccgggatcgcctccgtggccttgcaagcgtcccagaggcattgacagacttgcaaacttgcaaatatggaaaaaaaaaccccaataaaaaagtctagactctcacgctcgcttggtcctgtgactattttgtagaatggaagacatcaactttgcgtcgctggccccgcgtcacggctcgcgcccgttcctgggacactggaacgatatcggcaccagcaacatgagcggtggcgccttcagttggggctctctgtggagcggcattaaaagtatcgggtctgccgttaaaaattacggctcccgggcctggaacagcagcacgggccagatgttgagagacaagttgaaagagcagaacttccagcagaaggtggtggagggcctggcctccggcatcaacggggtggtggacctggccaaccaggccgtgcagaataagatcaacagcagactggacccccggccgccggtggaggaggtgccgccggcgctggagacggtgtcccccgatgggcgtggcgagaagcgcccgcggcccgatagggaagagaccactctggtcacgcagaccgatgagccgcccccgtatgaggaggccctgaagcaaggtctgcccaccacgcggcccatcgcgcccatggccaccggggtggtgggccgccacacccccgccacgctggacttgcctccgcccgccgatgtgccgcagcagcagaaggcggcacagccgggcccgcccgcgaccgcctcccgttcctccgccggtcctctgcgccgcgcggccagcggcccccgcgggggggtcgcgaggcacggcaactggcagagcacgctgaacagcatcgtgggtctgggggtgcggtccgtgaagcgccgccgatgctactgaatagcttagctaacgtgttgtatgtgtgtatgcgccctatgtcgccgccagaggagctgctgagtcgccgccgttcgcgcgcccaccaccaccgccactccgcccctcaagatggcgaccccatcgatgatgccgcagtggtcgtacatgcacatctcgggccaggacgcctcggagtacctgagccccgggctggtgcagttcgcccgcgccaccgagagctacttcagcctgagtaacaagtttaggaaccccacggtggcgcccacgcacgatgtgaccaccgaccggtctcagcgcctgacgctgcggttcattcccgtggaccgcgaggacaccgcgtactcgtacaaggcgcggttcaccctggccgtgggcgacaaccgcgtgctggacatggcctccacctactttgacatccgcggggtgctggaccggggtcccactttcaagccctactctggcaccgcctacaactccctggcccccaagggcgctcccaactcctgcgagtgggagcaagaggaaactcaggcagttgaagaagcagcagaagaggaagaagaagatgctgacggtcaagctgaggaagagcaagcagctaccaaaaagactcatgtatatgctcaggctcccctttctggcgaaaaaattagtaaagatggtctgcaaataggaacggacgctacagctacagaacaaaaacctatttatgcagaccctacattccagcccgaaccccaaatcggggagtcccagtggaatgaggcagatgctacagtcgccggcggtagagtgctaaagaaatctactcccatgaaaccatgctatggttcctatgcaagacccacaaatgctaatggaggtcagggtgtactaacggcaaatgcccagggacagctagaatctcaggttgaaatgcaattcttttcaacttctgaaaacgcccgtaacgaggctaacaacattcagcccaaattggtgctgtatagtgaggatgtgcacatggagaccccggatacgcacctttcttacaagcccgcaaaaagcgatgacaattcaaaaatcatgctgggtcagcagtccatgcccaacagacctaattacatcggcttcagagacaactttatcggcctcatgtattacaatagcactggcaacatgggagtgcttgcaggtcaggcctctcagttgaatgcagtggtggacttgcaagacagaaacacagaactgtcctaccagctcttgcttgattccatgggtgacagaaccagatacttttccatgtggaatcaggcagtggacagttatgacccagatgttagaattattgaaaatcatggaactgaagacgagctccccaactattgtttccctctgggtggcataggggtaactgacacttaccaggctgttaaaaccaacaatggcaataacgggggccaggtgacttggacaaaagatgaaacttttgcagatcgcaatgaaataggggtgggaaacaatttcgctatggagatcaacctcagtgccaacctgtggagaaacttcctgtactccaacgtggcgctgtacctaccagacaagcttaagtacaacccctccaatgtggacatctctgacaaccccaacacctacgattacatgaacaagcgagtggtggccccggggctggtggactgctacatcaacctgggcgcgcgctggtcgctggactacatggacaacgtcaaccccttcaaccaccaccgcaatgcgggcctgcgctaccgctccatgctcctgggcaacgggcgctacgtgcccttccacatccaggtgccccagaagttctttgccatcaagaacctcctcctcctgccgggctcctacacctacgagtggaacttcaggaaggatgtcaacatggtcctccagagctctctgggtaacgatctcagggtggacggggccagcatcaagttcgagagcatctgcctctacgccaccttcttccccatggcccacaacacggcctccacgctcgaggccatgctcaggaacgacaccaacgaccagtccttcaatgactacctctccgccgccaacatgctctaccccatacccgccaacgccaccaacgtccccatctccatcccctcgcgcaactgggcggccttccgcggctgggccttcacccgcctcaagaccaaggagaccccctccctgggctcgggattcgacccctactacacctactcgggctccattccctacctggacggcaccttctacctcaaccacactttcaagaaggtctcggtcaccttcgactcctcggtcagctggccgggcaacgaccgtctgctcacccccaacgagttcgagatcaagcgctcggtcgacggggagggctacaacgtggcccagtgcaacatgaccaaggactggttcctggtccagatgctggccaactacaacatcggctaccagggcttctacatcccagagagctacaaggacaggatgtactccttcttcaggaacttccagcccatgagccggcaggtggtggaccagaccaagtacaaggactaccaggaggtgggcatcatccaccagcacaacaactcgggcttcgtgggctacctcgcccccaccatgcgcgagggacaggcctaccccgccaacttcccctatccgctcataggcaagaccgcggtcgacagcatcacccagaaaaagttcctctgcgaccgcaccctctggcgcatccccttctccagcaacttcatgtccatgggtgcgctctcggacctgggccagaacttgctctacgccaactccgcccacgccctcgacatgaccttcgaggtcgaccccatggacgagcccacccttctctatgttctgttcgaagtctttgacgtggtccgggtccaccagccgcaccgcggcgtcatcgagaccgtgtacctgcgtacgcccttctcggccggcaacgccaccacctaaagaagcaagccgcagtcatcgccgcctgcatgccgtcgggttccaccgagcaagagctcagggccatcgtcagagacctgggatgcgggccctattttttgggcaccttcgacaagcgcttccctggctttgtctccccacacaagctggcctgcgccatcgtcaacacggccggccgcgagaccgggggcgtgcactggctggccttcgcctggaacccgcgctccaaaacatgcttcctctttgaccccttcggcttttcggaccagcggctcaagcaaatctacgagttcgagtacgagggcttgctgcgtcgcagcgccatcgcctcctcgcccgaccgctgcgtcaccctcgaaaagtccacccagaccgtgcaggggcccgactcggccgcctgcggtctcttctgctgcatgtttctgcacgcctttgtgcactggcctcagagtcccatggaccgcaaccccaccatgaacttgctgacgggggtgcccaactccatgctccagagcccccaggtcgagcccaccctgcgccgcaaccaggagcagctctacagcttcctggagcgccactcgccttacttccgccgccacagcgcacagatcaggagggccacctccttctgccacttgcaagagatgcaagaagggtaataacgatgtacacactttttttctcaataaatggcatctttttatttatacaagctctctggggtattcatttcccaccaccacccgccgttgtcgccatctggctctatttagaaatcgaaagggttctgccgggagtcgccgtgcgccacgggcagggacacgttgcgatactggtagcgggtgccccacttgaactcgggcaccaccaggcgaggcagctcggggaagttttcgctccacaggctgcgggtcagcaccagcgcgttcatcaggtcgggcgccgagatcttgaagtcgcagttggggccgccgccctgcgcgcgcgagttgcggtacaccgggttgcagcactggaacaccaacagcgccgggtgcttcacgctggccagcacgctgcggtcggagatcagctcggcgtccaggtcctccgcgttgctcagcgcgaacggggtcatcttgggcacttgccgccccaggaagggcgcgtgccccggtttcgagttgcagtcgcagcgcagcgggatcagcaggtgcccgtgcccggactcggcgttggggtacagcgcgcgcatgaaggcctgcatctggcggaaggccatctgggccttggcgccctccgagaagaacatgccgcaggacttgcccgagaactggtttgcggggcagctggcgtcgtgcaggcagcagcgcgcgtcggtgttggcgatctgcaccacgttgcgcccccaccggttcttcacgatcttggccttggacgattgctccttcagcgcgcgctgcccgttctcgctggtcacatccatctcgatcacatgttccttgttcaccatgctgctgccgtgcagacacttcagctcgccctccgtctcggtgcagcggtgctgccacagcgcgcagcccgtgggctcgaaagacttgtaggtcacctccgcgaaggactgcaggtacccctgcaaaaagcggcccatcatggtcacgaaggtcttgttgctgctgaaggtcagctgcagcccgcggtgctcctcgttcagccaggtcttgcacacggccgccagcgcctccacctggtcgggcagcatcttgaagttcaccttcagctcattctccacgtggtacttgtccatcagcgtgcgcgccgcctccatgcccttctcccaggccgacaccagcggcaggctcacggggttcttcaccatcaccgtggccgccgcctccgccgcgctttcgctttccgccccgctgttctcttcctcttcctcctcttcctcgccgccgcccactcgcagcccccgcaccacggggtcgtcttcctgcaggcgctgcaccttgcgcttgccgttgcgcccctgcttgatgcgcacgggcgggttgctgaagcccaccatcaccagcgcggcctcttcttgctcgtcctcgctgtccagaatgacctccggggagggggggttggtcatcctcagtaccgaggcacgcttctttttcttcctgggggcgttcgccagctccgcggctgcggccgctgccgaggtcgaaggccgagggctgggcgtgcgcggcaccagcgcgtcctgcgagccgtcctcgtcctcctcggactcgagacggaggcgggcccgcttcttcgggggcgcgcggggcggcggaggcggcggcggcgacggagacggggacgagacatcgtccagggtgggtggacggcgggccgcgccgcgtccgcgctcgggggtggtctcgcgctggtcctcttcccgactggccatctcccactgctccttctcctataggcagaaagagatcatggagtctctcatgcgagtcgagaaggaggaggacagcctaaccgccccctctgagccctccaccaccgccgccaccaccgccaatgccgccgcggacgacgcgcccaccgagaccaccgccagtaccaccctccccagcgacgcacccccgctcgagaatgaagtgctgatcgagcaggacccgggttttgtgagcggagaggaggatgaggtggatgagaaggagaaggaggaggtcgccgcctcagtgccaaaagaggataaaaagcaagaccaggacgacgcagataaggatgagacagcagtcgggcgggggaacggaagccatgatgctgatgacggctacctagacgtgggagacgacgtgctgcttaagcacctgcaccgccagtgcgtcatcgtctgcgacgcgctgcaggagcgctgcgaagtgcccctggacgtggcggaggtcagccgcgcctacgagcggcacctcttcgcgccgcacgtgccccccaagcgccgggagaacggcacctgcgagcccaacccgcgtctcaacttctacccggtcttcgcggtacccgaggtgctggccacctaccacatctttttccaaaactgcaagatccccctctcctgccgcgccaaccgcacccgcgccgacaaaaccctgaccctgcggcagggcgcccacatacctgatatcgcctctctggaggaagtgcccaagatcttcgagggtctcggtcgcgacgagaaacgggcggcgaacgctctgcacggagacagcgaaaacgagagtcactcgggggtgctggtggagctcgagggcgacaacgcgcgcctggccgtactcaagcgcagcatagaggtcacccactttgcctacccggcgctcaacctgccccccaaggtcatgagtgtggtcatgggcgagctcatcatgcgccgcgcccagcccctggccgcggatgcaaacttgcaagagtcctccgaggaaggcctgcccgcggtcagcgacgagcagctggcgcgctggctggagacccgcgaccccgcgcagctggaggagcggcgcaagctcatgatggccgcggtgctggtcaccgtggagctcgagtgtctgcagcgcttcttcgcggaccccgagatgcagcgcaagctcgaggagaccctgcactacaccttccgccagggctacgtgcgccaggcctgcaagatctccaacgtggagctctgcaacctggtctcctacctgggcatcctgcacgagaaccgcctcgggcagaacgtcctgcactccaccctcaaaggggaggcgcgccgcgactacatccgcgactgcgcctacctcttcctctgctacacctggcagacggccatgggggtctggcagcagtgcctggaggagcgcaacctcaaggagctggaaaagctcctcaagcgcaccctcagggacctctggacgggcttcaacgagcgctcggtggccgccgcgctggcggacatcatctttcccgagcgcctgctcaagaccctgcagcagggcctgcccgacttcaccagccagagcatgctgcagaacttcaggactttcatcctggagcgctcgggcatcctgccggccacttgctgcgcgctgcccagcgacttcgtgcccatcaagtacagggagtgcccgccgccgctctggggccactgctacctcttccagctggccaactacctcgcctaccactcggacctcatggaagacgtgagcggcgagggcctgctcgagtgccactgccgctgcaacctctgcacgccccaccgctctctagtctgcaacccgcagctgctcagcgagagtcagattatcggtaccttcgagctgcagggtccctcgcctgacgagaagtccgcggctccagggctgaaactcactccggggctgtggacttccgcctacctacgcaaatttgtacctgaggactaccacgcccacgagatcaggttctacgaagaccaatcccgcccgcccaaggcggagctcaccgcctgcgtcatcacccaggggcacatcctgggccaattgcaagccatcaacaaagcccgccgagagttcttgctgaaaaagggtcggggggtgtacctggacccccagtccggcgaggagctaaacccgctacccccgccgccgccccagcagcgggaccttgcttcccaggatggcacccagaaagaagcagcagccgccgccgccgccgcagccatacatgcttctggaggaagaggaggaggactgggacagtcaggcagaggaggtttcggacgaggagcaggaggagatgatggaagactgggaggaggacagcagcctagacgaggaagcttcagaggccgaagaggtggcagacgcaacaccatcgccctcggtcgcagccccctcgccggggcccctgaaatcctccgaacccagcaccagcgctataacctccgctcctccggcgccggcgccacccgcccgcagacccaaccgtagatgggacaccacaggaaccggggtcggtaagtccaagtgcccgccgccgccaccgcagcagcagcagcagcagcgccagggctaccgctcgtggcgcgggcacaagaacgccatagtcgcctgcttgcaagactgcgggggcaacatctctttcgcccgccgcttcctgctattccaccacggggtcgcctttccccgcaatgtcctgcattactaccgtcatctctacagcccctactgcagcggcgacccagaggcggcagcggcagccacagcggcgaccaccacctaggaagatatcctccgcgggcaagacagcggcagcagcggccaggagacccgcggcagcagcggcgggagcggtgggcgcactgcgcctctcgcccaacgaacccctctcgacccgggagctcagacacaggatcttccccactttgtatgccatcttccaacagagcagaggccaggagcaggagctgaaaataaaaaacagatctctgcgctccctcacccgcagctgtctgtatcacaaaagcgaagatcagcttcggcgcacgctggaggacgcggaggcactcttcagcaaatactgcgcgctcactcttaaagactagctccgcgcccttctcgaatttaggcgggagaaaactacgtcatcgccggccgccgcccagcccgcccagccgagatgagcaaagagattcccacgccatacatgtggagctaccagccgcagatgggactcgcggcgggagcggcccaggactactccacccgcatgaactacatgagcgcgggaccccacatgatctcacaggtcaacgggatccgcgcccagcgaaaccaaatactgctggaacaggcggccatcaccgccacgccccgccataatctcaacccccgaaattggcccgccgccctcgtgtaccaggaaaccccctccgccaccaccgtactacttccgcgtgacgcccaggccgaagtccagatgactaactcaggggcgcagctcgcgggcggctttcgtcacggggcgcggccgctccgaccaggtataagacacctgatgatcagaggccgaggtatccagctcaacgacgagtcggtgagctcttcgctcggtctccgtccggacggaactttccagctcgccggatccggccgctcttcgttcacgccccgccaggcgtacctgactctgcagacctcgtcctcggagccccgctccggcggcatcggaaccctccagttcgtggaggagttcgtgccctcggtctacttcaaccccttctcgggacctcccggacgctaccccgaccagttcattccgaactttgacgcggtgaaggactcggcggacggctacgactgaatgtcaggtgtcgaggcagagcagcttcgcctgagacacctcgagcactgccgccgccacaagtgcttcgcccgcggttctggtgagttctgctactttcagctacccgaggagcataccgaggggccggcgcacggcgtccgcctgaccacccagggcgaggttacctgttccctcatccgggagtttaccctccgtcccctgctagtggagcgggagcggggtccctgtgtcctaactatcgcctgcaactgccctaaccctggattacatcaagatctttgctgtcatctctgtgctgagtttaataaacgctgagatcagaatctactgggatttagtcccctttaactaatcaaacactggaatcaataaaaagaatcacttacttaaaatcagacagcaggtctctgtccagtttattcagcagcacctccttcccctcctcccaactctggtactccaaacgccttctggcggcaaacttcctccacaccctgaagggaatgtcagattcttgctcctgtccctccgcacccactatcttcatgttgttgcagatgaagcgcaccaaaacgtctgacgagagcttcaaccccgtgtacccctatgacacggaaagcggccctccctccgtccctttcctcacccctcccttcgtgtctcccgatggattccaagaaagtccccccggggtcctgtctctgaacctggccgagcccctggtcacttcccacggcatgctcgccctgaaaatgggaagtggcctctccctggacgacgctggcaacctcacctctcaagatatcaccaccgctagccctcccctcaaaaaaaccaagaccaacctcagcctagaaacctcatcccccctaactgtgagcacctcaggcgccctcaccgtagcagccgccgctcccctggcggtggccggcacctccctcaccatgcaatcagaggcccccctgacagtacaggatgcaaaactcaccctggccaccaaaggccccctgaccgtgtctgaaggcaaactggccttgcaaacatcggccccgctgacggccgctgacagcagcaccctcacagtcagtgccacaccaccccttagcacaagcaatggcagcttgggtattgacatgcaagcccccatttacaccaccaatggaaaactaggacttaactttggcgctcccctgcatgtggtagacagcctaaatgcactgactgtagttactggccaaggtcttacgataaacggaacagccctacaaactagagtctcaggtgccctcaactatgacacatcaggaaacctagaattgagagctgcagggggtatgcgagttgatgcaaatggtcaacttatccttgatgtagcttacccatttgatgcacaaaacaatctcagccttaggcttggacagggacccctgtttgttaactctgcccacaacttggatgttaactacaacagaggcctctacctgttcacatctggaaataccaaaaagctagaagttaatatcaaaacagccaagggtctcatttatgatgacactgctatagcaatcaatgcgggtgatgggctacagtttgactcaggctcagatacaaatccattaaaaactaaacttggattaggactggattatgactccagcagagccataattgctaaactgggaactggcctaagctttgacaacacaggtgccatcacagtaggcaacaaaaatgatgacaagcttaccttgtggaccacaccagacccatcccctaactgtagaatctattcagagaaagatgctaaattcacacttgttttgactaaatgcggcagtcaggtgttggccagcgtttctgttttatctgtaaaaggtagccttgcgcccatcagtggcacagtaactagtgctcagattgtcctcagatttgatgaaaatggagttctactaagcaattcttcccttgaccctcaatactggaactacagaaaaggtgaccttacagagggcactgcatataccaacgcagtgggatttatgcccaacctcacagcatacccaaaaacacagagccaaactgctaaaagcaacattgtaagtcaggtttacttgaatggggacaaatccaaacccatgaccctcaccattaccctcaatggaactaatgaaacaggagatgccacagtaagcacttactccatgtcattctcatggaactggaatggaagtaattacattaatgaaacgttccaaaccaactccttcaccttctcctacatcgcccaagaataaaaagcatgacgctgttgatttgattcaatgtgtttctgttttattttcaagcacaacaaaatcattcaagtcattcttccatcttagcttaatagacacagtagcttaatagacccagtagtgcaaagccccattctagcttataactagtggagaagtactcgcctacatgggggtagagtcataatcgtgcatcaggatagggcggtggtgctgcagcagcgcgcgaataaactgctgccgccgccgctccgtcctgcaggaatacaacatggcagtggtctcctcagcgatgattcgcaccgcccgcagcataaggcgccttgtcctccgggcacagcagcgcaccctgatctcacttaaatcagcacagtaactgcagcacagcaccacaatattgttcaaaatcccacagtgcaaggcgctgtatccaaagctcatggcggggaccacagaacccacgtggccatcataccacaagcgcaggtagattaagtggcgacccctcataaacacgctggacataaacattacctcttttggcatgttgtaattcaccacctcccggtaccatataaacctctgattaaacatggcgccatccaccaccatcctaaaccagctggccaaaacctgcccgccggctatacactgcagggaaccgggactggaacaatgacagtggagagcccaggactcgtaaccatggatcatcatgctcgtcatgatatcaatgttggcacaacacaggcacacgtgcatacacttcctcaggattacaagctcctcccgcgttagaaccatatcccagggaacaacccattcctgaatcagcgtaaatcccacactgcagggaagacctcgcacgtaactcacgttgtgcattgtcaaagtgttacattcgggcagcagcggatgatcctccagtatggtagcgcgggtttctgtctcaaaaggaggtagacgatccctactgtacggagtgcgccgagacaaccgagatcgtgttggtcgtagtgtcatgccaaatggaacgccggacgtagtcatatttcctgaagtcttagatctctcaacgcagcaccagcaccaacacttcgcagtgtaaaaggccaagtgccgagagagtatatataggaataaaaagtgacgtaaacgggcaaagtccaaaaaacgcccagaaaaaccgcacgcgaacctacgccccgaaacgaaagccaaaaaacactagacactcccttccggcgtcaacttccgctttcccacgctacgtcacttgccccagtcaaacaaactacatatcccgaacttccaagtcgccacgcccaaaacaccgcctacacctccccgcccgccggcccgcccccaaacccgcctcccgccccgcgccccgccccgcgccgcccatctcattatcatattggcttcaatccaaaataaggtatattattgatgatggtttaaacggatcctctagagtcgacctgcaggcatgcaagcttgagtattctatagtgtcacctaaatagcttggcgtaatcatggtcatagctgtttcctgtgtgaaattgttatccgctcacaattccacacaacatacgagccggaagcataaagtgtaaagcctggggtgcctaatgagtgagctaactcacattaattgcgttgcgctcactgcccgctttccagtcgggaaacctgtcgtgccagctgcattaatgaatcggccaacgcgaaccccttgcggccgcccgggccgtcgaccaattctcatgtttgacagcttatcatcgaatttctgccattcatccgcttattatcacttattcaggcgtagcaaccaggcgtttaagggcaccaataactgccttaaaaaaattacgccccgccctgccactcatcgcagtactgttgtaattcattaagcattctgccgacatggaagccatcacaaacggcatgatgaacctgaatcgccagcggcatcagcaccttgtcgccttgcgtataatatttgcccatggtgaaaacgggggcgaagaagttgtccatattggccacgtttaaatcaaaactggtgaaactcacccagggattggctgagacgaaaaacatattctcaataaaccctttagggaaataggccaggttttcaccgtaacacgccacatcttgcgaatatatgtgtagaaactgccggaaatcgtcgtggtattcactccagagcgatgaaaacgtttcagtttgctcatggaaaacggtgtaacaagggtgaacactatcccatatcaccagctcaccgtctttcattgccatacggaattccggatgagcattcatcaggcgggcaagaatgtgaataaaggccggataaaacttgtgcttatttttctttacggtctttaaaaaggccgtaatatccagctgaacggtctggttataggtacattgagcaactgactgaaatgcctcaaaatgttctttacgatgccattgggatatatcaacggtggtatatccagtgatttttttctccattttagcttccttagctcctgaaaatctcgataactcaaaaaatacgcccggtagtgatcttatttcattatggtgaaagttggaacctcttacgtgccgatcaacgtctcattttcgccaaaagttggcccagggcttcccggtatcaacagggacaccaggatttatttattctgcgaagtgatcttccgtcacaggtatttattcgcgataagctcatggagcggcgtaaccgtcgcacaggaaggacagagaaagcgcggatctgggaagtgacggacagaacggtcaggacctggattggggaggcggttgccgccgctgctgctgacggtgtgacgttctctgttccggtcacaccacatacgttccgccattcctatgcgatgcacatgctgtatgccggtataccgctgaaagttctgcaaagcctgatgggacataagtccatcagttcaacggaagtctacacgaaggtttttgcgctggatgtggctgcccggcaccgggtgcagtttgcgatgccggagtctgatgcggttgcgatgctgaaacaattatcctgagaataaatgccttggcctttatatggaaatgtggaactgagtggatatgctgtttttgtctgttaaacagagaagctggctgttatccactgagaagcgaacgaaacagtcgggaaaatctcccattatcgtagagatccgcattattaatctcaggagcctgtgtagcgtttataggaagtagtgttctgtcatgatgcctgcaagcggtaacgaaaacgatttgaatatgccttcaggaacaatagaaatcttcgtgcggtgttacgttgaagtggagcggattatgtcagcaatggacagaacaacctaatgaacacagaaccatgatgtggtctgtccttttacagccagtagtgctcgccgcagtcgagcgacagggcgaagccctcgagtgagcgaggaagcaccagggaacagcacttatatattctgcttacacacgatgcctgaaaaaacttcccttggggttatccacttatccacggggatatttttataattattttttttatagtttttagatcttcttttttagagcgccttgtaggcctttatccatgctggttctagagaaggtgttgtgacaaattgccctttcagtgtgacaaatcaccctcaaatgacagtcctgtctgtgacaaattgcccttaaccctgtgacaaattgccctcagaagaagctgttttttcacaaagttatccctgcttattgactcttttttatttagtgtgacaatctaaaaacttgtcacacttcacatggatctgtcatggcggaaacagcggttatcaatcacaagaaacgtaaaaatagcccgcgaatcgtccagtcaaacgacctcactgaggcggcatatagtctctcccgggatcaaaaacgtatgctgtatctgttcgttgaccagatcagaaaatctgatggcaccctacaggaacatgacggtatctgcgagatccatgttgctaaatatgctgaaatattcggattgacctctgcggaagccagtaaggatatacggcaggcattgaagagtttcgcggggaaggaagtggttttttatcgccctgaagaggatgccggcgatgaaaaaggctatgaatcttttccttggtttatcaaacgtgcgcacagtccatccagagggctttacagtgtacatatcaacccatatctcattcccttctttatcgggttacagaaccggtttacgcagtttcggcttagtgaaacaaaagaaatcaccaatccgtatgccatgcgtttatacgaatccctgtgtcagtatcgtaagccggatggctcaggcatcgtctctctgaaaatcgactggatcatagagcgttaccagctgcctcaaagttaccagcgtatgcctgacttccgccgccgcttcctgcaggtctgtgttaatgagatcaacagcagaactccaatgcgcctctcatacattgagaaaaagaaaggccgccagacgactcatatcgtattttccttccgcgatatcacttccatgacgacaggatagtctgagggttatctgtcacagatttgagggtggttcgtcacatttgttctgacctactgagggtaatttgtcacagttttgctgtttccttcagcctgcatggattttctcatactttttgaactgtaatttttaaggaagccaaatttgagggcagtttgtcacagttgatttccttctctttcccttcgtcatgtgacctgatatcgggggttagttcgtcatcattgatgagggttgattatcacagtttattactctgaattggctatccgcgtgtgtacctctacctggagtttttcccacggtggatatttcttcttgcgctgagcgtaagagctatctgacagaacagttcttctttgcttcctcgccagttcgctcgctatgctcggttacacggctgcggcgagcgctagtgataataagtgactgaggtatgtgctcttcttatctccttttgtagtgttgctcttattttaaacaactttgcggttttttgatgactttgcgattttgttgttgctttgcagtaaattgcaagatttaataaaaaaacgcaaagcaatgattaaaggatgttcagaatgaaactcatggaaacacttaaccagtgcataaacgctggtcatgaaatgacgaaggctatcgccattgcacagtttaatgatgacagcccggaagcgaggaaaataacccggcgctggagaataggtgaagcagcggatttagttggggtttcttctcaggctatcagagatgccgagaaagcagggcgactaccgcacccggatatggaaattcgaggacgggttgagcaacgtgttggttatacaattgaacaaattaatcatatgcgtgatgtgtttggtacgcgattgcgacgtgctgaagacgtatttccaccggtgatcggggttgctgcccataaaggtggcgtttacaaaacctcagtttctgttcatcttgctcaggatctggctctgaaggggctacgtgttttgctcgtggaaggtaacgacccccagggaacagcctcaatgtatcacggatgggtaccagatcttcatattcatgcagaagacactctcctgcctttctatcttggggaaaaggacgatgtcacttatgcaataaagcccacttgctggccggggcttgacattattccttcctgtctggctctgcaccgtattgaaactgagttaatgggcaaatttgatgaaggtaaactgcccaccgatccacacctgatgctccgactggccattgaaactgttgctcatgactatgatgtcatagttattgacagcgcgcctaacctgggtatcggcacgattaatgtcgtatgtgctgctgatgtgctgattgttcccacgcctgctgagttgtttgactacacctccgcactgcagtttttcgatatgcttcgtgatctgctcaagaacgttgatcttaaagggttcgagcctgatgtacgtattttgcttaccaaatacagcaatagtaatggctctcagtccccgtggatggaggagcaaattcgggatgcctggggaagcatggttctaaaaaatgttgtacgtgaaacggatgaagttggtaaaggtcagatccggatgagaactgtttttgaacaggccattgatcaacgctcttcaactggtgcctggagaaatgctctttctatttgggaacctgtctgcaatgaaattttcgatcgtctgattaaaccacgctgggagattagataatgaagcgtgcgcctgttattccaaaacatacgctcaatactcaaccggttgaagatacttcgttatcgacaccagctgccccgatggtggattcgttaattgcgcgcgtaggagtaatggctcgcggtaatgccattactttgcctgtatgtggtcgggatgtgaagtttactcttgaagtgctccggggtgatagtgttgagaagacctctcgggtatggtcaggtaatgaacgtgaccaggagctgcttactgaggacgcactggatgatctcatcccttcttttctactgactggtcaacagacaccggcgttcggtcgaagagtatctggtgtcatagaaattgccgatgggagtcgccgtcgtaaagctgctgcacttaccgaaagtgattatcgtgttctggttggcgagctggatgatgagcagatggctgcattatccagattgggtaacgattatcgcccaacaagtgcttatgaacgtggtcagcgttatgcaagccgattgcagaatgaatttgctggaaatatttctgcgctggctgatgcggaaaatatttcacgtaagattattacccgctgtatcaacaccgccaaattgcctaaatcagttgttgctcttttttctcaccccggtgaactatctgcccggtcaggtgatgcacttcaaaaagcctttacagataaagaggaattacttaagcagcaggcatctaaccttcatgagcagaaaaaagctggggtgatatttgaagctgaagaagttatcactcttttaacttctgtgcttaaaacgtcatctgcatcaagaactagtttaagctcacgacatcagtttgctcctggagcgacagtattgtataagggcgataaaatggtgcttaacctggacaggtctcgtgttccaactgagtgtatagagaaaattgaggccattcttaaggaacttgaaaagccagcaccctgatgcgaccacgttttagtctacgtttatctgtctttacttaatgtcctttgttacaggccagaaagcataactggcctgaatattctctctgggcccactgttccacttgtatcgtcggtctgataatcagactgggaccacggtcccactcgtatcgtcggtctgattattagtctgggaccacggtcccactcgtatcgtcggtctgattattagtctgggaccacggtcccactcgtatcgtcggtctgataatcagactgggaccacggtcccactcgtatcgtcggtctgattattagtctgggaccatggtcccactcgtatcgtcggtctgattattagtctgggaccacggtcccactcgtatcgtcggtctgattattagtctggaaccacggtcccactcgtatcgtcggtctgattattagtctgggaccacggtcccactcgtatcgtcggtctgattattagtctgggaccacgatcccactcgtgttgtcggtctgattatcggtctgggaccacggtcccacttgtattgtcgatcagactatcagcgtgagactacgattccatcaatgcctgtcaagggcaagtattgacatgtcgtcgtaacctgtagaacggagtaacctcggtgtgcggttgtatgcctgctgtggattgctgctgtgtcctgcttatccacaacattttgcgcacggttatgtggacaaaatacctggttacccaggccgtgccggcacgttaaccgggctgcatccgatgcaagtgtgtcgctgtcgacgagctcgcgagctcggacatgaggttgccccgtattcagtgtcgctgatttgtattgtctgaagttgtttttacgttaagttgatgcagatcaattaatacgatacctgcgtcataattgattatttgacgtggtttgatggcctccacgcacgttgtgatatgtagatgataatcattatcactttacgggtcctttccggtgatccgacaggttacggggcggcgacctcgcgggttttcgctatttatgaaaattttccggtttaaggcgtttccgttcttcttcgtcataacttaatgtttttatttaaaataccctctgaaaagaaaggaaacgacaggtgctgaaagcgagctttttggcctctgtcgtttcctttctctgtttttgtccgtggaatgaacaatggaagtccgagctcatcgctaataacttcgtatagcatacattatacgaagttatattcgatgcggccgcaaggggttcgcgtcagcgggtgttggcgggtgtcggggctggcttaactatgcggcatcagagcagattgtactgagagtgcaccatatgcggtgtgaaataccgcacagatgcgtaaggagaaaataccgcatcaggcgccattcgccattcaggctgcgcaactgttgggaagggcgatcggtgcgggcctcttcgctattacgccagctggcgaaagggggatgtgctgcaaggcgattaagttgggtaacgccagggttttcccagtcacgacgttgtaaaacgacggccagtgaattgtaatacgactcactatagggcgaattcgagctcggtacccggggatcctcgtttaaac

SEQ ID NO: 52 - DNA, 43711 bp, Artificial Sequence
  source: /note="Description of Artificial Sequence: Synthetic polynucleotide"
  modified_base (15388)..(15388): a, c, t, g, unknown or other
catcatcaataatataccttattttggattgaagccaatatgataatgagatgggcggcgcggggcggggcgcggggcgggaggcgggtttgggggcgggccggcgggcggggcggtgtggcggaagtggactttgtaagtgtggcggatgtgacttgctagtgccgggcgcggtaaaagtgacgttttccgtgcgcgacaacgcccccgggaagtgacatttttcccgcggtttttaccggatgttgtagtgaatttgggcgtaaccaagtaagatttggccattttcgcgggaaaactgaaacggggaagtgaaatctgattaattttgcgttagtcataccgcgtaatatttgtctagggccgagggactttggccgattacgtggaggactcgcccaggtgttttttgaggtgaatttccgcgttccgggtcaaagtctgcgttttattattataggatatcccattgcatacgttgtatccatatcataatatgtacatttatattggctcatgtccaacattaccgccatgttgacattgattattgactagttattaatagtaatcaattacggggtcattagttcatagcccatatatggagttccgcgttacataacttacggtaaatggcccgcctggctgaccgcccaacgacccccgcccattgacgtcaataatgacgtatgttcccatagtaacgccaatagggactttccattgacgtcaatgggtggagtatttacggtaaactgcccacttggcagtacatcaagtgtatcatatgccaagtacgccccctattgacgtcaatgacggtaaatggcccgcctggcattatgcccagtacatgaccttatgggactttcctacttggcagtacatctacgtattagtcatcgctattaccatggtgatgcggttttggcagtacatcaatgggcgtggatagcggtttgactcacggggatttccaagtctccaccccattgacgtcaatgggagtttgttttggcaccaaaatcaacgggactttccaaaatgtcgtaacaactccgccccattgacgcaaatgggcggtaggcgtgtacggtgggaggtctatataagcagagctctccctatcagtgatagagatctccctatcagtgatagagatcgtcgacgagctcgtttagtgaaccgtcagatcgcctggagacgccatccacgctgttttgacctccatagaagacaccgggaccgatccagcctccgcggccgggaacggtgcattggaacgcggattccccgtgccaagagtgagatcttccgtttatctaggtaccagatatcgccaccatgtccgaggactttctgattctgatcgccatcctggtgatcgtgattctcgtgggcacaatcacaaccctggtgggcgccatcggcggcattagggccaggaggagcttcctcttcatttgcatcttcttcctgttcctctccctcttcctgacaatcctcgccctgctgctgggcttcagctggctcctgctggtggccatcctgttctgggtgctctggctggtcatcctcattctgctgctgctggtgtaccctattcctcaccaccccctgcccacctccctcaggtttagaatgaagcagagggtgagcagcgaccccacaggttctgacagaagccctcagggcagccataatagcctgaactcccccgatgaggaggaccccaaggatgacaccaagcaacctctgtgcaacatgacccagggcggacctcccgtcaatggacagctcctcggacaacatgctcaatgcccccctcactatccctgctgccatattcagcatcccgacggagaggattccgatggagacgatggcaagtcctggggcgatgccggagaggaagacaatggccctaacgaccctaacaccgccagcaccagagagtccatttacgaggacctcagataccccacaagggacgccaatggcgagtatgagaacgtgggatacccccctagggacggagatgcccctcataggctcggagagcctgtgtatgacgatgtggagcaagccaccgctaacgaggtgagaatctcccctctgttcagactgccctacggaagcgctttcggacctggcccccagcctggacccattctggagagctccacatggggctttctggtcttcacacagacctccctgttcgccgacgacattgccgacgctattagggactactgcacaacccaccctggccccacaaggaacacccaggtggtcctcatgaacttcgagggcagcggagtgcccctgcctatgttttttccccctggagaggagacagaagagcagagagagggcgatagagctagcgactccgacgagtccgaagacgctcagatcctgaccgtgttctgcctgttttgccagtggacactctttatctgcctgggaatcaggatgatctgtaactggaggggcaaactcaccaggatcatctgcctgaagttctgcctctacggactgatttccgcctccctgtccttcggctggtacgcttttctgaaggaagtgaccctccccaccacagccaccgttgatcctaggcaactccccctgttcctcttcatcctgagctccgtgctggtgattctcgccatcatgatggagtttcaaacatcctccagcctcttcgctgctctgttcgtgattatcgccggaatgctgtgcgtcacagtgggcgtgatttttctgctggctggcgtcaagcctctcctgagcggcatgatctgcgcctccggcatcacaatgctcgtgctcggcgtcgtgctgctggtggtgtgcaccagaagccccagcccttgtcatcacagggatgaacccccctccagaagccccagccctcaacccaccgtctccgagcagtcccagcagtcccccaggcagcagagccctcaaggcacatcccagggttctacaagacctcaggtgcctggaggcgccaccaccagaaaaagaggcggcgtgagaggccaacctgccaagtgtcacggcaagtacaccacaaccgccgagggactgaccgctctcctgaataggaggcacagccccaggacatccaacgagggcaggtggatgaatggagtcatggctgtgaacctctccaaatggcccctgtacagcctgaggagagccctggccctcgccatggctcctagaaggaggctctccggccctccctggctgacagtgctgctgctgctgtccacactgagcgtggccgccctgctgattctcttcctgattttcagcgccggcgccaccattagcacagaagccagcctgctggtcctgctcctgctgtttgtgaccctgctgctgcctctcctgtcctccaacggactccagctccctgccgccctgattctgatccagtgtttcctcctggccgctgattatctcgcctacctgattctgcctaccattatgcccaggggcagaagcacaggaaggaagggcagggacacagagaaagagaggagcagatcccctctcagagctcctggcggttctgatggacccagcacaagggctggctgtggagccggaccctgtcagctgagcagccccatcgccggaaacaacggcaatgaaggcggcgagggcgacgactacaagagctggaggaagcccgaggaagaggacaacggccccaatgaccccaataccaacaacaggattgaggatggagacggcgacgacggaaaatcctggaggaatcctgaggaggaggataacagaaagcaggacaggctgggcaccaagcctttcatggccggccactggtatgagagcgtgattcccggcctgttcctctgccccctgatcctcccttccctgttctggatttgctccctgctgaccttcctggtgggccacggagccaatattgtgagcgccgtcctgttcctcgtgctggcttggtgtctcctcattgccaactggaacgtgacaagagaggacttcgtgtccggcaggagaagctccatgagcagcctgtccgtggccgcttccaccgccacagccatgttcgccagcttcctcaccctgagctttgatggcctgggcctgctgctgtttggcaccgccctggtgatccagacaatttacgtgctgtatctggtggtcatggagatcaccgtgtggatcatgatgtttaggtatctccacttttggatcaccctgctgttcctgctgagccccattattctctccgtcgcctgtctcatcatccaatcctccgccctgctgatcgaggctgtggtcgtcaccaccatcacagtcctggccatttttctgtggctccctcctcaaggcgctgaggccgatctcggcaccgccctgctgattctgaataccgccctgtgcctggtcgtgctgatcctgaccgctatccctacatgatgatgagcggccgcgatctgctgtgccttctagttgccagccatctgttgtttgcccctcccccgtgccttccttgaccctggaaggtgccactcccactgtcctttcctaataaaatgaggaaattgcatcgcattgtctgagtaggtgtcattctattctggggggtggggtggggcaggacagcaagggggaggattgggaagacaatagcaggcatgctggggatgcggtgggctctatggccgatcagcgatcgctgaggtgggtgagtgggcgtggcctggggtggtcatgaaaatatataagttgggggtcttagggtctctttatttgtgttgcagagaccgccggagccatgagcgggagcagcagcagcagcagtagcagcagcgccttggatggcagcatcgtgagcccttatttgacgacgcggatgccccactgggccggggtgcgtcagaatgtgatgggctccagcatcgacggccgacccgtcctgcccgcaaattccgccacgctgacctatgcgaccgtcgcggggacgccgttggacgccaccgccgccgccgccgccaccgcagccgcctcggccgtgcgcagcctggccacggactttgcattcctgggaccactggcgacaggggctacttctcgggccgctgctgccgccgttcgcgatgacaagctgaccgccctgctggcgcagttggatgcgcttactcgggaactgggtgacctttctcagcaggtcatggccctgcgccagcaggtctcctccctgcaagctggcgggaatgcttctcccacaaatgccgtttaagataaataaaaccagactctgtttggattaaagaaaagtagcaagtgcattgctctctttatttcataattttccgcgcgcgataggccctagaccagcgttctcggtcgttgagggtgcggtgtatcttctccaggacgtggtagaggtggctctggacgttgagatacatgggcatgagcccgtcccgggggtggaggtagcaccactgcagagcttcatgctccggggtggtgttgtagatgatccagtcgtagcaggagcgctgggcatggtgcctaaaaatgtccttcagcagcaggccgatggccagggggaggcccttggtgtaagtgtttacaaaacggttaagttgggaagggtgcattcggggagagatgatgtgcatcttggactgtatttttagattggcgatgtttccgcccagatcccttctgggattcatgttgtgcaggaccaccagtacagtgtatccggtgcacttggggaatttgtcatgcagcttagagggaaaagcgtggaagaacttggagacgcctttgtggcctcccagattttccatgcattcgtccatgatgatggcaatgggcccgcgggaggcagcttgggcaaagatatttctggggtcgctgacgtcgtagttgtgttccagggtgaggtcgtcataggccatttttacaaagcgcgggcggagggtgcccgactgggggatgatggtcccctctggccctggggcgtagttgccctcgcagatctgcatttcccaggccttaatctcggaggggggaatcatatccacctgcggggcgatgaagaaaacggtttccggagccggggagattaactgggatgagagcaggtttctaagcagctgtgattttccacaaccggtgggcccataaataacacctataaccggttgcagctggtagtttagagagctgcagctgccgtcgtcccggaggaggggggccacctcgttgagcatgtccctgacgcgcatgttctccccgaccagatccgccagaaggcgctcgccgcccagggacagcagctcttgcaaggaagcaaagtttttcagcggcttgaggccgtccgccgtgggcatgtttttcagggtctggctcagcagctccaggcggtcccagagctcggtgacgtgctctacggcatctctatccagcatatctcctcgtttcgcgggttggggcgactttcgctgtagggcaccaagcggtggtcgtccagcggggccagagtcatgtccttccatgggcgcagggtcctcgtcagggtggtctgggtcacggtgaaggggtgcgctccgggctgagcgcttgccaaggtgcgcttgaggctggttctgctggtgctgaagcgctgccggtcttcgccctgcgcgtcggccaggtagcatttgaccatggtgtcatagtccagcccctccgcggcgtgtcccttggcgcgcagcttgcccttggaggtggcgccgcacgaggggcagagcaggctcttgagcgcgtagagcttgggggcgaggaagaccgattcgggggagtaggcgtccgcgccgcagaccccgcacacggtctcgcactccaccagccaggtgagctcggggcgcgccgggtcaaaaaccaggtttcccccatgctttttgatgcgtttcttacctcgggtctccatgaggtggtgtccccgctcggtgacgaagaggctgtccgtgtctccgtagaccgacttgaggggtcttttctccaggggggtccctcggtcttcctcgtagaggaactcggaccactctgagacgaaggcccgcgtccaggccaggacgaaggaggctatgtgggaggggtagcggtcgttgtccactagggggtccaccttctccaaggtgtgaagacacatgtcgccttcctcggcgtccaggaaggtgattggcttgtaggtgtaggccacgtgaccgggggttcctgacgggggggtataaaagggggtgggggcgcgctcgtcgtcactctcttccgcatcgctgtctgcgagggccagctgctggggtgagtattccctctcgaaggcgggcatgacctccgcgctgaggttgtcagtttccaaaaacgaggaggatttgatgttcacctgtcccgaggtgatacctttgagggtacccgcgtccatctggtcagaaaacacgatctttttattgtccagcttggtggcgaacgacccgtagagggcgttggagagcagcttggcgatggagcgcagggtctggttcttgtccctgtcggcgcgctccttggccgcgatgttgagctgcacgtactcgcgcgcgacgcagcgccactcggggaagacggtggtgcgctcgtcgggcaccaggcgcacgcgccagccgcggttgtgcagggtgaccaggtccacgctggtggcgacctcgccgcgcaggcgctcgttggtccagcagagacggccgcccttgcgcgagcagaaggggggcagggggtcgagctgggtctcgtccggggggtccgcgtccacggtgaaaaccccggggcgcaggcgcgcgtcgaagtagtctatcttgcaaccttgcatgtccagcgcctgctgccagtcgcgggcggcgagcgcgcgctcgtaggggttgagcggcgggccccagggcatggggtgggtgagtgcggaggcgtacatgccgcagatgtcatagacgtagaggggctcccgcaggaccccgatgtaggtggggtagcagcggccgccgcggatgctggcgcgcacgtagtcatacagctcgtgcgagggggcgaggaggtcggggcccaggttggtgcgggcggggcgctccgcgcggaagacgatctgcctgaagatggcatgcgagttggaagagatggtggggcgctggaagacgttgaagctggcgtcctgcaggccgacggcgtcgcgcacgaaggaggcgtaggagtcgcgcagcttgtgtaccagctcggcggtgacctgcacgtcgagcgcgcagtagtcgagggtctcgcggatgatgtcatatttagcctgccccttctttttccacagctcgcggttgaggacaaactcttcgcggtctttccagtactcttggatcgggaaaccgtccggttccgaacggtaagagcctagcatgtagaactggttgacggcctggtaggcgcagcagcccttctccacggggagggcgtaggcctgcgcggccttgcggagcgaggtgtgggtcagggcgaaggtgtccctgaccatgactttgaggtactggtgcttgaagtcggagtcgtcgcagccgccccgctcccagagcgagaagtcggtgcgcttcttggagcgggggttgggcagagcgaaggtgacatcgttgaagaggattttgcccgcgcggggcatgaagttgcgggtgatgcggaagggccccggcacttcagagcggttgttgatgacctgggcggcgagcacgatctcgtcgaagccgttgatgttgtggcccacgatgtagagttccaggaagcggggccggccctttacggtgggcagcttctttagctcttcgtaggtgagctcctcgggcgaggcgaggccgtgctcggccagggcccagtccgcgaggtgcgggttgtctctgaggaaggacttccagaggtcgcgggccaggagggtctgcaggcggtctctgaaggtcctgaactggcggcccacggccattttttcgggggtgatgcagtagaaggtgagggggtcttgctgccagcggtcccagtcgagctgcagggcgaggtcgcgcgcggcggtgaccaggcgctcgtcgcccccgaatttcatgaccagcatgaagggcacgagctgctttccgaaggcccccatccaagtgtaggtctctacatcgtaggtgacaaagaggcgctccgtgcgaggatgcgagccgatcgggaagaactggatctcccgccaccagttggaggagtggctgttgatgtggtggaagtagaagtcccgtcgccgggccgaacactcgtgctggcttttgtaaaagcgagcgcagtactggcagcgctgcacgggctgtacctcatgcacgagatgcacctttcgcccgcgcacgaggaagccgaggggaaatctgagccccccgcctggctcgcggcatggctggttctcttctactttggatgcgtgtccgtctccgtctggctcctcgaggggtgttacggtggagcggaccaccacgccgcgcgagccgcaggtccagatatcggcgcgcggcggtcggagtttgatgacgacatcgcgcagctgggagctgtccatggtctggagctcccgcggcggcggcaggtcagccgggagttcttgcaggttcacctcgcagagtcgggccagggcgcggggcaggtctaggtggtacctgatctctaggggcgtgttggtggcggcgtcgatggcttgcaggagcccgcagccccggggggcgacgacggtgccccgcggggtggtggtggtggtggcggtgcagctcagaagcggtgccgcgggcgggcccccggaggtagggggggctccggtcccgcgggcaggggcggcagcggcacgtcggcgtggagcgcgggcaggagttggtgctgtgcccggaggttgctggcgaaggcgacgacgcggcggttgatctcctggatctggcgcctctgcgtgaagacgacgggcccggtgagcttgaacctgaaagagagttcgacagaatcaatctcggtgtcattgaccgcggcctggcgcaggatctcctgcacgtctcccgagttgtcttggtaggcgatctcggccatgaactgctcgatctcttcctcctggaggtctccgcgtccggcgcgttccacggtggccgccaggtcgttggagatgcgccccatgagctgcgagaaggcgttgagtccgccctcgttccagactcggctgtagaccacgcccccctggtcatcgcgggcgcgcatgaccacctgcgcgaggttgagctccacgtgccgcgcgaagacggcgtagttgcgcagacgctggaagaggtagttgagggtggtggcggtgtgctcggccacgaagaagttcatgacccagcggcgcaacgtggattcgttgatgtcccccaaggcctccagccgttccatggcctcgtagaagtccacggcgaagttgaaaaactgggagttgcgcgccgacacggtcaactcctcctccagaagacggatgagctcggcgacggtgtcgcgcacctcgcgctcgaaggctatggggatctcttcctccgctagcatcaccacctcctcctcttcctcctcttctggcacttccatgatggcttcctcctcttcggggggtggcggcggcggcggtgggggagggggcgctctgcgccggcggcggcgcaccgggaggcggtccacgaagcgcgcgatcatctccccgcggcggcggcgcatggtctcggtgacggcgcggccgttctcccgggggcgcagttggaagacgccgccggacatctggtgctggggcgggtggccgtgaggcagcgagacggcgctgacgatgcatctcaacaattgctgcgtaggtacgccgccgagggacctgagggagtccatatccaccggatccgaaaacctttcgaggaaggcgtctaaccagtcgcagtcgcaaggtaggctgagcaccgtggcgggcggcggggggtggggggagtgtctggcggaggtgctgctgatgatgtaattgaagtaggcggacttgacacggcggatggtcgacaggagcaccatgtccttgggtccggcctgctggatgcggaggcggtcggctatgccccaggcttcgttctggcatcggcgcaggtccttgtagtagtcttgcatgagcctttccaccggcacctcttctccttcctcttctgcttcttccatgtctgcttcggccctggggcggcgccgcgcccccctgccccccatgcgcgtgaccccgaaccccctgagcggttggagcagggccaggtcggcgacgacgcgctcggccaggatggcctgctgcacctgcgtgagggtggtttggaagtcatccaagtccacgaagcggtggtaggcgcccgtgttgatggtgtaggtgcagttggccatgacggaccagttgacggtctggtggcccggttgcgacatctcggtgtacctgagtcgcgagtaggcgcgggagtcgaagacgtagtcgttgcaagtccgcaccaggtactggtagcccaccaggaagtgcggcggcggctggcggtagaggggccagcgcagggtggcgggggctccgggggccaggtcttccagcatgaggcggtggtaggcgtagatgtacctggacatccaggtgatacccgcggcggtggtggaggcgcgcgggaagtcgcgcacccggttccagatgttgcgcaggggcagaaagtgctccatggtaggcgtgctctgtccagtcagacgcgcgcagtcgttgatactctagaccagggaaaacgaaagccggtcagcgggcactcttccgtggtctggtgaatagatcgcaagggtatcatggcggagggcctcggttcgagccccgggtccgggccggacggtccgccatgatccacgcggttaccgcccgcgtgtcgaacccaggtgtgcgacgtcagacaacggtggagtgttccttttggcgtttttctggccgggcgccggcgccgcgtaagagactaagccgcgaaagcgaaagcagtaagtggctcgctccccgtagccggagggatccttgctaagggttgcgttgcggcgaaccccggttcgaatcccgtactcgggccggccggacccgcggctaaggtgttggattggcctccccctcgtataaagaccccgcttgcggattgactccggacacggggacgagccccttttatttttgctttccccagatgcatccggtgctgcggcagatgcgccccccgccccagcagcagcaacaacaccagcaagagcggcagcaacagcagcgggagtcatgcagggccccctcacccaccctcggcgggccggccacctcggcgtccgcggccgtgtctggcgcctgcggcggcggcggggggccggctgacgaccccgaggagcccccgcggcgcagggccagacactacctggacctggaggagggcgagggcctggcgcggctgggggcgccgtctcccgagcgccacccgcgggtgcagctgaagcgcgactcgcgcgaggcgtacgtgcctcggcagaacctgttcagggaccgcgcgggcgaggagcccgaggagatgcgggacaggaggttcagcgcagggcgggagctgcggcaggggctgaaccgcgagcggctgctgcgcgaggaggactttgagcccgacgcgcggacggggatcagccccgcgcgcgcgcacgtggcggccgccgacctggtgacggcgtacgagcagacggtgaaccaggagatcaacttccaaaagagtttcaacaaccacgtgcgcacgctggtggcgcgcgaggaggtgaccatcgggctgatgcacctgtgggactttgtaagcgcgctggtgcagaaccccaacagcaagcctctgacggcgcagctgttcctgatagtgcagcacagcagggacaacgaggcgtttagggacgcgctgctgaacatcaccgagcccgagggtcggtggctgctggacctgattaacatcctgcagagcatagtggtgcaggagcgcagcctgagcctggccgacaaggtggcggccatcaactactcgatgctgagcctgggcaagttttacgcgcgcaagatctaccagacgccgtacgtgcccatagacaaggaggtgaagatcgacggtttttacatgcgcatggcgctgaaggtgctcaccctgagcgacgacctgggcgtgtaccgcaacgagcgcatccacaaggccgtgagcgtgagccggcggcgcgagctgagcgaccgcgagctgatgcacagcctgcagcgggcgctggcgggcgccggcagcggcgacagggaggcggagtcctacttcgatgcgggggcggacctgcgctgggcgcccagccggcgggccctggaggccgcgggggtccgcgaggactatgacgaggacggcgaggaggatgaggagtacgagctagaggagggcgagtacctggactaaaccgcgggtggtgtttccggtagatgcaagacccgaacgtggtggacccggcgctgcgggcggctctgcagagccagccgtccggccttaactcctcagacgactggcgacaggtcatggaccgcatcatgtcgctgacggcgcgtaacccggacgcgttccggcagcagccgcaggccaacaggctctccgccatcctggaggcggtggtgcctgcgcgctcgaaccccacgcacgagaaggtgctggccatagtgaacgcgctggccgagaacagggccatccgcccggacgaggccgggctggtgtacgacgcgctgctgcagcgcgtggcccgctacaacagcggcaacgtgcagaccaacctggaccggctggtgggggacgtgcgcgaggcggtggcgcagcgcgagcgcgcggatcggcagggcaacctgggctccatggtggcgctgaatgccttcctgagcacgcagccggccaacgtgccgcgggggcaggaagactacaccaactttgtgagcgcgctgcggctgatggtgaccgagaccccccagagcgaggtgtaccagtcgggcccggactacttcttccagaccagcagacagggcctgcagacggtgaacctgagccaggctttcaagaacctgcgggggctgtggggcgtgaaggcgcccaccggcgaccgggcgacggtgtccagcctgctgacgcccaactcgcgcctgctgctgctgctgatcgcgccgttcacggacagcggcagcgtgtcccgggacacctacctggggcacctgctgaccctgtaccgcgaggccatcgggcaggcgcaggtggacgagcacaccttccaggagatcaccagcgtgagccgcgcgctggggcaggaggacacgagcagcctggaggcgactctgaactacctgctgaccaaccggcggcagaagattccctcgctgcacagcctgacctccgaggaggagcgcatcttgcgctacgtgcagcagagcgtgagcctgaacctgatgcgcgacggggtgacgcccagcgtggcgctggacatgaccgcgcgcaacatggaaccgggcatgtacgccgcgcaccggccttacatcaaccgcctgatggactacctgcatcgcgcggcggccgtgaaccccgagtactttaccaacgccatcctgaacccgcactggctcccgccgcccgggttctacagcgggggcttcgaggtcccggagaccaacgatggcttcctgtgggacgacatggacgacagcgtgttctccccgcggccgcaggcgctggcggaagcgtccctgctgcgtcccaagaaggaggaggaggaggaggcgagtcgccgccgcggcagcagcggcgtggcttctctgtccgagctgggggcggcagccgccgcgcgccccgggtccctgggcggcagcccctttccgagcctggtggggtctctgcacagcgagcgcaccacccgccctcggctgctgggcgaggacgagtacctgaataactccctgctgcagccggtgcgggagaaaaacctgcctcccgccttccccaacaacgggatagagagcctggtggacaagatgagcagatggaagacctatgcgcaggagcacagggacgcgcctgcgctccggccgcccacgcggcgccagcgccacgaccggcagcgggggctggtgtgggatgacgaggactccgcggacgatagcagcgtgctggacctgggagggagcggcaacccgttcgcgcacctgcgcccccgcctggggaggatgttttaaaaaaaaaaaaaaaangcaagaagcatgatgcaaaaattaaataaaactcaccaaggccatggcgaccgagcgttggtttcttgtgttcccttcagtatgcggcgcgcggcgatgtaccaggagggacctcctccctcttacgagagcgtggtgggcgcggcggcggcggcgccctcttctccctttgcgtcgcagctgctggagccgccgtacgtgcctccgcgctacctgcggcctacgggggggagaaacagcatccgttactcggagctggcgcccctgttcgacaccacccgggtgtacctggtggacaacaagtcggcggacgtggcctccctgaactaccagaacgaccacagcaattttttgaccacggtcatccagaacaatgactacagcccgagcgaggccagcacccagaccatcaatctggatgaccggtcgcactggggcggcgacctgaaaaccatcctgcacaccaacatgcccaacgtgaacgagttcatgttcaccaataagttcaaggcgcgggtgatggtgtcgcgctcgcacaccaaggaagaccgggtggagctgaagtacgagtgggtggagttcgagctgccagagggcaactactccgagaccatgaccattgacctgatgaacaacgcgatcgtggagcactatctgaaagtgggcaggcagaacggggtcctggagagcgacatcggggtcaagttcgacaccaggaacttccgcctggggctggaccccgtgaccgggctggttatgcccggggtgtacaccaacgaggccttccatcccgacatcatcctgctgcccggctgcggggtggacttcacttacagccgcctgagcaacctcctgggcatccgcaagcggcagcccttccaggagggcttcaggatcacctacgaggacctggaggggggcaacatccccgcgctcctcgatgtggaggcctaccaggatagcttgaaggaaaatgaggcgggacaggaggataccgcccccgccgcctccgccgccgccgagcagggcgaggatgctgctgacaccgcggccgcggacggggcagaggccgaccccgctatggtggtggaggctcccgagcaggaggaggacatgaatgacagtgcggtgcgcggagacaccttcgtcacccggggggaggaaaagcaagcggaggccgaggccgcggccgaggaaaagcaactggcggcagcagcggcggcggcggcgttggccgcggcggaggctgagtctgaggggaccaagcccgccaaggagcccgtgattaagcccctgaccgaagatagcaagaagcgcagttacaacctgctcaaggacagcaccaacaccgcgtaccgcagctggtacctggcctacaactacggcgacccgtcgacgggggtgcgctcctggaccctgctgtgcacgccggacgtgacctgcggctcggagcaggtgtactggtcgctgcccgacatgatgcaagaccccgtgaccttccgctccacgcggcaggtcagcaacttcccggtggtgggcgccgagctgctgcccgtgcactccaagagcttctacaacgaccaggccgtctactcccagctcatccgccagttcacctctctgacccacgtgttcaatcgctttcctgagaaccagattctggcgcgcccgcccgcccccaccatcaccaccgtcagtgaaaacgttcctgctctcacagatcacgggacgctaccgctgcgcaacagcatcggaggagtccagcgagtgaccgttactgacgccagacgccgcacctgcccctacgtttacaaggccttgggcatagtctcgccgcgcgtcctttccagccgcactttttgagcaacaccaccatcatgtccatcctgatctcacccagcaataactccggctggggactgctgcgcgcgcccagcaagatgttcggaggggcgaggaagcgttccgagcagcaccccgtgcgcgtgcgcgggcacttccgcgccccctggggagcgcacaaacgcggccgcgcggggcgcaccaccgtggacgacgccatcgactcggtggtggagcaggcgcgcaactacaggcccgcggtctctaccgtggacgcggccatccagaccgtggtgcggggcgcgcggcggtacgccaagctgaagagccgccggaagcgcgtggcccgccgccaccgccgccgacccggggccgccgccaaacgcgccgccgcggccctgcttcgccgggccaagcgcacgggccgccgcgccgccatgagggccgcgcgccgcttggccgccggcatcaccgccgccaccatggccccccgtacccgaagacgcgcggccgccgccgccgccgccgccatcagtgacatggccagcaggcgccggggcaacgtgtactgggtgcgcgactcggtgaccggcacgcgcgtgcccgtgcgcttccgccccccgcggacttgagatgatgtgaaaaaacaacactgagtctcctgctgttgtgtgtatcccagcggcggcggcgcgcgcagcgtcatgtccaagcgcaaaatcaaagaagagatgctccaggtcgtcgcgccggagatctatgggcccccgaagaaggaagagcaggattcgaagccccgcaagataaagcgggtcaaaaagaaaaagaaagatgatgacgatgccgatggggaggtggagttcctgcgcgccacggcgcccaggcgcccggtgcagtggaagggccggcgcgtaaagcgcgtcctgcgccccggcaccgcggtggtcttcacgcccggcgagcgctccacccggactttcaagcgcgtctatgacgaggtgtacggcgacgaagacctgctggagcaggccaacgagcgcttcggagagtttgcttacgggaagcgtcagcgggcgctggggaaggaggacctgctggcgctgccgctggaccagggcaaccccacccccagtctgaagcccgtgaccctgcagcaggtgctgccgagcagcgcaccctccgaggcgaagcggggtctgaagcgcgagggcggcgacctggcgcccaccgtgcagctcatggtgcccaagcggcagaggctggaggatgtgctggagaaaatgaaagtagaccccggtctgcagccggacatcagggtccgccccatcaagcaggtggcgccgggcctcggcgtgcagaccgtggacgtggtcatccccaccggcaactcccccgccgccgccaccactaccgctgcctccacggacatggagacacagaccgatcccgccgcagccgcagccgcagccgccgccgcgacctcctcggcggaggtgcagacggacccctggctgccgccggcgatgtcagctccccgcgcgcgtcgcgggcgcaggaagtacggcgccgccaacgcgctcctgcccgagtacgccttgcatccttccatcgcgcccacccccggctaccgaggctatacctaccgcccgcgaagagccaagggttccacccgccgtccccgccgacgcgccgccgccaccacccgccgccgccgccgcagacgccagcccgcactggctccagtctccgtgaggaaagtggcgcgcgacggacacaccctggtgctgcccagggcgcgctaccaccccagcatcgtttaaaagcctgttgtggttcttgcagatatggccctcacttgccgcctccgtttcccggtgccgggataccgaggaggaagatcgcgccgcaggaggggtctggccggccgcggcctgagcggaggcagccgccgcgcgcaccggcggcgacgcgccaccagccgacgcatgcgcggcggggtgctgcccctgttaatccccctgatcgccgcggcgatcggcgccgtgcccgggatcgcctccgtggccttgcaagcgtcccagaggcattgacagacttgcaaacttgcaaatatggaaaaaaaaaccccaataaaaaagtctagactctcacgctcgcttggtcctgtgactattttgtagaatggaagacatcaactttgcgtcgctggccccgcgtcacggctcgcgcccgttcctgggacactggaacgatatcggcaccagcaacatgagcggtggcgccttcagttggggctctctgtggagcggcattaaaagtatcgggtctgccgttaaaaattacggctcccgggcctggaacagcagcacgggccagatgttgagagacaagttgaaagagcagaacttccagcagaaggtggtggagggcctggcctccggcatcaacggggtggtggacctggccaaccaggccgtgcagaataagatcaacagcagactggacccccggccgccggtggaggaggtgccgccggcgctggagacggtgtcccccgatgggcgtggcgagaagcgcccgcggcccgatagggaagagaccactctggtcacgcagaccgatgagccgcccccgtatgaggaggccctgaagcaaggtctgcccaccacgcggcccatcgcgcccatggccaccggggtggtgggccgccacacccccgccacgctggacttgcctccgcccgccgatgtgccgcagcagcagaaggcggcacagccgggcccgcccgcgaccgcctcccgttcctccgccggtcctctgcgccgcgcggccagcggcccccgcgggggggtcgcgaggcacggcaactggcagagcacgctgaacagcatcgtgggtctgggggtgcggtccgtgaagcgccgccgatgctactgaatagcttagctaacgtgttgtatgtgtgtatgcgccctatgtcgccgccagaggagctgctgagtcgccgccgttcgcgcgcccaccaccaccgccactccgcccctcaagatggcgaccccatcgatgatgccgcagtggtcgtacatgcacatctcgggccaggacgcctcggagtacctgagccccgggctggtgcagttcgcccgcgccaccgagagctacttcagcctgagtaacaagtttaggaaccccacggtggcgcccacgcacgatgtgaccaccgaccggtctcagcgcctgacgctgcggttcattcccgtggaccgcgaggacaccgcgtactcgtacaaggcgcggttcaccctggccgtgggcgacaaccgcgtgctggacatggcctccacctactttgacatccgcggggtgctggaccggggtcccactttcaagccctactctggcaccgcctacaactccctggcccccaagggcgctcccaactcctgcgagtgggagcaagaggaaactcaggcagttgaagaagcagcagaagaggaagaagaagatgctgacggtcaagctgaggaagagcaagcagctaccaaaaagactcatgtatatgctcaggctcccctttctggcgaaaaaattagtaaagatggtctgcaaataggaacggacgctacagctacagaacaaaaacctatttatgcagaccctacattccagcccgaaccccaaatcggggagtcccagtggaatgaggcagatgctacagtcgccggcggtagagtgctaaagaaatctactcccatgaaaccatgctatggttcctatgcaagacccacaaatgctaatggaggtcagggtgtactaacggcaaatgcccagggacagctagaatctcaggttgaaatgcaattcttttcaacttctgaaaacgcccgtaacgaggctaacaacattcagcccaaattggtgctgtatagtgaggatgtgcacatggagaccccggatacgcacctttcttacaagcccgcaaaaagcgatgacaattcaaaaatcatgctgggtcagcagtccatgcccaacagacctaattacatcggcttcagagacaactttatcggcctcatgtattacaatagcactggcaacatgggagtgcttgcaggtcaggcctctcagttgaatgcagtggtggacttgcaagacagaaacacagaactgtcctaccagctcttgcttgattccatgggtgacagaaccagatacttttccatgtggaatcaggcagtggacagttatgacccagatgttagaattattgaaaatcatggaactgaagacgagctccccaactattgtttccctctgggtggcataggggtaactgacacttaccaggctgttaaaaccaacaatggcaataacgggggccaggtgacttggacaaaagatgaaacttttgcagatcgcaatgaaataggggtgggaaacaatttcgctatggagatcaacctcagtgccaacctgtggagaaacttcctgtactccaacgtggcgctgtacctaccagacaagcttaagtacaacccctccaatgtggacatctctgacaaccccaacacctacgattacatgaacaagcgagtggtggccccggggctggtggactgctacatcaacctgggcgcgcgctggtcgctggactacatggacaacgtcaaccccttcaaccaccaccgcaatgcgggcctgcgctaccgctccatgctcctgggcaacgggcgctacgtgcccttccacatccaggtgccccagaagttctttgccatcaagaacctcctcctcctgccgggctcctacacctacgagtggaacttcaggaaggatgtcaacatggtcctccagagctctctgggtaacgatctcagggtggacggggccagcatcaagttcgagagcatctgcctctacgccaccttcttccccatggcccacaacacggcctccacgctcgaggccatgctcaggaacgacaccaacgaccagtccttcaatgactacctctccgccgccaacatgctctaccccatacccgccaacgccaccaacgtccccatctccatcccctcgcgcaactgggcggccttccgcggctgggccttcacccgcctcaagaccaaggagaccccctccctgggctcgggattcgacccctactacacctactcgggctccattccctacctggacggcaccttctacctcaaccacactttcaagaaggtctcggtcaccttcgactcctcggtcagctggccgggcaacgaccgtctgctcacccccaacgagttcgagatcaagcgctcggtcgacggggagggctacaacgtggcccagtgcaacatgaccaaggactggttcctggtccagatgctggccaactacaacatcggctaccagggcttctacatcccagagagctacaaggacaggatgtactccttcttcaggaacttccagcccatgagccggcaggtggtggaccagaccaagtacaaggactaccaggaggtgggcatcatccaccagcacaacaactcgggcttcgtgggctacctcgcccccaccatgcgcgagggacaggcctaccccgccaacttcccctatccgctcataggcaagaccgcggtcgacagcatcacccagaaaaagttcctctgcgaccgcaccctctggcgcatccccttctccagcaacttcatgtccatgggtgcgctctcggacctgggccagaacttgctctacgccaactccgcccacgccctcgacatgaccttcgaggtcgaccccatggacgagcccacccttctctatgttctgttcgaagtctttgacgtggtccgggtccaccagccgcaccgcggcgtcatcgagaccgtgtacctgcgtacgcccttctcggccggcaacgccaccacctaaagaagcaagccgcagtcatcgccgcctgcatgccgtcgggttccaccgagcaagagctcagggccatcgtcagagacctgggatgcgggccctattttttgggcaccttcgacaagcgcttccctggctttgtctccccacacaagctggcctgcgccatcgtcaacacggccggccgcgagaccgggggcgtgcactggctggccttcgcctggaacccgcgctccaaaacatgcttcctctttgaccccttcggcttttcggaccagcggctcaagcaaatctacgagttcgagtacgagggcttgctgcgtcgcagcgccatcgcctcctcgcccgaccgctgcgtcaccctcgaaaagtccacccagaccgtgcaggggcccgactcggccgcctgcggtctcttctgctgcatgtttctgcacgcctttgtgcactggcctcagagtcccatggaccgcaaccccaccatgaacttgctgacgggggtgcccaactccatgctccagagcccccaggtcgagcccaccctgcgccgcaaccaggagcagctctacagcttcctggagcgccactcgccttacttccgccgccacagcgcacagatcaggagggccacctccttctgccacttgcaagagatgcaagaagggtaataacgatgtacacactttttttctcaataaatggcatctttttatttatacaagctctctggggtattcatttcccaccaccacccgccgttgtcgccatctggctctatttagaaatcgaaagggttctgccgggagtcgccgtgcgccacgggcagggacacgttgcgatactggtagcgggtgccccacttgaactcgggcaccaccaggcgaggcagctcggggaagttttcgctccacaggctgcgggtcagcaccagcgcgttcatcaggtcgggcgccgagatcttgaagtcgcagttggggccgccgccctgcgcgcgcgagttgcggtacaccgggttgcagcactggaacaccaacagcgccgggtgcttcacgctggccagcacgctgcggtcggagatcagctcggcgtccaggtcctccgcgttgctcagcgcgaacggggtcatcttgggcacttgccgccccaggaagggcgcgtgccccggtttcgagttgcagtcgcagcgcagcgggatcagcaggtgcccgtgcccggactcggcgttggggtacagcgcgcgcatgaaggcctgcatctggcggaaggccatctgggccttggcgccctccgagaagaacatgccgcaggacttgcccgagaactggtttgcggggcagctggcgtcgtgcaggcagcagcgcgcgtcggtgttggcgatctgcaccacgttgcgcccccaccggttcttcacgatcttggccttggacgattgctccttcagcgcgcgctgcccgttctcgctggtcacatccatctcgatcacatgttccttgttcaccatgctgctgccgtgcagacacttcagctcgccctccgtctcggtgcagcggtgctgccacagcgcgcagcccgtgggctcgaaagacttgtaggtcacctccgcgaaggactgcaggtacccctgcaaaaagcggcccatcatggtcacgaaggtcttgttgctgctgaaggtcagctgcagcccgcggtgctcctcgttcagccaggtcttgcacacggccgccagcgcctccacctggtcgggcagcatcttgaagttcaccttcagctcattctccacgtggtacttgtccatcagcgtgcgcgccgcctccatgcccttctcccaggccgacaccagcggcaggctcacggggttcttcaccatcaccgtggccgccgcctccgccgcgctttcgctttccgccccgctgttctcttcctcttcctcctcttcctcgccgccgcccactcgcagcccccgcaccacggggtcgtcttcctgcaggcgctgcaccttgcgcttgccgttgcgcccctgcttgatgcgcacgggcgggttgctgaagcccaccatcaccagcgcggcctcttcttgctcgtcctcgctgtccagaatgacctccggggagggggggttggtcatcctcagtaccgaggcacgcttctttttcttcctgggggcgttcgccagctccgcggctgcggccgctgccgaggtcgaaggccgagggctgggcgtgcgcggcaccagcgcgtcctgcgagccgtcctcgtcctcctcggactcgagacggaggcgggcccgcttcttcgggggcgcgcggggcggcggaggcggcggcggcgacggagacggggacgagacatcgtccagggtgggtggacggcgggccgcgccgcgtccgcgctcgggggtggtctcgcgctggtcctcttcccgactggccatctcccactgctccttctcctataggcagaaagagatcatggagtctctcatgcgagtcgagaaggaggaggacagcctaaccgccccctctgagccctccaccaccgccgccaccaccgccaatgccgccgcggacgacgcgcccaccgagaccaccgccagtaccaccctccccagcgacgcacccccgctcgagaatgaagtgctgatcgagcaggacccgggttttgtgagcggagaggaggatgaggtggatgagaaggagaaggaggaggtcgccgcctcagtgccaaaagaggataaaaagcaagaccaggacgacgcagataaggatgagacagcagtcgggcgggggaacggaagccatgatgctgatgacggctacctagacgtgggagacgacgtgctgcttaagcacctgcaccgccagtgcgtcatcgtctgcgacgcgctgcaggagcgctgcgaagtgcccctggacgtggcggaggtcagccgcgcctacgagcggcacctcttcgcgccgcacgtgccccccaagcgccgggagaacggcacctgcgagcccaacccgcgtctcaacttctacccggtcttcgcggtacccgaggtgctggccacctaccacatctttttccaaaactgcaagatccccctctcctgccgcgccaaccgcacccgcgccgacaaaaccctgaccctgcggcagggcgcccacatacctgatatcgcctctctggaggaagtgcccaagatcttcgagggtctcggtcgcgacgagaaacgggcggcgaacgctctgcacggagacagcgaaaacgagagtcactcgggggtgctggtggagctcgagggcgacaacgcgcgcctggccgtactcaagcgcagcatagaggtcacccactttgcctacccggcgctcaacctgccccccaaggtcatgagtgtggtcatgggcgagctcatcatgcgccgcgcccagcccctggccgcggatgcaaacttgcaagagtcctccgaggaaggcctgcccgcggtcagcgacgagcagctggcgcgctggctggagacccgcgaccccgcgcagctggaggagcggcgcaagctcatgatggccgcggtgctggtcaccgtggagctcgagtgtctgcagcgcttcttcgcggaccccgagatgcagcgcaagctcgaggagaccctgcactacaccttccgccagggctacgtgcgccaggcctgcaagatctccaacgtggagctctgcaacctggtctcctacctgggcatcctgcacgagaaccgcctcgggcagaacgtcctgcactccaccctcaaaggggaggcgcgccgcgactacatccgcgactgcgcctacctcttcctctgctacacctggcagacggccatgggggtctggcagcagtgcctggaggagcgcaacctcaaggagctggaaaagctcctcaagcgcaccctcagggacctctggacgggcttcaacgagcgctcggtggccgccgcgctggcggacatcatctttcccgagcgcctgctcaagaccctgcagcagggcctgcccgacttcaccagccagagcatgctgcagaacttcaggactttcatcctggagcgctcgggcatcctgccggccacttgctgcgcgctgcccagcgacttcgtgcccatcaagtacagggagtgcccgccgccgctctggggccactgctacctcttccagctggccaactacctcgcctaccactcggacctcatggaagacgtgagcggcgagggcctgctcgagtgccactgccgctgcaacctctgcacgccccaccgctctctagtctgcaacccgcagctgctcagcgagagtcagattatcggtaccttcgagctgcagggtccctcgcctgacgagaagtccgcggctccagggctgaaactcactccggggctgtggacttccgcctacctacgcaaatttgtacctgaggactaccacgcccacgagatcaggttctacgaagaccaatcccgcccgcccaaggcggagctcaccgcctgcgtcatcacccaggggcacatcctgggccaattgcaagccatcaacaaagcccgccgagagttcttgctgaaaaagggtcggggggtgtacctggacccccagtccggcgaggagctaaacccgctacccccgccgccgccccagcagcgggaccttgcttcccaggatggcacccagaaagaagcagcagccgccgccgccgccgcagccatacatgcttctggaggaagaggaggaggactgggacagtcaggcagaggaggtttcggacgaggagcaggaggagatgatggaagactgggaggaggacagcagcctagacgaggaagcttcagaggccgaagaggtggcagacgcaacaccatcgccctcggtcgcagccccctcgccggggcccctgaaatcctccgaacccagcaccagcgctataacctccgctcctccggcgccggcgccacccgcccgcagacccaaccgtagatgggacaccacaggaaccggggtcggtaagtccaagtgcccgccgccgccaccgcagcagcagcagcagcagcgccagggctaccgctcgtggcgcgggcacaagaacgccatagtcgcctgcttgcaagactgcgggggcaacatctctttcgcccgccgcttcctgctattccaccacggggtcgcctttccccgcaatgtcctgcattactaccgtcatctctacagcccctactgcagcggcgacccagaggcggcagcggcagccacagcggcgaccaccacctaggaagatatcctccgcgggcaagacagcggcagcagcggccaggagacccgcggcagcagcggcgggagcggtgggcgcactgcgcctctcgcccaacgaacccctctcgacccgggagctcagacacaggatcttccccactttgtatgccatcttccaacagagcagaggccaggagcaggagctgaaaataaaaaacagatctctgcgctccctcacccgcagctgtctgtatcacaaaagcgaagatcagcttcggcgcacgctggaggacgcggaggcactcttcagcaaatactgcgcgctcactcttaaagactagctccgcgcccttctcgaatttaggcgggagaaaactacgtcatcgccggccgccgcccagcccgcccagccgagatgagcaaagagattcccacgccatacatgtggagctaccagccgcagatgggactcgcggcgggagcggcccaggactactccacccgcatgaactacatgagcgcgggaccccacatgatctcacaggtcaacgggatccgcgcccagcgaaaccaaatactgctggaacaggcggccatcaccgccacgccccgccataatctcaacccccgaaattggcccgccgccctcgtgtaccaggaaaccccctccgccaccaccgtactacttccgcgtgacgcccaggccgaagtccagatgactaactcaggggcgcagctcgcgggcggctttcgtcacggggcgcggccgctccgaccaggtataagacacctgatgatcagaggccgaggtatccagctcaacgacgagtcggtgagctcttcgctcggtctccgtccggacggaactttccagctcgccggatccggccgctcttcgttcacgccccgccaggcgtacctgactctgcagacctcgtcctcggagccccgctccggcggcatcggaaccctccagttcgtggaggagttcgtgccctcggtctacttcaaccccttctcgggacctcccggacgctaccccgaccagttcattccgaactttgacgcggtgaaggactcggcggacggctacgactgaatgtcaggtgtcgaggcagagcagcttcgcctgagacacctcgagcactgccgccgccacaagtgcttcgcccgcggttctggtgagttctgctactttcagctacccgaggagcataccgaggggccggcgcacggcgtccgcctgaccacccagggcgaggttacctgttccctcatccgggagtttaccctccgtcccctgctagtggagcgggagcggggtccctgtgtcctaactatcgcctgcaactgccctaaccctggattacatcaagatctttgctgtcatctctgtgctgagtttaataaacgctgagatcagaatctactggggctcctgtcgccatcctgtgaacgccaccgtcttcacccaccccgaccaggcccaggcgaacctcacctgcggtctgcatcggagggccaagaagtacctcacctggtacttcaacggcaccccctttgtggtttacaacagcttcgacggggacggagtctccctgaaagaccagctctccggtctcagctactccatccacaagaacaccaccctccaactcttccctccctacctgccgggaacctacgagtgcgtcaccggccgctgcacccacctcacccgcctgatcgtaaaccagagctttccgggaacagataactccctcttccccagaacaggaggtgagctcaggaaactccccggggaccagggcggagacgtaccttcgacccttgtggggttaggattttttattaccgggttgctggctcttttaatcaaagtttccttgagatttgttctttccttctacgtgtatgaacacctcaacctccaataactctaccctttcttcggaatcaggtgacttctctgaaatcgggcttggtgtgctgcttactctgttgatttttttccttatcatactcagccttctgtgcctcaggctcgccgcctgctgcgcacacatctatatctactgctggttgctcaagtgcaggggtcgccacccaagatgaacaggtacatggtcctatcgatcctaggcctgctggccctggcggcctgcagcgccgccaaaaaagagattacctttgaggagcccgcttgcaatgtaactttcaagcccgagggtgaccaatgcaccaccctcgtcaaatgcgttaccaatcatgagaggctgcgcatcgactacaaaaacaaaactggccagtttgcggtctatagtgtgtttacgcccggagacccctctaactactctgtcaccgtcttccagggcggacagtctaagatattcaattacactttccctttttatgagttatgcgatgcggtcatgtacatgtcaaaacagtacaacctgtggcctccctctccccaggcgtgtgtggaaaatactgggtcttactgctgtatggctttcgcaatcactacgctcgctctaatctgcacggtgctatacataaaattcaggcagaggcgaatctttatcgatgaaaagaaaatgccttgatcgctaacaccggctttctatctgcagaatgaatgcaatcacctccctactaatcaccaccaccctccttgcgattgcccatgggttgacacgaatcgaagtgccagtggggtccaatgtcaccatggtgggccccgccggcaattccaccctcatgtgggaaaaatttgtccgcaatcaatgggttcatttctgctctaaccgaatcagtatcaagcccagagccatctgcgatgggcaaaatctaactctgatcaatgtgcaaatgatggatgctgggtactattacgggcagcggggagaaatcattaattactggcgaccccacaaggactacatgctgcatgtagtcgaggcacttcccactaccacccccactaccacctctcccaccaccaccaccactactactactactactactactactactactaccactaccgctgcccgccatacccgcaaaagcaccatgattagcacaaagccccctcgtgctcactcccacgccggcgggcccatcggtgcgacctcagaaaccaccgagctttgcttctgccaatgcactaacgccagcgctcatgaactgttcgacctggagaatgaggatgtccagcagagctccgcttgcctgacccaggaggctgtggagcccgttgccctgaagcagatcggtgattcaataattgactcttcttcttttgccactcccgaataccctcccgattctactttccacatcacgggtaccaaagaccctaacctctctttctacctgatgctgctgctctgtatctctgtggtctcttccgcgctgatgttactggggatgttctgctgcctgatctgccgcagaaagagaaaagctcgctctcagggccaaccactgatgcccttcccctaccccccggattttgcagataacaagatatgagctcgctgctgacactaaccgctttactagcctgcgctctaacccttgtcgcttgcgactcgagattccacaatgtcacagctgtggcaggagaaaatgttactttcaactccacggccgatacccagtggtcgtggagtggctcaggtagctacttaactatctgcaatagctccacttcccccggcatatccccaaccaagtaccaatgcaatgccagcctgttcaccctcatcaacgcttccaccctggacaatggactctatgtaggctatgtaccctttggtgggcaaggaaagacccacgcttacaacctggaagttcgccagcccagaaccactacccaagcttctcccaccaccaccaccaccaccaccatcaccagcagcagcagcagcagcagccacagcagcagcagcagattattgactttggttttggccagctcatctgccgctacccaggccatctacagctctgtgcccgaaaccactcagatccaccgcccagaaacgaccaccgccaccaccctacacacctccagcgatcagatgccgaccaacatcacccccttggctcttcaaatgggacttacaagccccactccaaaaccagtggatgcggccgaggtctccgccctcgtcaatgactgggcggggctgggaatgtggtggttcgccataggcatgatggcgctctgcctgcttctgctctggctcatctgctgcctccaccgcaggcgagccagaccccccatctatagacccatcattgtcctgaaccccgataatgatgggatccatagattggatggcctgaaaaacctacttttttcttttacagtatgataaattgagacatgcctcgcattttcttgtacatgttccttctcccaccttttctggggtgttctacgctggccgctgtgtctcacctggaggtagactgcctctcacccttcactgtctacctgctttacggattggtcaccctcactctcatctgcagcctaatcacagtaatcatcgccttcatccagtgcattgattacatctgtgtgcgcctcgcatacttcagacaccacccgcagtaccgagacaggaacattgcccaacttctaagactgctctaatcatgcataagactgtgatctgccttctgatcctctgcatcctgcccaccctcacctcctgccagtacaccacaaaatctccgcgcaaaagacatgcctcctgccgcttcacccaactgtggaatatacccaaatgctacaacgaaaagagcgagctctccgaagcttggctgtatggggtcatctgtgtcttagttttctgcagcactgtctttgccctcataatctacccctactttgatttgggatggaacgcgatcgatgccatgaattaccccacctttcccgcacccgagataattccactgcgacaagttgtacccgttgtcgttaatcaacgccccccatcccctacgcccactgaaatcagctactttaacctaacaggcggagatgactgacgccctagatctagaaatggacggcatcagtaccgagcagcgtctcctagagaggcgcaggcaggcggctgagcaagagcgcctcaatcaggagctccgagatctcgttaacctgcaccagtgcaaaagaggcatcttttgtctggtaaagcaggccaaagtcacctacgagaagaccggcaacagccaccgcctcagttacaaattgcccacccagcgccagaagctggtgctcatggtgggtgagaatcccatcaccgtcacccagcactcggtagagaccgaggggtgtctgcactccccctgtcggggtccagaagacctctgcaccctggtaaagaccctgtgcggtctcagagatttagtcccctttaactaatcaaacactggaatcaataaaaagaatcacttacttaaaatcagacagcaggtctctgtccagtttattcagcagcacctccttcccctcctcccaactctggtactccaaacgccttctggcggcaaacttcctccacaccctgaagggaatgtcagattcttgctcctgtccctccgcacccactatcttcatgttgttgcagatgaagcgcaccaaaacgtctgacgagagcttcaaccccgtgtacccctatgacacggaaagcggccctccctccgtccctttcctcacccctcccttcgtgtctcccgatggattccaagaaagtccccccggggtcctgtctctgaacctggccgagcccctggtcacttcccacggcatgctcgccctgaaaatgggaagtggcctctccctggacgacgctggcaacctcacctctcaagatatcaccaccgctagccctcccctcaaaaaaaccaagaccaacctcagcctagaaacctcatcccccctaactgtgagcacctcaggcgccctcaccgtagcagccgccgctcccctggcggtggccggcacctccctcaccatgcaatcagaggcccccctgacagtacaggatgcaaaactcaccctggccaccaaaggccccctgaccgtgtctgaaggcaaactggccttgcaaacatcggccccgctgacggccgctgacagcagcaccctcacagtcagtgccacaccaccccttagcacaagcaatggcagcttgggtattgacatgcaagcccccatttacaccaccaatggaaaactaggacttaactttggcgctcccctgcatgtggtagacagcctaaatgcactgactgtagttactggccaaggtcttacgataaacggaacagccctacaaactagagtctcaggtgccctcaactatgacacatcaggaaacctagaattgagagctgcagggggtatgcgagttgatgcaaatggtcaacttatccttgatgtagcttacccatttgatgcacaaaacaatctcagccttaggcttggacagggacccctgtttgttaactctgcccacaacttggatgttaactacaacagaggcctctacctgttcacatctggaaataccaaaaagctagaagttaatatcaaaacagccaagggtctcatttatgatgacactgctatagcaatcaatgcgggtgatgggctacagtttgactcaggctcagatacaaatccattaaaaactaaacttggattaggactggattatgactccagcagagccataattgctaaactgggaactggcctaagctttgacaacacaggtgccatcacagtaggcaacaaaaatgatgacaagcttaccttgtggaccacaccagacccatcccctaactgtagaatctattcagagaaagatgctaaattcacacttgttttgactaaatgcggcagtcaggtgttggccagcgtttctgttttatctgtaaaaggtagccttgcgcccatcagtggcacagtaactagtgctcagattgtcctcagatttgatgaaaatggagttctactaagcaattcttcccttgaccctcaatactggaactacagaaaaggtgaccttacagagggcactgcatataccaacgcagtgggatttatgcccaacctcacagcatacccaaaaacacagagccaaactgctaaaagcaacattgtaagtcaggtttacttgaatggggacaaatccaaacccatgaccctcaccattaccctcaatggaactaatgaaacaggagatgccacagtaagcacttactccatgtcattctcatggaactggaatggaagtaattacattaatgaaacgttccaaaccaactccttcaccttctcctacatcgcccaagaataaaaagcatgacgctgttgatttgattcaatgtgtttctgttttattttcaagcacaacaaaatcattcaagtcattcttccatcttagcttaatagacacagtagcttaatagacccagtagtgcaaagccccattctagcttataactagtggagaagtactcgcctacatgggggtagagtcataatcgtgcatcaggatagggcggtggtgctgcagcagcgcgcgaataaactgctgccgccgccgctccgtcctgcaggaatacaacatggcagtggtctcctcagcgatgattcgcaccgcccgcagcataaggcgccttgtcctccgggcacagcagcgcaccctgatctcacttaaatcagcacagtaactgcagcacagcaccacaatattgttcaaaatcccacagtgcaaggcgctgtatccaaagctcatggcggggaccacagaacccacgtggccatcataccacaagcgcaggtagattaagtggcgacccctcataaacacgctggacataaacattacctcttttggcatgttgtaattcaccacctcccggtaccatataaacctctgattaaacatggcgccatccaccaccatcctaaaccagctggccaaaacctgcccgccggctatacactgcagggaaccgggactggaacaatgacagtggagagcccaggactcgtaaccatggatcatcatgctcgtcatgatatcaatgttggcacaacacaggcacacgtgcatacacttcctcaggattacaagctcctcccgcgttagaaccatatcccagggaacaacccattcctgaatcagcgtaaatcccacactgcagggaagacctcgcacgtaactcacgttgtgcattgtcaaagtgttacattcgggcagcagcggatgatcctccagtatggtagcgcgggtttctgtctcaaaaggaggtagacgatccctactgtacggagtgcgccgagacaaccgagatcgtgttggtcgtagtgtcatgccaaatggaacgccggacgtagtcatatttcctgaagtcttagatctctcaacgcagcaccagcaccaacacttcgcagtgtaaaaggccaagtgccgagagagtatatataggaataaaaagtgacgtaaacgggcaaagtccaaaaaacgcccagaaaaaccgcacgcgaacctacgccccgaaacgaaagccaaaaaacactagacactcccttccggcgtcaacttccgctttcccacgctacgtcacttgccccagtcaaacaaactacatatcccgaacttccaagtcgccacgcccaaaacaccgcctacacctccccgcccgccggcccgcccccaaacccgcctcccgccccgcgccccgccccgcgccgcccatctcattatcatattggcttcaatccaaaataaggtatattattgatgatggtttaaacggatcctctagagtcgacctgcaggcatgcaagcttgagtataacccccttgcggccgcccgggccgtcgaccaattctcatgtttgacagcttatcatcgaatttctgccattcatccgcttattatcacttattcaggcgtagcaaccaggcgtttaagggcaccaataactgccttaaaaaaattacgccccgccctgccactcatcgcagtactgttgtaattcattaagcattctgccgacatggaagccatcacaaacggcatgatgaacctgaatcgccagcggcatcagcaccttgtcgccttgcgtataatatttgcccatggtgaaaacgggggcgaagaagttgtccatattggccacgtttaaatcaaaactggtgaaactcacccagggattggctgagacgaaaaacatattctcaataaaccctttagggaaataggccaggttttcaccgtaacacgccacatcttgcgaatatatgtgtagaaactgccggaaatcgtcgtggtattcactccagagcgatgaaaacgtttcagtttgctcatggaaaacggtgtaacaagggtgaacactatcccatatcaccagctcaccgtctttcattgccatacggaattccggatgagcattcatcaggcgggcaagaatgtgaataaaggccggataaaacttgtgcttatttttctttacggtctttaaaaaggccgtaatatccagctgaacggtctggttataggtacattgagcaactgactgaaatgcctcaaaatgttctttacgatgccattgggatatatcaacggtggtatatccagtgatttttttctccattttagcttccttagctcctgaaaatctcgataactcaaaaaatacgcccggtagtgatcttatttcattatggtgaaagttggaacctcttacgtgccgatcaacgtctcattttcgccaaaagttggcccagggcttcccggtatcaacagggacaccaggatttatttattctgcgaagtgatcttccgtcacaggtatttattcgcgataagctcatggagcggcgtaaccgtcgcacaggaaggacagagaaagcgcggatctgggaagtgacggacagaacggtcaggacctggattggggaggcggttgccgccgctgctgctgacggtgtgacgttctctgttccggtcacaccacatacgttccgccattcctatgcgatgcacatgctgtatgccggtataccgctgaaagttctgcaaagcctgatgggacataagtccatcagttcaacggaagtctacacgaaggtttttgcgctggatgtggctgcccggcaccgggtgcagtttgcgatgccggagtctgatgcggttgcgatgctgaaacaattatcctgagaataaatgccttggcctttatatggaaatgtggaactgagtggatatgctgtttttgtctgttaaacagagaagctggctgttatccactgagaagcgaacgaaacagtcgggaaaatctcccattatcgtagagatccgcattattaatctcaggagcctgtgtagcgtttataggaagtagtgttctgtcatgatgcctgcaagcggtaacgaaaacgatttgaatatgccttcaggaacaatagaaatcttcgtgcggtgttacgttgaagtggagcggattatgtcagcaatggacagaacaacctaatgaacacagaaccatgatgtggtctgtccttttacagccagtagtgctcgccgcagtcgagcgacagggcgaagccctcgagtgagcgaggaagcaccagggaacagcacttatatattctgcttacacacgatgcctgaaaaaacttcccttggggttatccacttatccacggggatatttttataattattttttttatagtttttagatcttcttttttagagcgccttgtaggcctttatccatgctggttctagagaaggtgttgtgacaaattgccctttcagtgtgacaaatcaccctcaaatgacagtcctgtctgtgacaaattgcccttaaccctgtgacaaattgccctcagaagaagctgttttttcacaaagttatccctgcttattgactcttttttatttagtgtgacaatctaaaaacttgtcacacttcacatggatctgtcatggcggaaacagcggttatcaatcacaagaaacgtaaaaatagcccgcgaatcgtccagtcaaacgacctcactgaggcggcatatagtctctcccgggatcaaaaacgtatgctgtatctgttcgttgaccagatcagaaaatctgatggcaccctacaggaacatgacggtatctgcgagatccatgttgctaaatatgctgaaatattcggattgacctctgcggaagccagtaaggatatacggcaggcattgaagagtttcgcggggaaggaagtggttttttatcgccctgaagaggatgccggcgatgaaaaaggctatgaatcttttccttggtttatcaaacgtgcgcacagtccatccagagggctttacagtgtacatatcaacccatatctcattcccttctttatcgggttacagaaccggtttacgcagtttcggcttagtgaaacaaaagaaatcaccaatccgtatgccatgcgtttatacgaatccctgtgtcagtatcgtaagccggatggctcaggcatcgtctctctgaaaatcgactggatcatagagcgttaccagctgcctcaaagttaccagcgtatgcctgacttccgccgccgcttcctgcaggtctgtgttaatgagatcaacagcagaactccaatgcgcctctcatacattgagaaaaagaaaggccgccagacgactcatatcgtattttccttccgcgatatcacttccatgacgacaggatagtctgagggttatctgtcacagatttgagggtggttcgtcacatttgttctgacctactgagggtaatttgtcacagttttgctgtttccttcagcctgcatggattttctcatactttttgaactgtaatttttaaggaagccaaatttgagggcagtttgtcacagttgatttccttctctttcccttcgtcatgtgacctgatatcgggggttagttcgtcatcattgatgagggttgattatcacagtttattactctgaattggctatccgcgtgtgtacctctacctggagtttttcccacggtggatatttcttcttgcgctgagcgtaagagctatctgacagaacagttcttctttgcttcctcgccagttcgctcgctatgctcggttacacggctgcggcgagcgctagtgataataagtgactgaggtatgtgctcttcttatctccttttgtagtgttgctcttattttaaacaactttgcggttttttgatgactttgcgattttgttgttgctttgcagtaaattgcaagatttaataaaaaaacgcaaagcaatgattaaaggatgttcagaatgaaactcatggaaacacttaaccagtgcataaacgctggtcatgaaatgacgaaggctatcgccattgcacagtttaatgatgacagcccggaagcgaggaaaataacccggcgctggagaataggtgaagcagcggatttagttggggtttcttctcaggctatcagagatgccgagaaagcagggcgactaccgcacccggatatggaaattcgaggacgggttgagcaacgtgttggttatacaattgaacaaattaatcatatgcgtgatgtgtttggtacgcgattgcgacgtgctgaagacgtatttccaccggtgatcggggttgctgcccataaaggtggcgtttacaaaacctcagtttctgttcatcttgctcaggatctggctctgaaggggctacgtgttttgctcgtggaaggtaacgacccccagggaacagcctcaatgtatcacggatgggtaccagatcttcatattcatgcagaagacactctcctgcctttctatcttggggaaaaggacgatgtcacttatgcaataaagcccacttgctggccggggcttgacattattccttcctgtctggctctgcaccgtattgaaactgagttaatgggcaaatttgatgaaggtaaactgcccaccgatccacacctgatgctccgactggccattgaaactgttgctcatgactatgatgtcatagttattgacagcgcgcctaacctgggtatcggcacgattaatgtcgtatgtgctgctgatgtgctgattgttcccacgcctgctgagttgtttgactacacctccgcactgcagtttttcgatatgcttcgtgatctgctcaagaacgttgatcttaaagggttcgagcctgatgtacgtattttgcttaccaaatacagcaatagtaatggctctcagtccccgtggatggaggagcaaattcgggatgcctggggaagcatggttctaaaaaatgttgtacgtgaaacggatgaagttggtaaaggtcagatccggatgagaactgtttttgaacaggccattgatcaacgctcttcaactggtgcctggagaaatgctctttctatttgggaacctgtctgcaatgaaattttcgatcgtctgattaaaccacgctgggagattagataatgaagcgtgcgcctgttattccaaaacatacgctcaatactcaaccggttgaagatacttcgttatcgacaccagctgccccgatggtggattcgttaattgcgcgcgtaggagtaatggctcgcggtaatgccattactttgcctgtatgtggtcgggatgtgaagtttactcttgaagtgctccggggtgatagtgttgagaagacctctcgggtatggtcaggtaatgaacgtgaccaggagctgcttactgaggacgcactggatgatctcatcccttcttttctactgactggtcaacagacaccggcgttcggtcgaagagtatctggtgtcatagaaattgccgatgggagtcgccgtcgtaaagctgctgcacttaccgaaagtgattatcgtgttctggttggcgagctggatgatgagcagatggctgcattatccagattgggtaacgattatcgcccaacaagtgcttatgaacgtggtcagcgttatgcaagccgattgcagaatgaatttgctggaaatatttctgcgctggctgatgcggaaaatatttcacgtaagattattacccgctgtatcaacaccgccaaattgcctaaatcagttgttgctcttttttctcaccccggtgaactatctgcccggtcaggtgatgcacttcaaaaagcctttacagataaagaggaattacttaagcagcaggcatctaaccttcatgagcagaaaaaagctggggtgatatttgaagctgaagaagttatcactcttttaacttctgtgcttaaaacgtcatctgcatcaagaactagtttaagctcacgacatcagtttgctcctggagcgacagtattgtataagggcgataaaatggtgcttaacctggacaggtctcgtgttccaactgagtgtatagagaaaattgaggccattcttaaggaacttgaaaagccagcaccctgatgcgaccacgttttagtctacgtttatctgtctttacttaatgtcctttgttacaggccagaaagcataactggcctgaatattctctctgggcccactgttccacttgtatcgtcggtctgataatcagactgggaccacggtcccactcgtatcgtcggtctgattattagtctgggaccacggtcccactcgtatcgtcggtctgattattagtctgggaccacggtcccactcgtatcgtcggtctgataatcagactgggaccacggtcccactcgtatcgtcggtctgattattagtctgggaccatggtcccactcgtatcgtcggtctgattattagtctgggaccacggtcccactcgtatcgtcggtctgattattagtctggaaccacggtcccactcgtatcgtcggtctgattattagtctgggaccacggtcccactcgtatcgtcggtctgattattagtctgggaccacgatcccactcgtgttgtcggtctgattatcggtctgggaccacggtcccacttgtattgtcgatcagactatcagcgtgagactacgattccatcaatgcctgtcaagggcaagtattgacatgtcgtcgtaacctgtagaacggagtaacctcggtgtgcggttgtatgcctgctgtggattgctgctgtgtcctgcttatccacaacattttgcgcacggttatgtggacaaaatacctggttacccaggccgtgccggcacgctcggtacccggggatcctcgtttaaac

SEQ ID NO: 53 - DNA, 41545 bp, Artificial Sequence
  source: /note="Description of Artificial Sequence: Synthetic polynucleotide"
  modified_base (16144)..(16144): a, c, t, g, unknown or other
catcatcaataatataccttattttggattgaagccaatatgataatgagatgggcggcgcggggcggggcgcggggcgggaggcgggtttgggggcgggccggcgggcggggcggtgtggcggaagtggactttgtaagtgtggcggatgtgacttgctagtgccgggcgcggtaaaagtgacgttttccgtgcgcgacaacgcccccgggaagtgacatttttcccgcggtttttaccggatgttgtagtgaatttgggcgtaaccaagtaagatttggccattttcgcgggaaaactgaaacggggaagtgaaatctgattaattttgcgttagtcataccgcgtaatatttgtctagggccgagggactttggccgattacgtggaggactcgcccaggtgttttttgaggtgaatttccgcgttccgggtcaaagtctgcgttttattattataggatatcccattgcatacgttgtatccatatcataatatgtacatttatattggctcatgtccaacattaccgccatgttgacattgattattgactagttattaatagtaatcaattacggggtcattagttcatagcccatatatggagttccgcgttacataacttacggtaaatggcccgcctggctgaccgcccaacgacccccgcccattgacgtcaataatgacgtatgttcccatagtaacgccaatagggactttccattgacgtcaatgggtggagtatttacggtaaactgcccacttggcagtacatcaagtgtatcatatgccaagtacgccccctattgacgtcaatgacggtaaatggcccgcctggcattatgcccagtacatgaccttatgggactttcctacttggcagtacatctacgtattagtcatcgctattaccatggtgatgcggttttggcagtacatcaatgggcgtggatagcggtttgactcacggggatttccaagtctccaccccattgacgtcaatgggagtttgttttggcaccaaaatcaacgggactttccaaaatgtcgtaacaactccgccccattgacgcaaatgggcggtaggcgtgtacggtgggaggtctatataagcagagctctccctatcagtgatagagatctccctatcagtgatagagatcgtcgacgagctcgtttagtgaaccgtcagatcgcctggagacgccatccacgctgttttgacctccatagaagacaccgggaccgatccagcctccgcggccgggaacggtgcattggaacgcggattccccgtgccaagagtgagatcttccgtttatctaggtaccagatatcgccaccatgtccgaggactttctgattctgatcgccatcctggtgatcgtgattctcgtgggcacaatcacaaccctggtgggcgccatcggcggcattagggccaggaggagcttcctcttcatttgcatcttcttcctgttcctctccctcttcctgacaatcctcgccctgctgctgggcttcagctggctcctgctggtggccatcctgttctgggtgctctggctggtcatcctcattctgctgctgctggtgtaccctattcctcaccaccccctgcccacctccctcaggtttagaatgaagcagagggtgagcagcgaccccacaggttctgacagaagccctcagggcagccataatagcctgaactcccccgatgaggaggaccccaaggatgacaccaagcaacctctgtgcaacatgacccagggcggacctcccgtcaatggacagctcctcggacaacatgctcaatgcccccctcactatccctgctgccatattcagcatcccgacggagaggattccgatggagacgatggcaagtcctggggcgatgccggagaggaagacaatggccctaacgaccctaacaccgccagcaccagagagtccatttacgaggacctcagataccccacaagggacgccaatggcgagtatgagaacgtgggatacccccctagggacggagatgcccctcataggctcggagagcctgtgtatgacgatgtggagcaagccaccgctaacgaggtgagaatctcccctctgttcagactgccctacggaagcgctttcggacctggcccccagcctggacccattctggagagctccacatggggctttctggtcttcacacagacctccctgttcgccgacgacattgccgacgctattagggactactgcacaacccaccctggccccacaaggaacacccaggtggtcctcatgaacttcgagggcagcggagtgcccctgcctatgttttttccccctggagaggagacagaagagcagagagagggcgatagagctagcgactccgacgagtccgaagacgctcagatcctgaccgtgttctgcctgttttgccagtggacactctttatctgcctgggaatcaggatgatctgtaactggaggggcaaactcaccaggatcatctgcctgaagttctgcctctacggactgatttccgcctccctgtccttcggctggtacgcttttctgaaggaagtgaccctccccaccacagccaccgttgatcctaggcaactccccctgttcctcttcatcctgagctccgtgctggtgattctcgccatcatgatggagtttcaaacatcctccagcctcttcgctgctctgttcgtgattatcgccggaatgctgtgcgtcacagtgggcgtgatttttctgctggctggcgtcaagcctctcctgagcggcatgatctgcgcctccggcatcacaatgctcgtgctcggcgtcgtgctgctggtggtgtgcaccagagatgagcacgctatttccgccagccaccatgctagcgatggctccgtgaatcagcagaaggaaaatcagccccagaccctggaggaatgcaagacagatcaggagaggaagaggtacaggaacaggctggcctccaggaggtgtagagctaagttcaggaaccagctggaacattttaggacagtcgccgctgctaagacagaggagaacaacaggctcagggtgctcatcaggcagatgtgtcctacactggacgtggaatccatcgtcccctccacctccgccggctaccacgagcctctgaatcacctgacccacagccccagcccttgtcatcacagggatgaacccccctccagaagccccagccctcaacccaccgtctccgagcagtcccagcagtcccccaggcagcagagccctcaaggcacatcccagggttctacaagacctcaggtgcctggaggcgccaccaccagaaaaagaggcggcgtgagaggccaacctgccaagtgtcacggcaagtacaccacaaccgccgagggactgaccgctctcctgaataggaggcacagccccaggacatccaacgagggcaggtggatgaatggagtcatggctgtgaacctctccaaatggcccctgtacagcctgaggagagccctggccctcgccatggctcctagaaggaggctctccggccctccctggctgacagtgctgctgctgctgtccacactgagcgtggccgccctgctgattctcttcctgattttcagcgccggcgccaccattagcacagaagccagcctgctggtcctgctcctgctgtttgtgaccctgctgctgcctctcctgtcctccaacggactccagctccctgccgccctgattctgatccagtgtttcctcctggccgctgattatctcgcctacctgattctgcctaccattatgcccaggggcagaagcacaggaaggaagggcagggacacagagaaagagaggagcagatcccctctcagagctcctggcggttctgatggacccagcacaagggctggctgtggagccggaccctgtcagctgagcagccccatcgccggaaacaacggcaatgaaggcggcgagggcgacgactacaagagctggaggaagcccgaggaagaggacaacggccccaatgaccccaataccaacaacaggattgaggatggagacggcgacgacggaaaatcctggaggaatcctgaggaggaggataacagaaagcaggacaggctgggcaccaagcctttcatggacctcgacggaaccggcggaggcgagggctacagccagatggtccctatcgccaccgcccccggaagcggccacgccgctacctatcaggatctccaggccgccccttacatcatctggcctctccagaccgattgccagcctgtggctaccaccttcgcctcccccggacagatccagtggtatacaagcgccgtcccccagcccacagagcattgctcccagtttacaaacgctcccaccgtcaaccagcagcagcctattagccaaccccagcccgaaaatccccctgctttcacctttacccagcccgcttccatcattcccggcgtcattagcgcctccaacctgaacgtgagcgcttcccctatcatccctagcgaccatgtcctccccatcattacctccgtgaccagcctcgcccaacctaataacatggccggccactggtatgagagcgtgattcccggcctgttcctctgccccctgatcctcccttccctgttctggatttgctccctgctgaccttcctggtgggccacggagccaatattgtgagcgccgtcctgttcctcgtgctggcttggtgtctcctcattgccaactggaacgtgacaagagaggacttcgtgtccggcaggagaagctccatgagcagcctgtccgtggccgcttccaccgccacagccatgttcgccagcttcctcaccctgagctttgatggcctgggcctgctgctgtttggcaccgccctggtgatccagacaatttacgtgctgtatctggtggtcatggagatcaccgtgtggatcatgatgtttaggtatctccacttttggatcaccctgctgttcctgctgagccccattattctctccgtcgcctgtctcatcatccaatcctccgccctgctgatcgaggctgtggtcgtcaccaccatcacagtcctggccatttttctgtggctccctcctcaaggcgctgaggccgatctcggcaccgccctgctgattctgaataccgccctgtgcctggtcgtgctgatcctgaccgctatccctacatgatgatgagcggccgcgatctgctgtgccttctagttgccagccatctgttgtttgcccctcccccgtgccttccttgaccctggaaggtgccactcccactgtcctttcctaataaaatgaggaaattgcatcgcattgtctgagtaggtgtcattctattctggggggtggggtggggcaggacagcaagggggaggattgggaagacaatagcaggcatgctggggatgcggtgggctctatggccgatcagcgatcgctgaggtgggtgagtgggcgtggcctggggtggtcatgaaaatatataagttgggggtcttagggtctctttatttgtgttgcagagaccgccggagccatgagcgggagcagcagcagcagcagtagcagcagcgccttggatggcagcatcgtgagcccttatttgacgacgcggatgccccactgggccggggtgcgtcagaatgtgatgggctccagcatcgacggccgacccgtcctgcccgcaaattccgccacgctgacctatgcgaccgtcgcggggacgccgttggacgccaccgccgccgccgccgccaccgcagccgcctcggccgtgcgcagcctggccacggactttgcattcctgggaccactggcgacaggggctacttctcgggccgctgctgccgccgttcgcgatgacaagctgaccgccctgctggcgcagttggatgcgcttactcgggaactgggtgacctttctcagcaggtcatggccctgcgccagcaggtctcctccctgcaagctggcgggaatgcttctcccacaaatgccgtttaagataaataaaaccagactctgtttggattaaagaaaagtagcaagtgcattgctctctttatttcataattttccgcgcgcgataggccctagaccagcgttctcggtcgttgagggtgcggtgtatcttctccaggacgtggtagaggtggctctggacgttgagatacatgggcatgagcccgtcccgggggtggaggtagcaccactgcagagcttcatgctccggggtggtgttgtagatgatccagtcgtagcaggagcgctgggcatggtgcctaaaaatgtccttcagcagcaggccgatggccagggggaggcccttggtgtaagtgtttacaaaacggttaagttgggaagggtgcattcggggagagatgatgtgcatcttggactgtatttttagattggcgatgtttccgcccagatcccttctgggattcatgttgtgcaggaccaccagtacagtgtatccggtgcacttggggaatttgtcatgcagcttagagggaaaagcgtggaagaacttggagacgcctttgtggcctcccagattttccatgcattcgtccatgatgatggcaatgggcccgcgggaggcagcttgggcaaagatatttctggggtcgctgacgtcgtagttgtgttccagggtgaggtcgtcataggccatttttacaaagcgcgggcggagggtgcccgactgggggatgatggtcccctctggccctggggcgtagttgccctcgcagatctgcatttcccaggccttaatctcggaggggggaatcatatccacctgcggggcgatgaagaaaacggtttccggagccggggagattaactgggatgagagcaggtttctaagcagctgtgattttccacaaccggtgggcccataaataacacctataaccggttgcagctggtagtttagagagctgcagctgccgtcgtcccggaggaggggggccacctcgttgagcatgtccctgacgcgcatgttctccccgaccagatccgccagaaggcgctcgccgcccagggacagcagctcttgcaaggaagcaaagtttttcagcggcttgaggccgtccgccgtgggcatgtttttcagggtctggctcagcagctccaggcggtcccagagctcggtgacgtgctctacggcatctctatccagcatatctcctcgtttcgcgggttggggcgactttcgctgtagggcaccaagcggtggtcgtccagcggggccagagtcatgtccttccatgggcgcagggtcctcgtcagggtggtctgggtcacggtgaaggggtgcgctccgggctgagcgcttgccaaggtgcgcttgaggctggttctgctggtgctgaagcgctgccggtcttcgccctgcgcgtcggccaggtagcatttgaccatggtgtcatagtccagcccctccgcggcgtgtcccttggcgcgcagcttgcccttggaggtggcgccgcacgaggggcagagcaggctcttgagcgcgtagagcttgggggcgaggaagaccgattcgggggagtaggcgtccgcgccgcagaccccgcacacggtctcgcactccaccagccaggtgagctcggggcgcgccgggtcaaaaaccaggtttcccccatgctttttgatgcgtttcttacctcgggtctccatgaggtggtgtccccgctcggtgacgaagaggctgtccgtgtctccgtagaccgacttgaggggtcttttctccaggggggtccctcggtcttcctcgtagaggaactcggaccactctgagacgaaggcccgcgtccaggccaggacgaaggaggctatgtgggaggggtagcggtcgttgtccactagggggtccaccttctccaaggtgtgaagacacatgtcgccttcctcggcgtccaggaaggtgattggcttgtaggtgtaggccacgtgaccgggggttcctgacgggggggtataaaagggggtgggggcgcgctcgtcgtcactctcttccgcatcgctgtctgcgagggccagctgctggggtgagtattccctctcgaaggcgggcatgacctccgcgctgaggttgtcagtttccaaaaacgaggaggatttgatgttcacctgtcccgaggtgatacctttgagggtacccgcgtccatctggtcagaaaacacgatctttttattgtccagcttggtggcgaacgacccgtagagggcgttggagagcagcttggcgatggagcgcagggtctggttcttgtccctgtcggcgcgctccttggccgcgatgttgagctgcacgtactcgcgcgcgacgcagcgccactcggggaagacggtggtgcgctcgtcgggcaccaggcgcacgcgccagccgcggttgtgcagggtgaccaggtccacgctggtggcgacctcgccgcgcaggcgctcgttggtccagcagagacggccgcccttgcgcgagcagaaggggggcagggggtcgagctgggtctcgtccggggggtccgcgtccacggtgaaaaccccggggcgcaggcgcgcgtcgaagtagtctatcttgcaaccttgcatgtccagcgcctgctgccagtcgcgggcggcgagcgcgcgctcgtaggggttgagcggcgggccccagggcatggggtgggtgagtgcggaggcgtacatgccgcagatgtcatagacgtagaggggctcccgcaggaccccgatgtaggtggggtagcagcggccgccgcggatgctggcgcgcacgtagtcatacagctcgtgcgagggggcgaggaggtcggggcccaggttggtgcgggcggggcgctccgcgcggaagacgatctgcctgaagatggcatgcgagttggaagagatggtggggcgctggaagacgttgaagctggcgtcctgcaggccgacggcgtcgcgcacgaaggaggcgtaggagtcgcgcagcttgtgtaccagctcggcggtgacctgcacgtcgagcgcgcagtagtcgagggtctcgcggatgatgtcatatttagcctgccccttctttttccacagctcgcggttgaggacaaactcttcgcggtctttccagtactcttggatcgggaaaccgtccggttccgaacggtaagagcctagcatgtagaactggttgacggcctggtaggcgcagcagcccttctccacggggagggcgtaggcctgcgcggccttgcggagcgaggtgtgggtcagggcgaaggtgtccctgaccatgactttgaggtactggtgcttgaagtcggagtcgtcgcagccgccccgctcccagagcgagaagtcggtgcgcttcttggagcgggggttgggcagagcgaaggtgacatcgttgaagaggattttgcccgcgcggggcatgaagttgcgggtgatgcggaagggccccggcacttcagagcggttgttgatgacctgggcggcgagcacgatctcgtcgaagccgttgatgttgtggcccacgatgtagagttccaggaagcggggccggccctttacggtgggcagcttctttagctcttcgtaggtgagctcctcgggcgaggcgaggccgtgctcggccagggcccagtccgcgaggtgcgggttgtctctgaggaaggacttccagaggtcgcgggccaggagggtctgcaggcggtctctgaaggtcctgaactggcggcccacggccattttttcgggggtgatgcagtagaaggtgagggggtcttgctgccagcggtcccagtcgagctgcagggcgaggtcgcgcgcggcggtgaccaggcgctcgtcgcccccgaatttcatgaccagcatgaagggcacgagctgctttccgaaggcccccatccaagtgtaggtctctacatcgtaggtgacaaagaggcgctccgtgcgaggatgcgagccgatcgggaagaactggatctcccgccaccagttggaggagtggctgttgatgtggtggaagtagaagtcccgtcgccgggccgaacactcgtgctggcttttgtaaaagcgagcgcagtactggcagcgctgcacgggctgtacctcatgcacgagatgcacctttcgcccgcgcacgaggaagccgaggggaaatctgagccccccgcctggctcgcggcatggctggttctcttctactttggatgcgtgtccgtctccgtctggctcctcgaggggtgttacggtggagcggaccaccacgccgcgcgagccgcaggtccagatatcggcgcgcggcggtcggagtttgatgacgacatcgcgcagctgggagctgtccatggtctggagctcccgcggcggcggcaggtcagccgggagttcttgcaggttcacctcgcagagtcgggccagggcgcggggcaggtctaggtggtacctgatctctaggggcgtgttggtggcggcgtcgatggcttgcaggagcccgcagccccggggggcgacgacggtgccccgcggggtggtggtggtggtggcggtgcagctcagaagcggtgccgcgggcgggcccccggaggtagggggggctccggtcccgcgggcaggggcggcagcggcacgtcggcgtggagcgcgggcaggagttggtgctgtgcccggaggttgctggcgaaggcgacgacgcggcggttgatctcctggatctggcgcctctgcgtgaagacgacgggcccggtgagcttgaacctgaaagagagttcgacagaatcaatctcggtgtcattgaccgcggcctggcgcaggatctcctgcacgtctcccgagttgtcttggtaggcgatctcggccatgaactgctcgatctcttcctcctggaggtctccgcgtccggcgcgttccacggtggccgccaggtcgttggagatgcgccccatgagctgcgagaaggcgttgagtccgccctcgttccagactcggctgtagaccacgcccccctggtcatcgcgggcgcgcatgaccacctgcgcgaggttgagctccacgtgccgcgcgaagacggcgtagttgcgcagacgctggaagaggtagttgagggtggtggcggtgtgctcggccacgaagaagttcatgacccagcggcgcaacgtggattcgttgatgtcccccaaggcctccagccgttccatggcctcgtagaagtccacggcgaagttgaaaaactgggagttgcgcgccgacacggtcaactcctcctccagaagacggatgagctcggcgacggtgtcgcgcacctcgcgctcgaaggctatggggatctcttcctccgctagcatcaccacctcctcctcttcctcctcttctggcacttccatgatggcttcctcctcttcggggggtggcggcggcggcggtgggggagggggcgctctgcgccggcggcggcgcaccgggaggcggtccacgaagcgcgcgatcatctccccgcggcggcggcgcatggtctcggtgacggcgcggccgttctcccgggggcgcagttggaagacgccgccggacatctggtgctggggcgggtggccgtgaggcagcgagacggcgctgacgatgcatctcaacaattgctgcgtaggtacgccgccgagggacctgagggagtccatatccaccggatccgaaaacctttcgaggaaggcgtctaaccagtcgcagtcgcaaggtaggctgagcaccgtggcgggcggcggggggtggggggagtgtctggcggaggtgctgctgatgatgtaattgaagtaggcggacttgacacggcggatggtcgacaggagcaccatgtccttgggtccggcctgctggatgcggaggcggtcggctatgccccaggcttcgttctggcatcggcgcaggtccttgtagtagtcttgcatgagcctttccaccggcacctcttctccttcctcttctgcttcttccatgtctgcttcggccctggggcggcgccgcgcccccctgccccccatgcgcgtgaccccgaaccccctgagcggttggagcagggccaggtcggcgacgacgcgctcggccaggatggcctgctgcacctgcgtgagggtggtttggaagtcatccaagtccacgaagcggtggtaggcgcccgtgttgatggtgtaggtgcagttggccatgacggaccagttgacggtctggtggcccggttgcgacatctcggtgtacctgagtcgcgagtaggcgcgggagtcgaagacgtagtcgttgcaagtccgcaccaggtactggtagcccaccaggaagtgcggcggcggctggcggtagaggggccagcgcagggtggcgggggctccgggggccaggtcttccagcatgaggcggtggtaggcgtagatgtacctggacatccaggtgatacccgcggcggtggtggaggcgcgcgggaagtcgcgcacccggttccagatgttgcgcaggggcagaaagtgctccatggtaggcgtgctctgtccagtcagacgcgcgcagtcgttgatactctagaccagggaaaacgaaagccggtcagcgggcactcttccgtggtctggtgaatagatcgcaagggtatcatggcggagggcctcggttcgagccccgggtccgggccggacggtccgccatgatccacgcggttaccgcccgcgtgtcgaacccaggtgtgcgacgtcagacaacggtggagtgttccttttggcgtttttctggccgggcgccggcgccgcgtaagagactaagccgcgaaagcgaaagcagtaagtggctcgctccccgtagccggagggatccttgctaagggttgcgttgcggcgaaccccggttcgaatcccgtactcgggccggccggacccgcggctaaggtgttggattggcctccccctcgtataaagaccccgcttgcggattgactccggacacggggacgagccccttttatttttgctttccccagatgcatccggtgctgcggcagatgcgccccccgccccagcagcagcaacaacaccagcaagagcggcagcaacagcagcgggagtcatgcagggccccctcacccaccctcggcgggccggccacctcggcgtccgcggccgtgtctggcgcctgcggcggcggcggggggccggctgacgaccccgaggagcccccgcggcgcagggccagacactacctggacctggaggagggcgagggcctggcgcggctgggggcgccgtctcccgagcgccacccgcgggtgcagctgaagcgcgactcgcgcgaggcgtacgtgcctcggcagaacctgttcagggaccgcgcgggcgaggagcccgaggagatgcgggacaggaggttcagcgcagggcgggagctgcggcaggggctgaaccgcgagcggctgctgcgcgaggaggactttgagcccgacgcgcggacggggatcagccccgcgcgcgcgcacgtggcggccgccgacctggtgacggcgtacgagcagacggtgaaccaggagatcaacttccaaaagagtttcaacaaccacgtgcgcacgctggtggcgcgcgaggaggtgaccatcgggctgatgcacctgtgggactttgtaagcgcgctggtgcagaaccccaacagcaagcctctgacggcgcagctgttcctgatagtgcagcacagcagggacaacgaggcgtttagggacgcgctgctgaacatcaccgagcccgagggtcggtggctgctggacctgattaacatcctgcagagcatagtggtgcaggagcgcagcctgagcctggccgacaaggtggcggccatcaactactcgatgctgagcctgggcaagttttacgcgcgcaagatctaccagacgccgtacgtgcccatagacaaggaggtgaagatcgacggtttttacatgcgcatggcgctgaaggtgctcaccctgagcgacgacctgggcgtgtaccgcaacgagcgcatccacaaggccgtgagcgtgagccggcggcgcgagctgagcgaccgcgagctgatgcacagcctgcagcgggcgctggcgggcgccggcagcggcgacagggaggcggagtcctacttcgatgcgggggcggacctgcgctgggcgcccagccggcgggccctggaggccgcgggggtccgcgaggactatgacgaggacggcgaggaggatgaggagtacgagctagaggagggcgagtacctggactaaaccgcgggtggtgtttccggtagatgcaagacccgaacgtggtggacccggcgctgcgggcggctctgcagagccagccgtccggccttaactcctcagacgactggcgacaggtcatggaccgcatcatgtcgctgacggcgcgtaacccggacgcgttccggcagcagccgcaggccaacaggctctccgccatcctggaggcggtggtgcctgcgcgctcgaaccccacgcacgagaaggtgctggccatagtgaacgcgctggccgagaacagggccatccgcccggacgaggccgggctggtgtacgacgcgctgctgcagcgcgtggcccgctacaacagcggcaacgtgcagaccaacctggaccggctggtgggggacgtgcgcgaggcggtggcgcagcgcgagcgcgcggatcggcagggcaacctgggctccatggtggcgctgaatgccttcctgagcacgcagccggccaacgtgccgcgggggcaggaagactacaccaactttgtgagcgcgctgcggctgatggtgaccgagaccccccagagcgaggtgtaccagtcgggcccggactacttcttccagaccagcagacagggcctgcagacggtgaacctgagccaggctttcaagaacctgcgggggctgtggggcgtgaaggcgcccaccggcgaccgggcgacggtgtccagcctgctgacgcccaactcgcgcctgctgctgctgctgatcgcgccgttcacggacagcggcagcgtgtcccgggacacctacctggggcacctgctgaccctgtaccgcgaggccatcgggcaggcgcaggtggacgagcacaccttccaggagatcaccagcgtgagccgcgcgctggggcaggaggacacgagcagcctggaggcgactctgaactacctgctgaccaaccggcggcagaagattccctcgctgcacagcctgacctccgaggaggagcgcatcttgcgctacgtgcagcagagcgtgagcctgaacctgatgcgcgacggggtgacgcccagcgtggcgctggacatgaccgcgcgcaacatggaaccgggcatgtacgccgcgcaccggccttacatcaaccgcctgatggactacctgcatcgcgcggcggccgtgaaccccgagtactttaccaacgccatcctgaacccgcactggctcccgccgcccgggttctacagcgggggcttcgaggtcccggagaccaacgatggcttcctgtgggacgacatggacgacagcgtgttctccccgcggccgcaggcgctggcggaagcgtccctgctgcgtcccaagaaggaggaggaggaggaggcgagtcgccgccgcggcagcagcggcgtggcttctctgtccgagctgggggcggcagccgccgcgcgccccgggtccctgggcggcagcccctttccgagcctggtggggtctctgcacagcgagcgcaccacccgccctcggctgctgggcgaggacgagtacctgaataactccctgctgcagccggtgcgggagaaaaacctgcctcccgccttccccaacaacgggatagagagcctggtggacaagatgagcagatggaagacctatgcgcaggagcacagggacgcgcctgcgctccggccgcccacgcggcgccagcgccacgaccggcagcgggggctggtgtgggatgacgaggactccgcggacgatagcagcgtgctggacctgggagggagcggcaacccgttcgcgcacctgcgcccccgcctggggaggatgttttaaaaaaaaaaaaaaaangcaagaagcatgatgcaaaaattaaataaaactcaccaaggccatggcgaccgagcgttggtttcttgtgttcccttcagtatgcggcgcgcggcgatgtaccaggagggacctcctccctcttacgagagcgtggtgggcgcggcggcggcggcgccctcttctccctttgcgtcgcagctgctggagccgccgtacgtgcctccgcgctacctgcggcctacgggggggagaaacagcatccgttactcggagctggcgcccctgttcgacaccacccgggtgtacctggtggacaacaagtcggcggacgtggcctccctgaactaccagaacgaccacagcaattttttgaccacggtcatccagaacaatgactacagcccgagcgaggccagcacccagaccatcaatctggatgaccggtcgcactggggcggcgacctgaaaaccatcctgcacaccaacatgcccaacgtgaacgagttcatgttcaccaataagttcaaggcgcgggtgatggtgtcgcgctcgcacaccaaggaagaccgggtggagctgaagtacgagtgggtggagttcgagctgccagagggcaactactccgagaccatgaccattgacctgatgaacaacgcgatcgtggagcactatctgaaagtgggcaggcagaacggggtcctggagagcgacatcggggtcaagttcgacaccaggaacttccgcctggggctggaccccgtgaccgggctggttatgcccggggtgtacaccaacgaggccttccatcccgacatcatcctgctgcccggctgcggggtggacttcacttacagccgcctgagcaacctcctgggcatccgcaagcggcagcccttccaggagggcttcaggatcacctacgaggacctggaggggggcaacatccccgcgctcctcgatgtggaggcctaccaggatagcttgaaggaaaatgaggcgggacaggaggataccgcccccgccgcctccgccgccgccgagcagggcgaggatgctgctgacaccgcggccgcggacggggcagaggccgaccccgctatggtggtggaggctcccgagcaggaggaggacatgaatgacagtgcggtgcgcggagacaccttcgtcacccggggggaggaaaagcaagcggaggccgaggccgcggccgaggaaaagcaactggcggcagcagcggcggcggcggcgttggccgcggcggaggctgagtctgaggggaccaagcccgccaaggagcccgtgattaagcccctgaccgaagatagcaagaagcgcagttacaacctgctcaaggacagcaccaacaccgcgtaccgcagctggtacctggcctacaactacggcgacccgtcgacgggggtgcgctcctggaccctgctgtgcacgccggacgtgacctgcggctcggagcaggtgtactggtcgctgcccgacatgatgcaagaccccgtgaccttccgctccacgcggcaggtcagcaacttcccggtggtgggcgccgagctgctgcccgtgcactccaagagcttctacaacgaccaggccgtctactcccagctcatccgccagttcacctctctgacccacgtgttcaatcgctttcctgagaaccagattctggcgcgcccgcccgcccccaccatcaccaccgtcagtgaaaacgttcctgctctcacagatcacgggacgctaccgctgcgcaacagcatcggaggagtccagcgagtgaccgttactgacgccagacgccgcacctgcccctacgtttacaaggccttgggcatagtctcgccgcgcgtcctttccagccgcactttttgagcaacaccaccatcatgtccatcctgatctcacccagcaataactccggctggggactgctgcgcgcgcccagcaagatgttcggaggggcgaggaagcgttccgagcagcaccccgtgcgcgtgcgcgggcacttccgcgccccctggggagcgcacaaacgcggccgcgcggggcgcaccaccgtggacgacgccatcgactcggtggtggagcaggcgcgcaactacaggcccgcggtctctaccgtggacgcggccatccagaccgtggtgcggggcgcgcggcggtacgccaagctgaagagccgccggaagcgcgtggcccgccgccaccgccgccgacccggggccgccgccaaacgcgccgccgcggccctgcttcgccgggccaagcgcacgggccgccgcgccgccatgagggccgcgcgccgcttggccgccggcatcaccgccgccaccatggccccccgtacccgaagacgcgcggccgccgccgccgccgccgccatcagtgacatggccagcaggcgccggggcaacgtgtactgggtgcgcgactcggtgaccggcacgcgcgtgcccgtgcgcttccgccccccgcggacttgagatgatgtgaaaaaacaacactgagtctcctgctgttgtgtgtatcccagcggcggcggcgcgcgcagcgtcatgtccaagcgcaaaatcaaagaagagatgctccaggtcgtcgcgccggagatctatgggcccccgaagaaggaagagcaggattcgaagccccgcaagataaagcgggtcaaaaagaaaaagaaagatgatgacgatgccgatggggaggtggagttcctgcgcgccacggcgcccaggcgcccggtgcagtggaagggccggcgcgtaaagcgcgtcctgcgccccggcaccgcggtggtcttcacgcccggcgagcgctccacccggactttcaagcgcgtctatgacgaggtgtacggcgacgaagacctgctggagcaggccaacgagcgcttcggagagtttgcttacgggaagcgtcagcgggcgctggggaaggaggacctgctggcgctgccgctggaccagggcaaccccacccccagtctgaagcccgtgaccctgcagcaggtgctgccgagcagcgcaccctccgaggcgaagcggggtctgaagcgcgagggcggcgacctggcgcccaccgtgcagctcatggtgcccaagcggcagaggctggaggatgtgctggagaaaatgaaagtagaccccggtctgcagccggacatcagggtccgccccatcaagcaggtggcgccgggcctcggcgtgcagaccgtggacgtggtcatccccaccggcaactcccccgccgccgccaccactaccgctgcctccacggacatggagacacagaccgatcccgccgcagccgcagccgcagccgccgccgcgacctcctcggcggaggtgcagacggacccctggctgccgccggcgatgtcagctccccgcgcgcgtcgcgggcgcaggaagtacggcgccgccaacgcgctcctgcccgagtacgccttgcatccttccatcgcgcccacccccggctaccgaggctatacctaccgcccgcgaagagccaagggttccacccgccgtccccgccgacgcgccgccgccaccacccgccgccgccgccgcagacgccagcccgcactggctccagtctccgtgaggaaagtggcgcgcgacggacacaccctggtgctgcccagggcgcgctaccaccccagcatcgtttaaaagcctgttgtggttcttgcagatatggccctcacttgccgcctccgtttcccggtgccgggataccgaggaggaagatcgcgccgcaggaggggtctggccggccgcggcctgagcggaggcagccgccgcgcgcaccggcggcgacgcgccaccagccgacgcatgcgcggcggggtgctgcccctgttaatccccctgatcgccgcggcgatcggcgccgtgcccgggatcgcctccgtggccttgcaagcgtcccagaggcattgacagacttgcaaacttgcaaatatggaaaaaaaaaccccaataaaaaagtctagactctcacgctcgcttggtcctgtgactattttgtagaatggaagacatcaactttgcgtcgctggccccgcgtcacggctcgcgcccgttcctgggacactggaacgatatcggcaccagcaacatgagcggtggcgccttcagttggggctctctgtggagcggcattaaaagtatcgggtctgccgttaaaaattacggctcccgggcctggaacagcagcacgggccagatgttgagagacaagttgaaagagcagaacttccagcagaaggtggtggagggcctggcctccggcatcaacggggtggtggacctggccaaccaggccgtgcagaataagatcaacagcagactggacccccggccgccggtggaggaggtgccgccggcgctggagacggtgtcccccgatgggcgtggcgagaagcgcccgcggcccgatagggaagagaccactctggtcacgcagaccgatgagccgcccccgtatgaggaggccctgaagcaaggtctgcccaccacgcggcccatcgcgcccatggccaccggggtggtgggccgccacacccccgccacgctggacttgcctccgcccgccgatgtgccgcagcagcagaaggcggcacagccgggcccgcccgcgaccgcctcccgttcctccgccggtcctctgcgccgcgcggccagcggcccccgcgggggggtcgcgaggcacggcaactggcagagcacgctgaacagcatcgtgggtctgggggtgcggtccgtgaagcgccgccgatgctactgaatagcttagctaacgtgttgtatgtgtgtatgcgccctatgtcgccgccagaggagctgctgagtcgccgccgttcgcgcgcccaccaccaccgccactccgcccctcaagatggcgaccccatcgatgatgccgcagtggtcgtacatgcacatctcgggccaggacgcctcggagtacctgagccccgggctggtgcagttcgcccgcgccaccgagagctacttcagcctgagtaacaagtttaggaaccccacggtggcgcccacgcacgatgtgaccaccgaccggtctcagcgcctgacgctgcggttcattcccgtggaccgcgaggacaccgcgtactcgtacaaggcgcggttcaccctggccgtgggcgacaaccgcgtgctggacatggcctccacctactttgacatccgcggggtgctggaccggggtcccactttcaagccctactctggcaccgcctacaactccctggcccccaagggcgctcccaactcctgcgagtgggagcaagaggaaactcaggcagttgaagaagcagcagaagaggaagaagaagatgctgacggtcaagctgaggaagagcaagcagctaccaaaaagactcatgtatatgctcaggctcccctttctggcgaaaaaattagtaaagatggtctgcaaataggaacggacgctacagctacagaacaaaaacctatttatgcagaccctacattccagcccgaaccccaaatcggggagtcccagtggaatgaggcagatgctacagtcgccggcggtagagtgctaaagaaatctactcccatgaaaccatgctatggttcctatgcaagacccacaaatgctaatggaggtcagggtgtactaacggcaaatgcccagggacagctagaatctcaggttgaaatgcaattcttttcaacttctgaaaacgcccgtaacgaggctaacaacattcagcccaaattggtgctgtatagtgaggatgtgcacatggagaccccggatacgcacctttcttacaagcccgcaaaaagcgatgacaattcaaaaatcatgctgggtcagcagtccatgcccaacagacctaattacatcggcttcagagacaactttatcggcctcatgtattacaatagcactggcaacatgggagtgcttgcaggtcaggcctctcagttgaatgcagtggtggacttgcaagacagaaacacagaactgtcctaccagctcttgcttgattccatgggtgacagaaccagatacttttccatgtggaatcaggcagtggacagttatgacccagatgttagaattattgaaaatcatggaactgaagacgagctccccaactattgtttccctctgggtggcataggggtaactgacacttaccaggctgttaaaaccaacaatggcaataacgggggccaggtgacttggacaaaagatgaaacttttgcagatcgcaatgaaataggggtgggaaacaatttcgctatggagatcaacctcagtgccaacctgtggagaaacttcctgtactccaacgtggcgctgtacctaccagacaagcttaagtacaacccctccaatgtggacatctctgacaaccccaacacctacgattacatgaacaagcgagtggtggccccggggctggtggactgctacatcaacctgggcgcgcgctggtcgctggactacatggacaacgtcaaccccttcaaccaccaccgcaatgcgggcctgcgctaccgctccatgctcctgggcaacgggcgctacgtgcccttccacatccaggtgccccagaagttctttgccatcaagaacctcctcctcctgccgggctcctacacctacgagtggaacttcaggaaggatgtcaacatggtcctccagagctctctgggtaacgatctcagggtggacggggccagcatcaagttcgagagcatctgcctctacgccaccttcttccccatggcccacaacacggcctccacgctcgaggccatgctcaggaacgacaccaacgaccagtccttcaatgactacctctccgccgccaacatgctctaccccatacccgccaacgccaccaacgtccccatctccatcccctcgcgcaactgggcggccttccgcggctgggccttcacccgcctcaagaccaaggagaccccctccctgggctcgggattcgacccctactacacctactcgggctccattccctacctggacggcaccttctacctcaaccacactttcaagaaggtctcggtcaccttcgactcctcggtcagctggccgggcaacgaccgtctgctcacccccaacgagttcgagatcaagcgctcggtcgacggggagggctacaacgtggcccagtgcaacatgaccaaggactggttcctggtccagatgctggccaactacaacatcggctaccagggcttctacatcccagagagctacaaggacaggatgtactccttcttcaggaacttccagcccatgagccggcaggtggtggaccagaccaagtacaaggactaccaggaggtgggcatcatccaccagcacaacaactcgggcttcgtgggctacctcgcccccaccatgcgcgagggacaggcctaccccgccaacttcccctatccgctcataggcaagaccgcggtcgacagcatcacccagaaaaagttcctctgcgaccgcaccctctggcgcatccccttctccagcaacttcatgtccatgggtgcgctctcggacctgggccagaacttgctctacgccaactccgcccacgccctcgacatgaccttcgaggtcgaccccatggacgagcccacccttctctatgttctgttcgaagtctttgacgtggtccgggtccaccagccgcaccgcggcgtcatcgagaccgtgtacctgcgtacgcccttctcggccggcaacgccaccacctaaagaagcaagccgcagtcatcgccgcctgcatgccgtcgggttccaccgagcaagagctcagggccatcgtcagagacctgggatgcgggccctattttttgggcaccttcgacaagcgcttccctggctttgtctccccacacaagctggcctgcgccatcgtcaacacggccggccgcgagaccgggggcgtgcactggctggccttcgcctggaacccgcgctccaaaacatgcttcctctttgaccccttcggcttttcggaccagcggctcaagcaaatctacgagttcgagtacgagggcttgctgcgtcgcagcgccatcgcctcctcgcccgaccgctgcgtcaccctcgaaaagtccacccagaccgtgcaggggcccgactcggccgcctgcggtctcttctgctgcatgtttctgcacgcctttgtgcactggcctcagagtcccatggaccgcaaccccaccatgaacttgctgacgggggtgcccaactccatgctccagagcccccaggtcgagcccaccctgcgccgcaaccaggagcagctctacagcttcctggagcgccactcgccttacttccgccgccacagcgcacagatcaggagggccacctccttctgccacttgcaagagatgcaagaagggtaataacgatgtacacactttttttctcaataaatggcatctttttatttatacaagctctctggggtattcatttcccaccaccacccgccgttgtcgccatctggctctatttagaaatcgaaagggttctgccgggagtcgccgtgcgccacgggcagggacacgttgcgatactggtagcgggtgccccacttgaactcgggcaccaccaggcgaggcagctcggggaagttttcgctccacaggctgcgggtcagcaccagcgcgttcatcaggtcgggcgccgagatcttgaagtcgcagttggggccgccgccctgcgcgcgcgagttgcggtacaccgggttgcagcactggaacaccaacagcgccgggtgcttcacgctggccagcacgctgcggtcggagatcagctcggcgtccaggtcctccgcgttgctcagcgcgaacggggtcatcttgggcacttgccgccccaggaagggcgcgtgccccggtttcgagttgcagtcgcagcgcagcgggatcagcaggtgcccgtgcccggactcggcgttggggtacagcgcgcgcatgaaggcctgcatctggcggaaggccatctgggccttggcgccctccgagaagaacatgccgcaggacttgcccgagaactggtttgcggggcagctggcgtcgtgcaggcagcagcgcgcgtcggtgttggcgatctgcaccacgttgcgcccccaccggttcttcacgatcttggccttggacgattgctccttcagcgcgcgctgcccgttctcgctggtcacatccatctcgatcacatgttccttgttcaccatgctgctgccgtgcagacacttcagctcgccctccgtctcggtgcagcggtgctgccacagcgcgcagcccgtgggctcgaaagacttgtaggtcacctccgcgaaggactgcaggtacccctgcaaaaagcggcccatcatggtcacgaaggtcttgttgctgctgaaggtcagctgcagcccgcggtgctcctcgttcagccaggtcttgcacacggccgccagcgcctccacctggtcgggcagcatcttgaagttcaccttcagctcattctccacgtggtacttgtccatcagcgtgcgcgccgcctccatgcccttctcccaggccgacaccagcggcaggctcacggggttcttcaccatcaccgtggccgccgcctccgccgcgctttcgctttccgccccgctgttctcttcctcttcctcctcttcctcgccgccgcccactcgcagcccccgcaccacggggtcgtcttcctgcaggcgctgcaccttgcgcttgccgttgcgcccctgcttgatgcgcacgggcgggttgctgaagcccaccatcaccagcgcggcctcttcttgctcgtcctcgctgtccagaatgacctccggggagggggggttggtcatcctcagtaccgaggcacgcttctttttcttcctgggggcgttcgccagctccgcggctgcggccgctgccgaggtcgaaggccgagggctgggcgtgcgcggcaccagcgcgtcctgcgagccgtcctcgtcctcctcggactcgagacggaggcgggcccgcttcttcgggggcgcgcggggcggcggaggcggcggcggcgacggagacggggacgagacatcgtccagggtgggtggacggcgggccgcgccgcgtccgcgctcgggggtggtctcgcgctggtcctcttcccgactggccatctcccactgctccttctcctataggcagaaagagatcatggagtctctcatgcgagtcgagaaggaggaggacagcctaaccgccccctctgagccctccaccaccgccgccaccaccgccaatgccgccgcggacgacgcgcccaccgagaccaccgccagtaccaccctccccagcgacgcacccccgctcgagaatgaagtgctgatcgagcaggacccgggttttgtgagcggagaggaggatgaggtggatgagaaggagaaggaggaggtcgccgcctcagtgccaaaagaggataaaaagcaagaccaggacgacgcagataaggatgagacagcagtcgggcgggggaacggaagccatgatgctgatgacggctacctagacgtgggagacgacgtgctgcttaagcacctgcaccgccagtgcgtcatcgtctgcgacgcgctgcaggagcgctgcgaagtgcccctggacgtggcggaggtcagccgcgcctacgagcggcacctcttcgcgccgcacgtgccccccaagcgccgggagaacggcacctgcgagcccaacccgcgtctcaacttctacccggtcttcgcggtacccgaggtgctggccacctaccacatctttttccaaaactgcaagatccccctctcctgccgcgccaaccgcacccgcgccgacaaaaccctgaccctgcggcagggcgcccacatacctgatatcgcctctctggaggaagtgcccaagatcttcgagggtctcggtcgcgacgagaaacgggcggcgaacgctctgcacggagacagcgaaaacgagagtcactcgggggtgctggtggagctcgagggcgacaacgcgcgcctggccgtactcaagcgcagcatagaggtcacccactttgcctacccggcgctcaacctgccccccaaggtcatgagtgtggtcatgggcgagctcatcatgcgccgcgcccagcccctggccgcggatgcaaacttgcaagagtcctccgaggaaggcctgcccgcggtcagcgacgagcagctggcgcgctggctggagacccgcgaccccgcgcagctggaggagcggcgcaagctcatgatggccgcggtgctggtcaccgtggagctcgagtgtctgcagcgcttcttcgcggaccccgagatgcagcgcaagctcgaggagaccctgcactacaccttccgccagggctacgtgcgccaggcctgcaagatctccaacgtggagctctgcaacctggtctcctacctgggcatcctgcacgagaaccgcctcgggcagaacgtcctgcactccaccctcaaaggggaggcgcgccgcgactacatccgcgactgcgcctacctcttcctctgctacacctggcagacggccatgggggtctggcagcagtgcctggaggagcgcaacctcaaggagctggaaaagctcctcaagcgcaccctcagggacctctggacgggcttcaacgagcgctcggtggccgccgcgctggcggacatcatctttcccgagcgcctgctcaagaccctgcagcagggcctgcccgacttcaccagccagagcatgctgcagaacttcaggactttcatcctggagcgctcgggcatcctgccggccacttgctgcgcgctgcccagcgacttcgtgcccatcaagtacagggagtgcccgccgccgctctggggccactgctacctcttccagctggccaactacctcgcctaccactcggacctcatggaagacgtgagcggcgagggcctgctcgagtgccactgccgctgcaacctctgcacgccccaccgctctctagtctgcaacccgcagctgctcagcgagagtcagattatcggtaccttcgagctgcagggtccctcgcctgacgagaagtccgcggctccagggctgaaactcactccggggctgtggacttccgcctacctacgcaaatttgtacctgaggactaccacgcccacgagatcaggttctacgaagaccaatcccgcccgcccaaggcggagctcaccgcctgcgtcatcacccaggggcacatcctgggccaattgcaagccatcaacaaagcccgccgagagttcttgctgaaaaagggtcggggggtgtacctggacccccagtccggcgaggagctaaacccgctacccccgccgccgccccagcagcgggaccttgcttcccaggatggcacccagaaagaagcagcagccgccgccgccgccgcagccatacatgcttctggaggaagaggaggaggactgggacagtcaggcagaggaggtttcggacgaggagcaggaggagatgatggaagactgggaggaggacagcagcctagacgaggaagcttcagaggccgaagaggtggcagacgcaacaccatcgccctcggtcgcagccccctcgccggggcccctgaaatcctccgaacccagcaccagcgctataacctccgctcctccggcgccggcgccacccgcccgcagacccaaccgtagatgggacaccacaggaaccggggtcggtaagtccaagtgcccgccgccgccaccgcagcagcagcagcagcagcgccagggctaccgctcgtggcgcgggcacaagaacgccatagtcgcctgcttgcaagactgcgggggcaacatctctttcgcccgccgcttcctgctattccaccacggggtcgcctttccccgcaatgtcctgcattactaccgtcatctctacagcccctactgcagcggcgacccagaggcggcagcggcagccacagcggcgaccaccacctaggaagatatcctccgcgggcaagacagcggcagcagcggccaggagacccgcggcagcagcggcgggagcggtgggcgcactgcgcctctcgcccaacgaacccctctcgacccgggagctcagacacaggatcttccccactttgtatgccatcttccaacagagcagaggccaggagcaggagctgaaaataaaaaacagatctctgcgctccctcacccgcagctgtctgtatcacaaaagcgaagatcagcttcggcgcacgctggaggacgcggaggcactcttcagcaaatactgcgcgctcactcttaaagactagctccgcgcccttctcgaatttaggcgggagaaaactacgtcatcgccggccgccgcccagcccgcccagccgagatgagcaaagagattcccacgccatacatgtggagctaccagccgcagatgggactcgcggcgggagcggcccaggactactccacccgcatgaactacatgagcgcgggaccccacatgatctcacaggtcaacgggatccgcgcccagcgaaaccaaatactgctggaacaggcggccatcaccgccacgccccgccataatctcaacccccgaaattggcccgccgccctcgtgtaccaggaaaccccctccgccaccaccgtactacttccgcgtgacgcccaggccgaagtccagatgactaactcaggggcgcagctcgcgggcggctttcgtcacggggcgcggccgctccgaccaggtataagacacctgatgatcagaggccgaggtatccagctcaacgacgagtcggtgagctcttcgctcggtctccgtccggacggaactttccagctcgccggatccggccgctcttcgttcacgccccgccaggcgtacctgactctgcagacctcgtcctcggagccccgctccggcggcatcggaaccctccagttcgtggaggagttcgtgccctcggtctacttcaaccccttctcgggacctcccggacgctaccccgaccagttcattccgaactttgacgcggtgaaggactcggcggacggctacgactgaatgtcaggtgtcgaggcagagcagcttcgcctgagacacctcgagcactgccgccgccacaagtgcttcgcccgcggttctggtgagttctgctactttcagctacccgaggagcataccgaggggccggcgcacggcgtccgcctgaccacccagggcgaggttacctgttccctcatccgggagtttaccctccgtcccctgctagtggagcgggagcggggtccctgtgtcctaactatcgcctgcaactgccctaaccctggattacatcaagatctttgctgtcatctctgtgctgagtttaataaacgctgagatcagaatctactgggatttagtcccctttaactaatcaaacactggaatcaataaaaagaatcacttacttaaaatcagacagcaggtctctgtccagtttattcagcagcacctccttcccctcctcccaactctggtactccaaacgccttctggcggcaaacttcctccacaccctgaagggaatgtcagattcttgctcctgtccctccgcacccactatcttcatgttgttgcagatgaagcgcaccaaaacgtctgacgagagcttcaaccccgtgtacccctatgacacggaaagcggccctccctccgtccctttcctcacccctcccttcgtgtctcccgatggattccaagaaagtccccccggggtcctgtctctgaacctggccgagcccctggtcacttcccacggcatgctcgccctgaaaatgggaagtggcctctccctggacgacgctggcaacctcacctctcaagatatcaccaccgctagccctcccctcaaaaaaaccaagaccaacctcagcctagaaacctcatcccccctaactgtgagcacctcaggcgccctcaccgtagcagccgccgctcccctggcggtggccggcacctccctcaccatgcaatcagaggcccccctgacagtacaggatgcaaaactcaccctggccaccaaaggccccctgaccgtgtctgaaggcaaactggccttgcaaacatcggccccgctgacggccgctgacagcagcaccctcacagtcagtgccacaccaccccttagcacaagcaatggcagcttgggtattgacatgcaagcccccatttacaccaccaatggaaaactaggacttaactttggcgctcccctgcatgtggtagacagcctaaatgcactgactgtagttactggccaaggtcttacgataaacggaacagccctacaaactagagtctcaggtgccctcaactatgacacatcaggaaacctagaattgagagctgcagggggtatgcgagttgatgcaaatggtcaacttatccttgatgtagcttacccatttgatgcacaaaacaatctcagccttaggcttggacagggacccctgtttgttaactctgcccacaacttggatgttaactacaacagaggcctctacctgttcacatctggaaataccaaaaagctagaagttaatatcaaaacagccaagggtctcatttatgatgacactgctatagcaatcaatgcgggtgatgggctacagtttgactcaggctcagatacaaatccattaaaaactaaacttggattaggactggattatgactccagcagagccataattgctaaactgggaactggcctaagctttgacaacacaggtgccatcacagtaggcaacaaaaatgatgacaagcttaccttgtggaccacaccagacccatcccctaactgtagaatctattcagagaaagatgctaaattcacacttgttttgactaaatgcggcagtcaggtgttggccagcgtttctgttttatctgtaaaaggtagccttgcgcccatcagtggcacagtaactagtgctcagattgtcctcagatttgatgaaaatggagttctactaagcaattcttcccttgaccctcaatactggaactacagaaaaggtgaccttacagagggcactgcatataccaacgcagtgggatttatgcccaacctcacagcatacccaaaaacacagagccaaactgctaaaagcaacattgtaagtcaggtttacttgaatggggacaaatccaaacccatgaccctcaccattaccctcaatggaactaatgaaacaggagatgccacagtaagcacttactccatgtcattctcatggaactggaatggaagtaattacattaatgaaacgttccaaaccaactccttcaccttctcctacatcgcccaagaataaaaagcatgacgctgttgatttgattcaatgtgtttctgttttattttcaagcacaacaaaatcattcaagtcattcttccatcttagcttaatagacacagtagcttaatagacccagtagtgcaaagccccattctagcttataactagtggagaagtactcgcctacatgggggtagagtcataatcgtgcatcaggatagggcggtggtgctgcagcagcgcgcgaataaactgctgccgccgccgctccgtcctgcaggaatacaacatggcagtggtctcctcagcgatgattcgcaccgcccgcagcataaggcgccttgtcctccgggcacagcagcgcaccctgatctcacttaaatcagcacagtaactgcagcacagcaccacaatattgttcaaaatcccacagtgcaaggcgctgtatccaaagctcatggcggggaccacagaacccacgtggccatcataccacaagcgcaggtagattaagtggcgacccctcataaacacgctggacataaacattacctcttttggcatgttgtaattcaccacctcccggtaccatataaacctctgattaaacatggcgccatccaccaccatcctaaaccagctggccaaaacctgcccgccggctatacactgcagggaaccgggactggaacaatgacagtggagagcccaggactcgtaaccatggatcatcatgctcgtcatgatatcaatgttggcacaacacaggcacacgtgcatacacttcctcaggattacaagctcctcccgcgttagaaccatatcccagggaacaacccattcctgaatcagcgtaaatcccacactgcagggaagacctcgcacgtaactcacgttgtgcattgtcaaagtgttacattcgggcagcagcggatgatcctccagtatggtagcgcgggtttctgtctcaaaaggaggtagacgatccctactgtacggagtgcgccgagacaaccgagatcgtgttggtcgtagtgtcatgccaaatggaacgccggacgtagtcatatttcctgaagtcttagatctctcaacgcagcaccagcaccaacacttcgcagtgtaaaaggccaagtgccgagagagtatatataggaataaaaagtgacgtaaacgggcaaagtccaaaaaacgcccagaaaaaccgcacgcgaacctacgccccgaaacgaaagccaaaaaacactagacactcccttccggcgtcaacttccgctttcccacgctacgtcacttgccccagtcaaacaaactacatatcccgaacttccaagtcgccacgcccaaaacaccgcctacacctccccgcccgccggcccgcccccaaacccgcctcccgccccgcgccccgccccgcgccgcccatctcattatcatattggcttcaatccaaaataaggtatattattgatgatggtttaaacggatcctctagagtcgacctgcaggcatgcaagcttgagtattctatagtgtcacctaaatagcttggcgtaatcatggtcatagctgtttcctgtgtgaaattgttatccgctcacaattccacacaacatacgagccggaagcataaagtgtaaagcctggggtgcctaatgagtgagctaactcacattaattgcgttgcgctcactgcccgctttccagtcgggaaacctgtcgtgccagctgcattaatgaatcggccaacgcgaaccccttgcggccgcccgggccgtcgaccaattctcatgtttgacagcttatcatcgaatttctgccattcatccgcttattatcacttattcaggcgtagcaaccaggcgtttaagggcaccaataactgccttaaaaaaattacgccccgccctgccactcatcgcagtactgttgtaattcattaagcattctgccgacatggaagccatcacaaacggcatgatgaacctgaatcgccagcggcatcagcaccttgtcgccttgcgtataatatttgcccatggtgaaaacgggggcgaagaagttgtccatattggccacgtttaaatcaaaactggtgaaactcacccagggattggctgagacgaaaaacatattctcaataaaccctttagggaaataggccaggttttcaccgtaacacgccacatcttgcgaatatatgtgtagaaactgccggaaatcgtcgtggtattcactccagagcgatgaaaacgtttcagtttgctcatggaaaacggtgtaacaagggtgaacactatcccatatcaccagctcaccgtctttcattgccatacggaattccggatgagcattcatcaggcgggcaagaatgtgaataaaggccggataaaacttgtgcttatttttctttacggtctttaaaaaggccgtaatatccagctgaacggtctggttataggtacattgagcaactgactgaaatgcctcaaaatgttctttacgatgccattgggatatatcaacggtggtatatccagtgatttttttctccattttagcttccttagctcctgaaaatctcgataactcaaaaaatacgcccggtagtgatcttatttcattatggtgaaagttggaacctcttacgtgccgatcaacgtctcattttcgccaaaagttggcccagggcttcccggtatcaacagggacaccaggatttatttattctgcgaagtgatcttccgtcacaggtatttattcgcgataagctcatggagcggcgtaaccgtcgcacaggaaggacagagaaagcgcggatctgggaagtgacggacagaacggtcaggacctggattggggaggcggttgccgccgctgctgctgacggtgtgacgttctctgttccggtcacaccacatacgttccgccattcctatgcgatgcacatgctgtatgccggtataccgctgaaagttctgcaaagcctgatgggacataagtccatcagttcaacggaagtctacacgaaggtttttgcgctggatgtggctgcccggcaccgggtgcagtttgcgatgccggagtctgatgcggttgcgatgctgaaacaattatcctgagaataaatgccttggcctttatatggaaatgtggaactgagtggatatgctgtttttgtctgttaaacagagaagctggctgttatccactgagaagcgaacgaaacagtcgggaaaatctcccattatcgtagagatccgcattattaatctcaggagcctgtgtagcgtttataggaagtagtgttctgtcatgatgcctgcaagcggtaacgaaaacgatttgaatatgccttcaggaacaatagaaatcttcgtgcggtgttacgttgaagtggagcggattatgtcagcaatggacagaacaacctaatgaacacagaaccatgatgtggtctgtccttttacagccagtagtgctcgccgcagtcgagcgacagggcgaagccctcgagtgagcgaggaagcaccagggaacagcacttatatattctgcttacacacgatgcctgaaaaaacttcccttggggttatccacttatccacggggatatttttataattattttttttatagtttttagatcttcttttttagagcgccttgtaggcctttatccatgctggttctagagaaggtgttgtgacaaattgccctttcagtgtgacaaatcaccctcaaatgacagtcctgtctgtgacaaattgcccttaaccctgtgacaaattgccctcagaagaagctgttttttcacaaagttatccctgcttattgactcttttttatttagtgtgacaatctaaaaacttgtcacacttcacatggatctgtcatggcggaaacagcggttatcaatcacaagaaacgtaaaaatagcccgcgaatcgtccagtcaaacgacctcactgaggcggcatatagtctctcccgggatcaaaaacgtatgctgtatctgttcgttgaccagatcagaaaatctgatggcaccctacaggaacatgacggtatctgcgagatccatgttgctaaatatgctgaaatattcggattgacctctgcggaagccagtaaggatatacggcaggcattgaagagtttcgcggggaaggaagtggttttttatcgccctgaagaggatgccggcgatgaaaaaggctatgaatcttttccttggtttatcaaacgtgcgcacagtccatccagagggctttacagtgtacatatcaacccatatctcattcccttctttatcgggttacagaaccggtttacgcagtttcggcttagtgaaacaaaagaaatcaccaatccgtatgccatgcgtttatacgaatccctgtgtcagtatcgtaagccggatggctcaggcatcgtctctctgaaaatcgactggatcatagagcgttaccagctgcctcaaagttaccagcgtatgcctgacttccgccgccgcttcctgcaggtctgtgttaatgagatcaacagcagaactccaatgcgcctctcatacattgagaaaaagaaaggccgccagacgactcatatcgtattttccttccgcgatatcacttccatgacgacaggatagtctgagggttatctgtcacagatttgagggtggttcgtcacatttgttctgacctactgagggtaatttgtcacagttttgctgtttccttcagcctgcatggattttctcatactttttgaactgtaatttttaaggaagccaaatttgagggcagtttgtcacagttgatttccttctctttcccttcgtcatgtgacctgatatcgggggttagttcgtcatcattgatgagggttgattatcacagtttattactctgaattggctatccgcgtgtgtacctctacctggagtttttcccacggtggatatttcttcttgcgctgagcgtaagagctatctgacagaacagttcttctttgcttcctcgccagttcgctcgctatgctcggttacacggctgcggcgagcgctagtgataataagtgactgaggtatgtgctcttcttatctccttttgtagtgttgctcttattttaaacaactttgcggttttttgatgactttgcgattttgttgttgctttgcagtaaattgcaagatttaataaaaaaacgcaaagcaatgattaaaggatgttcagaatgaaactcatggaaacacttaaccagtgcataaacgctggtcatgaaatgacgaaggctatcgccattgcacagtttaatgatgacagcccggaagcgaggaaaataacccggcgctggagaataggtgaagcagcggatttagttggggtttcttctcaggctatcagagatgccgagaaagcagggcgactaccgcacccggatatggaaattcgaggacgggttgagcaacgtgttggttatacaattgaacaaattaatcatatgcgtgatgtgtttggtacgcgattgcgacgtgctgaagacgtatttccaccggtgatcggggttgctgcccataaaggtggcgtttacaaaacctcagtttctgttcatcttgctcaggatctggctctgaaggggctacgtgttttgctcgtggaaggtaacgacccccagggaacagcctcaatgtatcacggatgggtaccagatcttcatattcatgcagaagacactctcctgcctttctatcttggggaaaaggacgatgtcacttatgcaataaagcccacttgctggccggggcttgacattattccttcctgtctggctctgcaccgtattgaaactgagttaatgggcaaatttgatgaaggtaaactgcccaccgatccacacctgatgctccgactggccattgaaactgttgctcatgactatgatgtcatagttattgacagcgcgcctaacctgggtatcggcacgattaatgtcgtatgtgctgctgatgtgctgattgttcccacgcctgctgagttgtttgactacacctccgcactgcagtttttcgatatgcttcgtgatctgctcaagaacgttgatcttaaagggttcgagcctgatgtacgtattttgcttaccaaatacagcaatagtaatggctctcagtccccgtggatggaggagcaaattcgggatgcctggggaagcatggttctaaaaaatgttgtacgtgaaacggatgaagttggtaaaggtcagatccggatgagaactgtttttgaacaggccattgatcaacgctcttcaactggtgcctggagaaatgctctttctatttgggaacctgtctgcaatgaaattttcgatcgtctgattaaaccacgctgggagattagataatgaagcgtgcgcctgttattccaaaacatacgctcaatactcaaccggttgaagatacttcgttatcgacaccagctgccccgatggtggattcgttaattgcgcgcgtaggagtaatggctcgcggtaatgccattactttgcctgtatgtggtcgggatgtgaagtttactcttgaagtgctccggggtgatagtgttgagaagacctctcgggtatggtcaggtaatgaacgtgaccaggagctgcttactgaggacgcactggatgatctcatcccttcttttctactgactggtcaacagacaccggcgttcggtcgaagagtatctggtgtcatagaaattgccgatgggagtcgccgtcgtaaagctgctgcacttaccgaaagtgattatcgtgttctggttggcgagctggatgatgagcagatggctgcattatccagattgggtaacgattatcgcccaacaagtgcttatgaacgtggtcagcgttatgcaagccgattgcagaatgaatttgctggaaatatttctgcgctggctgatgcggaaaatatttcacgtaagattattacccgctgtatcaacaccgccaaattgcctaaatcagttgttgctcttttttctcaccccggtgaactatctgcccggtcaggtgatgcacttcaaaaagcctttacagataaagaggaattacttaagcagcaggcatctaaccttcatgagcagaaaaaagctggggtgatatttgaagctgaagaagttatcactcttttaacttctgtgcttaaaacgtcatctgcatcaagaactagtttaagctcacgacatcagtttgctcctggagcgacagtattgtataagggcgataaaatggtgcttaacctggacaggtctcgtgttccaactgagtgtatagagaaaattgaggccattcttaaggaacttgaaaagccagcaccctgatgcgaccacgttttagtctacgtttatctgtctttacttaatgtcctttgttacaggccagaaagcataactggcctgaatattctctctgggcccactgttccacttgtatcgtcggtctgataatcagactgggaccacggtcccactcgtatcgtcggtctgattattagtctgggaccacggtcccactcgtatcgtcggtctgattattagtctgggaccacggtcccactcgtatcgtcggtctgataatcagactgggaccacggtcccactcgtatcgtcggtctgattattagtctgggaccatggtcccactcgtatcgtcggtctgattattagtctgggaccacggtcccactcgtatcgtcggtctgattattagtctggaaccacggtcccactcgtatcgtcggtctgattattagtctgggaccacggtcccactcgtatcgtcggtctgattattagtctgggaccacgatcccactcgtgttgtcggtctgattatcggtctgggaccacggtcccacttgtattgtcgatcagactatcagcgtgagactacgattccatcaatgcctgtcaagggcaagtattgacatgtcgtcgtaacctgtagaacggagtaacctcggtgtgcggttgtatgcctgctgtggattgctgctgtgtcctgcttatccacaacattttgcgcacggttatgtggacaaaatacctggttacccaggccgtgccggcacgttaaccgggctgcatccgatgcaagtgtgtcgctgtcgacgagctcgcgagctcggacatgaggttgccccgtattcagtgtcgctgatttgtattgtctgaagttgtttttacgttaagttgatgcagatcaattaatacgatacctgcgtcataattgattatttgacgtggtttgatggcctccacgcacgttgtgatatgtagatgataatcattatcactttacgggtcctttccggtgatccgacaggttacggggcggcgacctcgcgggttttcgctatttatgaaaattttccggtttaaggcgtttccgttcttcttcgtcataacttaatgtttttatttaaaataccctctgaaaagaaaggaaacgacaggtgctgaaagcgagctttttggcctctgtcgtttcctttctctgtttttgtccgtggaatgaacaatggaagtccgagctcatcgctaataacttcgtatagcatacattatacgaagttatattcgatgcggccgcaaggggttcgcgtcagcgggtgttggcgggtgtcggggctggcttaactatgcggcatcagagcagattgtactgagagtgcaccatatgcggtgtgaaataccgcacagatgcgtaaggagaaaataccgcatcaggcgccattcgccattcaggctgcgcaactgttgggaagggcgatcggtgcgggcctcttcgctattacgccagctggcgaaagggggatgtgctgcaaggcgattaagttgggtaacgccagggttttcccagtcacgacgttgtaaaacgacggccagtgaattgtaatacgactcactatagggcgaattcgagctcggtacccggggatcctcgtttaaac

SEQ ID NO: 54 - DNA, 42220 bp, Artificial Sequence
  source: /note="Description of Artificial Sequence: Synthetic polynucleotide"
  modified_base (16789)..(16789): a, c, t, g, unknown or other
catcatcaataatataccttattttggattgaagccaatatgataatgagatgggcggcgcggggcggggcgcggggcgggaggcgggtttgggggcgggccggcgggcggggcggtgtggcggaagtggactttgtaagtgtggcggatgtgacttgctagtgccgggcgcggtaaaagtgacgttttccgtgcgcgacaacgcccccgggaagtgacatttttcccgcggtttttaccggatgttgtagtgaatttgggcgtaaccaagtaagatttggccattttcgcgggaaaactgaaacggggaagtgaaatctgattaattttgcgttagtcataccgcgtaatatttgtctagggccgagggactttggccgattacgtggaggactcgcccaggtgttttttgaggtgaatttccgcgttccgggtcaaagtctgcgttttattattataggatatcccattgcatacgttgtatccatatcataatatgtacatttatattggctcatgtccaacattaccgccatgttgacattgattattgactagttattaatagtaatcaattacggggtcattagttcatagcccatatatggagttccgcgttacataacttacggtaaatggcccgcctggctgaccgcccaacgacccccgcccattgacgtcaataatgacgtatgttcccatagtaacgccaatagggactttccattgacgtcaatgggtggagtatttacggtaaactgcccacttggcagtacatcaagtgtatcatatgccaagtacgccccctattgacgtcaatgacggtaaatggcccgcctggcattatgcccagtacatgaccttatgggactttcctacttggcagtacatctacgtattagtcatcgctattaccatggtgatgcggttttggcagtacatcaatgggcgtggatagcggtttgactcacggggatttccaagtctccaccccattgacgtcaatgggagtttgttttggcaccaaaatcaacgggactttccaaaatgtcgtaacaactccgccccattgacgcaaatgggcggtaggcgtgtacggtgggaggtctatataagcagagctctccctatcagtgatagagatctccctatcagtgatagagatcgtcgacgagctcgtttagtgaaccgtcagatcgcctggagacgccatccacgctgttttgacctccatagaagacaccgggaccgatccagcctccgcggccgggaacggtgcattggaacgcggattccccgtgccaagagtgagatcttccgtttatctaggtaccagatatcgccaccatggacgaccagcgggacctgatcagcaacaacgagcagctgcccatgctgggccagaggcctggcgcccctgagagcaagtgtagcagaggcgccgtgtacaccgtgttcagcatcctggtggccctgctgctggccggacaggccaccaccgcctactttctgtatcagcagcagggacggctggacaagctgaccgtgaccagccagaacctgcagctggaaaacctgcggatgaagctgcccaagcccgccaagcccctgagccagatgagaatggccacccccctgctgatgcaggccctgcctatggccggcctgccccagaaacccatgcagaacgccaccaagcacggcaacatgaccgaggaccacgtgatgcatctgctgctgaacgccgaccccctgaaggtgtaccccccactgaagggcagcctgagcgagaacctgaagcacctgaagaacaccatggaaaccatggactggaaggtgttcgagagctggctgcaccactggctgctgttcgagatgagcaagcacagcctggaacagaagcccaccgaggcccctcccaaagagagcctggaactggaagatcccagcagcggcctgggcgtgaccaagcaggatctgggccccgtggctatgtccgaggactttctgattctgatcgccatcctggtgatcgtgattctcgtgggcacaatcacaaccctggtgggcgccatcggcggcattagggccaggaggagcttcctcttcatttgcatcttcttcctgttcctctccctcttcctgacaatcctcgccctgctgctgggcttcagctggctcctgctggtggccatcctgttctgggtgctctggctggtcatcctcattctgctgctgctggtgtaccctattcctcaccaccccctgcccacctccctcaggtttagaatgaagcagagggtgagcagcgaccccacaggttctgacagaagccctcagggcagccataatagcctgaactcccccgatgaggaggaccccaaggatgacaccaagcaacctctgtgcaacatgacccagggcggacctcccgtcaatggacagctcctcggacaacatgctcaatgcccccctcactatccctgctgccatattcagcatcccgacggagaggattccgatggagacgatggcaagtcctggggcgatgccggagaggaagacaatggccctaacgaccctaacaccgccagcaccagagagtccatttacgaggacctcagataccccacaagggacgccaatggcgagtatgagaacgtgggatacccccctagggacggagatgcccctcataggctcggagagcctgtgtatgacgatgtggagcaagccaccgctaacgaggtgagaatctcccctctgttcagactgccctacggaagcgctttcggacctggcccccagcctggacccattctggagagctccacatggggctttctggtcttcacacagacctccctgttcgccgacgacattgccgacgctattagggactactgcacaacccaccctggccccacaaggaacacccaggtggtcctcatgaacttcgagggcagcggagtgcccctgcctatgttttttccccctggagaggagacagaagagcagagagagggcgatagagctagcgactccgacgagtccgaagacgctcagatcctgaccgtgttctgcctgttttgccagtggacactctttatctgcctgggaatcaggatgatctgtaactggaggggcaaactcaccaggatcatctgcctgaagttctgcctctacggactgatttccgcctccctgtccttcggctggtacgcttttctgaaggaagtgaccctccccaccacagccaccgttgatcctaggcaactccccctgttcctcttcatcctgagctccgtgctggtgattctcgccatcatgatggagtttcaaacatcctccagcctcttcgctgctctgttcgtgattatcgccggaatgctgtgcgtcacagtgggcgtgatttttctgctggctggcgtcaagcctctcctgagcggcatgatctgcgcctccggcatcacaatgctcgtgctcggcgtcgtgctgctggtggtgtgcaccagagatgagcacgctatttccgccagccaccatgctagcgatggctccgtgaatcagcagaaggaaaatcagccccagaccctggaggaatgcaagacagatcaggagaggaagaggtacaggaacaggctggcctccaggaggtgtagagctaagttcaggaaccagctggaacattttaggacagtcgccgctgctaagacagaggagaacaacaggctcagggtgctcatcaggcagatgtgtcctacactggacgtggaatccatcgtcccctccacctccgccggctaccacgagcctctgaatcacctgacccacagccccagcccttgtcatcacagggatgaacccccctccagaagccccagccctcaacccaccgtctccgagcagtcccagcagtcccccaggcagcagagccctcaaggcacatcccagggttctacaagacctcaggtgcctggaggcgccaccaccagaaaaagaggcggcgtgagaggccaacctgccaagtgtcacggcaagtacaccacaaccgccgagggactgaccgctctcctgaataggaggcacagccccaggacatccaacgagggcaggtggatgaatggagtcatggctgtgaacctctccaaatggcccctgtacagcctgaggagagccctggccctcgccatggctcctagaaggaggctctccggccctccctggctgacagtgctgctgctgctgtccacactgagcgtggccgccctgctgattctcttcctgattttcagcgccggcgccaccattagcacagaagccagcctgctggtcctgctcctgctgtttgtgaccctgctgctgcctctcctgtcctccaacggactccagctccctgccgccctgattctgatccagtgtttcctcctggccgctgattatctcgcctacctgattctgcctaccattatgcccaggggcagaagcacaggaaggaagggcagggacacagagaaagagaggagcagatcccctctcagagctcctggcggttctgatggacccagcacaagggctggctgtggagccggaccctgtcagctgagcagccccatcgccggaaacaacggcaatgaaggcggcgagggcgacgactacaagagctggaggaagcccgaggaagaggacaacggccccaatgaccccaataccaacaacaggattgaggatggagacggcgacgacggaaaatcctggaggaatcctgaggaggaggataacagaaagcaggacaggctgggcaccaagcctttcatggacctcgacggaaccggcggaggcgagggctacagccagatggtccctatcgccaccgcccccggaagcggccacgccgctacctatcaggatctccaggccgccccttacatcatctggcctctccagaccgattgccagcctgtggctaccaccttcgcctcccccggacagatccagtggtatacaagcgccgtcccccagcccacagagcattgctcccagtttacaaacgctcccaccgtcaaccagcagcagcctattagccaaccccagcccgaaaatccccctgctttcacctttacccagcccgcttccatcattcccggcgtcattagcgcctccaacctgaacgtgagcgcttcccctatcatccctagcgaccatgtcctccccatcattacctccgtgaccagcctcgcccaacctaataacatggccggccactggtatgagagcgtgattcccggcctgttcctctgccccctgatcctcccttccctgttctggatttgctccctgctgaccttcctggtgggccacggagccaatattgtgagcgccgtcctgttcctcgtgctggcttggtgtctcctcattgccaactggaacgtgacaagagaggacttcgtgtccggcaggagaagctccatgagcagcctgtccgtggccgcttccaccgccacagccatgttcgccagcttcctcaccctgagctttgatggcctgggcctgctgctgtttggcaccgccctggtgatccagacaatttacgtgctgtatctggtggtcatggagatcaccgtgtggatcatgatgtttaggtatctccacttttggatcaccctgctgttcctgctgagccccattattctctccgtcgcctgtctcatcatccaatcctccgccctgctgatcgaggctgtggtcgtcaccaccatcacagtcctggccatttttctgtggctccctcctcaaggcgctgaggccgatctcggcaccgccctgctgattctgaataccgccctgtgcctggtcgtgctgatcctgaccgctatccctacatgatgatgagcggccgcgatctgctgtgccttctagttgccagccatctgttgtttgcccctcccccgtgccttccttgaccctggaaggtgccactcccactgtcctttcctaataaaatgaggaaattgcatcgcattgtctgagtaggtgtcattctattctggggggtggggtggggcaggacagcaagggggaggattgggaagacaatagcaggcatgctggggatgcggtgggctctatggccgatcagcgatcgctgaggtgggtgagtgggcgtggcctggggtggtcatgaaaatatataagttgggggtcttagggtctctttatttgtgttgcagagaccgccggagccatgagcgggagcagcagcagcagcagtagcagcagcgccttggatggcagcatcgtgagcccttatttgacgacgcggatgccccactgggccggggtgcgtcagaatgtgatgggctccagcatcgacggccgacccgtcctgcccgcaaattccgccacgctgacctatgcgaccgtcgcggggacgccgttggacgccaccgccgccgccgccgccaccgcagccgcctcggccgtgcgcagcctggccacggactttgcattcctgggaccactggcgacaggggctacttctcgggccgctgctgccgccgttcgcgatgacaagctgaccgccctgctggcgcagttggatgcgcttactcgggaactgggtgacctttctcagcaggtcatggccctgcgccagcaggtctcctccctgcaagctggcgggaatgcttctcccacaaatgccgtttaagataaataaaaccagactctgtttggattaaagaaaagtagcaagtgcattgctctctttatttcataattttccgcgcgcgataggccctagaccagcgttctcggtcgttgagggtgcggtgtatcttctccaggacgtggtagaggtggctctggacgttgagatacatgggcatgagcccgtcccgggggtggaggtagcaccactgcagagcttcatgctccggggtggtgttgtagatgatccagtcgtagcaggagcgctgggcatggtgcctaaaaatgtccttcagcagcaggccgatggccagggggaggcccttggtgtaagtgtttacaaaacggttaagttgggaagggtgcattcggggagagatgatgtgcatcttggactgtatttttagattggcgatgtttccgcccagatcccttctgggattcatgttgtgcaggaccaccagtacagtgtatccggtgcacttggggaatttgtcatgcagcttagagggaaaagcgtggaagaacttggagacgcctttgtggcctcccagattttccatgcattcgtccatgatgatggcaatgggcccgcgggaggcagcttgggcaaagatatttctggggtcgctgacgtcgtagttgtgttccagggtgaggtcgtcataggccatttttacaaagcgcgggcggagggtgcccgactgggggatgatggtcccctctggccctggggcgtagttgccctcgcagatctgcatttcccaggccttaatctcggaggggggaatcatatccacctgcggggcgatgaagaaaacggtttccggagccggggagattaactgggatgagagcaggtttctaagcagctgtgattttccacaaccggtgggcccataaataacacctataaccggttgcagctggtagtttagagagctgcagctgccgtcgtcccggaggaggggggccacctcgttgagcatgtccctgacgcgcatgttctccccgaccagatccgccagaaggcgctcgccgcccagggacagcagctcttgcaaggaagcaaagtttttcagcggcttgaggccgtccgccgtgggcatgtttttcagggtctggctcagcagctccaggcggtcccagagctcggtgacgtgctctacggcatctctatccagcatatctcctcgtttcgcgggttggggcgactttcgctgtagggcaccaagcggtggtcgtccagcggggccagagtcatgtccttccatgggcgcagggtcctcgtcagggtggtctgggtcacggtgaaggggtgcgctccgggctgagcgcttgccaaggtgcgcttgaggctggttctgctggtgctgaagcgctgccggtcttcgccctgcgcgtcggccaggtagcatttgaccatggtgtcatagtccagcccctccgcggcgtgtcccttggcgcgcagcttgcccttggaggtggcgccgcacgaggggcagagcaggctcttgagcgcgtagagcttgggggcgaggaagaccgattcgggggagtaggcgtccgcgccgcagaccccgcacacggtctcgcactccaccagccaggtgagctcggggcgcgccgggtcaaaaaccaggtttcccccatgctttttgatgcgtttcttacctcgggtctccatgaggtggtgtccccgctcggtgacgaagaggctgtccgtgtctccgtagaccgacttgaggggtcttttctccaggggggtccctcggtcttcctcgtagaggaactcggaccactctgagacgaaggcccgcgtccaggccaggacgaaggaggctatgtgggaggggtagcggtcgttgtccactagggggtccaccttctccaaggtgtgaagacacatgtcgccttcctcggcgtccaggaaggtgattggcttgtaggtgtaggccacgtgaccgggggttcctgacgggggggtataaaagggggtgggggcgcgctcgtcgtcactctcttccgcatcgctgtctgcgagggccagctgctggggtgagtattccctctcgaaggcgggcatgacctccgcgctgaggttgtcagtttccaaaaacgaggaggatttgatgttcacctgtcccgaggtgatacctttgagggtacccgcgtccatctggtcagaaaacacgatctttttattgtccagcttggtggcgaacgacccgtagagggcgttggagagcagcttggcgatggagcgcagggtctggttcttgtccctgtcggcgcgctccttggccgcgatgttgagctgcacgtactcgcgcgcgacgcagcgccactcggggaagacggtggtgcgctcgtcgggcaccaggcgcacgcgccagccgcggttgtgcagggtgaccaggtccacgctggtggcgacctcgccgcgcaggcgctcgttggtccagcagagacggccgcccttgcgcgagcagaaggggggcagggggtcgagctgggtctcgtccggggggtccgcgtccacggtgaaaaccccggggcgcaggcgcgcgtcgaagtagtctatcttgcaaccttgcatgtccagcgcctgctgccagtcgcgggcggcgagcgcgcgctcgtaggggttgagcggcgggccccagggcatggggtgggtgagtgcggaggcgtacatgccgcagatgtcatagacgtagaggggctcccgcaggaccccgatgtaggtggggtagcagcggccgccgcggatgctggcgcgcacgtagtcatacagctcgtgcgagggggcgaggaggtcggggcccaggttggtgcgggcggggcgctccgcgcggaagacgatctgcctgaagatggcatgcgagttggaagagatggtggggcgctggaagacgttgaagctggcgtcctgcaggccgacggcgtcgcgcacgaaggaggcgtaggagtcgcgcagcttgtgtaccagctcggcggtgacctgcacgtcgagcgcgcagtagtcgagggtctcgcggatgatgtcatatttagcctgccccttctttttccacagctcgcggttgaggacaaactcttcgcggtctttccagtactcttggatcgggaaaccgtccggttccgaacggtaagagcctagcatgtagaactggttgacggcctggtaggcgcagcagcccttctccacggggagggcgtaggcctgcgcggccttgcggagcgaggtgtgggtcagggcgaaggtgtccctgaccatgactttgaggtactggtgcttgaagtcggagtcgtcgcagccgccccgctcccagagcgagaagtcggtgcgcttcttggagcgggggttgggcagagcgaaggtgacatcgttgaagaggattttgcccgcgcggggcatgaagttgcgggtgatgcggaagggccccggcacttcagagcggttgttgatgacctgggcggcgagcacgatctcgtcgaagccgttgatgttgtggcccacgatgtagagttccaggaagcggggccggccctttacggtgggcagcttctttagctcttcgtaggtgagctcctcgggcgaggcgaggccgtgctcggccagggcccagtccgcgaggtgcgggttgtctctgaggaaggacttccagaggtcgcgggccaggagggtctgcaggcggtctctgaaggtcctgaactggcggcccacggccattttttcgggggtgatgcagtagaaggtgagggggtcttgctgccagcggtcccagtcgagctgcagggcgaggtcgcgcgcggcggtgaccaggcgctcgtcgcccccgaatttcatgaccagcatgaagggcacgagctgctttccgaaggcccccatccaagtgtaggtctctacatcgtaggtgacaaagaggcgctccgtgcgaggatgcgagccgatcgggaagaactggatctcccgccaccagttggaggagtggctgttgatgtggtggaagtagaagtcccgtcgccgggccgaacactcgtgctggcttttgtaaaagcgagcgcagtactggcagcgctgcacgggctgtacctcatgcacgagatgcacctttcgcccgcgcacgaggaagccgaggggaaatctgagccccccgcctggctcgcggcatggctggttctcttctactttggatgcgtgtccgtctccgtctggctcctcgaggggtgttacggtggagcggaccaccacgccgcgcgagccgcaggtccagatatcggcgcgcggcggtcggagtttgatgacgacatcgcgcagctgggagctgtccatggtctggagctcccgcggcggcggcaggtcagccgggagttcttgcaggttcacctcgcagagtcgggccagggcgcggggcaggtctaggtggtacctgatctctaggggcgtgttggtggcggcgtcgatggcttgcaggagcccgcagccccggggggcgacgacggtgccccgcggggtggtggtggtggtggcggtgcagctcagaagcggtgccgcgggcgggcccccggaggtagggggggctccggtcccgcgggcaggggcggcagcggcacgtcggcgtggagcgcgggcaggagttggtgctgtgcccggaggttgctggcgaaggcgacgacgcggcggttgatctcctggatctggcgcctctgcgtgaagacgacgggcccggtgagcttgaacctgaaagagagttcgacagaatcaatctcggtgtcattgaccgcggcctggcgcaggatctcctgcacgtctcccgagttgtcttggtaggcgatctcggccatgaactgctcgatctcttcctcctggaggtctccgcgtccggcgcgttccacggtggccgccaggtcgttggagatgcgccccatgagctgcgagaaggcgttgagtccgccctcgttccagactcggctgtagaccacgcccccctggtcatcgcgggcgcgcatgaccacctgcgcgaggttgagctccacgtgccgcgcgaagacggcgtagttgcgcagacgctggaagaggtagttgagggtggtggcggtgtgctcggccacgaagaagttcatgacccagcggcgcaacgtggattcgttgatgtcccccaaggcctccagccgttccatggcctcgtagaagtccacggcgaagttgaaaaactgggagttgcgcgccgacacggtcaactcctcctccagaagacggatgagctcggcgacggtgtcgcgcacctcgcgctcgaaggctatggggatctcttcctccgctagcatcaccacctcctcctcttcctcctcttctggcacttccatgatggcttcctcctcttcggggggtggcggcggcggcggtgggggagggggcgctctgcgccggcggcggcgcaccgggaggcggtccacgaagcgcgcgatcatctccccgcggcggcggcgcatggtctcggtgacggcgcggccgttctcccgggggcgcagttggaagacgccgccggacatctggtgctggggcgggtggccgtgaggcagcgagacggcgctgacgatgcatctcaacaattgctgcgtaggtacgccgccgagggacctgagggagtccatatccaccggatccgaaaacctttcgaggaaggcgtctaaccagtcgcagtcgcaaggtaggctgagcaccgtggcgggcggcggggggtggggggagtgtctggcggaggtgctgctgatgatgtaattgaagtaggcggacttgacacggcggatggtcgacaggagcaccatgtccttgggtccggcctgctggatgcggaggcggtcggctatgccccaggcttcgttctggcatcggcgcaggtccttgtagtagtcttgcatgagcctttccaccggcacctcttctccttcctcttctgcttcttccatgtctgcttcggccctggggcggcgccgcgcccccctgccccccatgcgcgtgaccccgaaccccctgagcggttggagcagggccaggtcggcgacgacgcgctcggccaggatggcctgctgcacctgcgtgagggtggtttggaagtcatccaagtccacgaagcggtggtaggcgcccgtgttgatggtgtaggtgcagttggccatgacggaccagttgacggtctggtggcccggttgcgacatctcggtgtacctgagtcgcgagtaggcgcgggagtcgaagacgtagtcgttgcaagtccgcaccaggtactggtagcccaccaggaagtgcggcggcggctggcggtagaggggccagcgcagggtggcgggggctccgggggccaggtcttccagcatgaggcggtggtaggcgtagatgtacctggacatccaggtgatacccgcggcggtggtggaggcgcgcgggaagtcgcgcacccggttccagatgttgcgcaggggcagaaagtgctccatggtaggcgtgctctgtccagtcagacgcgcgcagtcgttgatactctagaccagggaaaacgaaagccggtcagcgggcactcttccgtggtctggtgaatagatcgcaagggtatcatggcggagggcctcggttcgagccccgggtccgggccggacggtccgccatgatccacgcggttaccgcccgcgtgtcgaacccaggtgtgcgacgtcagacaacggtggagtgttccttttggcgtttttctggccgggcgccggcgccgcgtaagagactaagccgcgaaagcgaaagcagtaagtggctcgctccccgtagccggagggatccttgctaagggttgcgttgcggcgaaccccggttcgaatcccgtactcgggccggccggacccgcggctaaggtgttggattggcctccccctcgtataaagaccccgcttgcggattgactccggacacggggacgagccccttttatttttgctttccccagatgcatccggtgctgcggcagatgcgccccccgccccagcagcagcaacaacaccagcaagagcggcagcaacagcagcgggagtcatgcagggccccctcacccaccctcggcgggccggccacctcggcgtccgcggccgtgtctggcgcctgcggcggcggcggggggccggctgacgaccccgaggagcccccgcggcgcagggccagacactacctggacctggaggagggcgagggcctggcgcggctgggggcgccgtctcccgagcgccacccgcgggtgcagctgaagcgcgactcgcgcgaggcgtacgtgcctcggcagaacctgttcagggaccgcgcgggcgaggagcccgaggagatgcgggacaggaggttcagcgcagggcgggagctgcggcaggggctgaaccgcgagcggctgctgcgcgaggaggactttgagcccgacgcgcggacggggatcagccccgcgcgcgcgcacgtggcggccgccgacctggtgacggcgtacgagcagacggtgaaccaggagatcaacttccaaaagagtttcaacaaccacgtgcgcacgctggtggcgcgcgaggaggtgaccatcgggctgatgcacctgtgggactttgtaagcgcgctggtgcagaaccccaacagcaagcctctgacggcgcagctgttcctgatagtgcagcacagcagggacaacgaggcgtttagggacgcgctgctgaacatcaccgagcccgagggtcggtggctgctggacctgattaacatcctgcagagcatagtggtgcaggagcgcagcctgagcctggccgacaaggtggcggccatcaactactcgatgctgagcctgggcaagttttacgcgcgcaagatctaccagacgccgtacgtgcccatagacaaggaggtgaagatcgacggtttttacatgcgcatggcgctgaaggtgctcaccctgagcgacgacctgggcgtgtaccgcaacgagcgcatccacaaggccgtgagcgtgagccggcggcgcgagctgagcgaccgcgagctgatgcacagcctgcagcgggcgctggcgggcgccggcagcggcgacagggaggcggagtcctacttcgatgcgggggcggacctgcgctgggcgcccagccggcgggccctggaggccgcgggggtccgcgaggactatgacgaggacggcgaggaggatgaggagtacgagctagaggagggcgagtacctggactaaaccgcgggtggtgtttccggtagatgcaagacccgaacgtggtggacccggcgctgcgggcggctctgcagagccagccgtccggccttaactcctcagacgactggcgacaggtcatggaccgcatcatgtcgctgacggcgcgtaacccggacgcgttccggcagcagccgcaggccaacaggctctccgccatcctggaggcggtggtgcctgcgcgctcgaaccccacgcacgagaaggtgctggccatagtgaacgcgctggccgagaacagggccatccgcccggacgaggccgggctggtgtacgacgcgctgctgcagcgcgtggcccgctacaacagcggcaacgtgcagaccaacctggaccggctggtgggggacgtgcgcgaggcggtggcgcagcgcgagcgcgcggatcggcagggcaacctgggctccatggtggcgctgaatgccttcctgagcacgcagccggccaacgtgccgcgggggcaggaagactacaccaactttgtgagcgcgctgcggctgatggtgaccgagaccccccagagcgaggtgtaccagtcgggcccggactacttcttccagaccagcagacagggcctgcagacggtgaacctgagccaggctttcaagaacctgcgggggctgtggggcgtgaaggcgcccaccggcgaccgggcgacggtgtccagcctgctgacgcccaactcgcgcctgctgctgctgctgatcgcgccgttcacggacagcggcagcgtgtcccgggacacctacctggggcacctgctgaccctgtaccgcgaggccatcgggcaggcgcaggtggacgagcacaccttccaggagatcaccagcgtgagccgcgcgctggggcaggaggacacgagcagcctggaggcgactctgaactacctgctgaccaaccggcggcagaagattccctcgctgcacagcctgacctccgaggaggagcgcatcttgcgctacgtgcagcagagcgtgagcctgaacctgatgcgcgacggggtgacgcccagcgtggcgctggacatgaccgcgcgcaacatggaaccgggcatgtacgccgcgcaccggccttacatcaaccgcctgatggactacctgcatcgcgcggcggccgtgaaccccgagtactttaccaacgccatcctgaacccgcactggctcccgccgcccgggttctacagcgggggcttcgaggtcccggagaccaacgatggcttcctgtgggacgacatggacgacagcgtgttctccccgcggccgcaggcgctggcggaagcgtccctgctgcgtcccaagaaggaggaggaggaggaggcgagtcgccgccgcggcagcagcggcgtggcttctctgtccgagctgggggcggcagccgccgcgcgccccgggtccctgggcggcagcccctttccgagcctggtggggtctctgcacagcgagcgcaccacccgccctcggctgctgggcgaggacgagtacctgaataactccctgctgcagccggtgcgggagaaaaacctgcctcccgccttccccaacaacgggatagagagcctggtggacaagatgagcagatggaagacctatgcgcaggagcacagggacgcgcctgcgctccggccgcccacgcggcgccagcgccacgaccggcagcgggggctggtgtgggatgacgaggactccgcggacgatagcagcgtgctggacctgggagggagcggcaacccgttcgcgcacctgcgcccccgcctggggaggatgttttaaaaaaaaaaaaaaaangcaagaagcatgatgcaaaaattaaataaaactcaccaaggccatggcgaccgagcgttggtttcttgtgttcccttcagtatgcggcgcgcggcgatgtaccaggagggacctcctccctcttacgagagcgtggtgggcgcggcggcggcggcgccctcttctccctttgcgtcgcagctgctggagccgccgtacgtgcctccgcgctacctgcggcctacgggggggagaaacagcatccgttactcggagctggcgcccctgttcgacaccacccgggtgtacctggtggacaacaagtcggcggacgtggcctccctgaactaccagaacgaccacagcaattttttgaccacggtcatccagaacaatgactacagcccgagcgaggccagcacccagaccatcaatctggatgaccggtcgcactggggcggcgacctgaaaaccatcctgcacaccaacatgcccaacgtgaacgagttcatgttcaccaataagttcaaggcgcgggtgatggtgtcgcgctcgcacaccaaggaagaccgggtggagctgaagtacgagtgggtggagttcgagctgccagagggcaactactccgagaccatgaccattgacctgatgaacaacgcgatcgtggagcactatctgaaagtgggcaggcagaacggggtcctggagagcgacatcggggtcaagttcgacaccaggaacttccgcctggggctggaccccgtgaccgggctggttatgcccggggtgtacaccaacgaggccttccatcccgacatcatcctgctgcccggctgcggggtggacttcacttacagccgcctgagcaacctcctgggcatccgcaagcggcagcccttccaggagggcttcaggatcacctacgaggacctggaggggggcaacatccccgcgctcctcgatgtggaggcctaccaggatagcttgaaggaaaatgaggcgggacaggaggataccgcccccgccgcctccgccgccgccgagcagggcgaggatgctgctgacaccgcggccgcggacggggcagaggccgaccccgctatggtggtggaggctcccgagcaggaggaggacatgaatgacagtgcggtgcgcggagacaccttcgtcacccggggggaggaaaagcaagcggaggccgaggccgcggccgaggaaaagcaactggcggcagcagcggcggcggcggcgttggccgcggcggaggctgagtctgaggggaccaagcccgccaaggagcccgtgattaagcccctgaccgaagatagcaagaagcgcagttacaacctgctcaaggacagcaccaacaccgcgtaccgcagctggtacctggcctacaactacggcgacccgtcgacgggggtgcgctcctggaccctgctgtgcacgccggacgtgacctgcggctcggagcaggtgtactggtcgctgcccgacatgatgcaagaccccgtgaccttccgctccacgcggcaggtcagcaacttcccggtggtgggcgccgagctgctgcccgtgcactccaagagcttctacaacgaccaggccgtctactcccagctcatccgccagttcacctctctgacccacgtgttcaatcgctttcctgagaaccagattctggcgcgcccgcccgcccccaccatcaccaccgtcagtgaaaacgttcctgctctcacagatcacgggacgctaccgctgcgcaacagcatcggaggagtccagcgagtgaccgttactgacgccagacgccgcacctgcccctacgtttacaaggccttgggcatagtctcgccgcgcgtcctttccagccgcactttttgagcaacaccaccatcatgtccatcctgatctcacccagcaataactccggctggggactgctgcgcgcgcccagcaagatgttcggaggggcgaggaagcgttccgagcagcaccccgtgcgcgtgcgcgggcacttccgcgccccctggggagcgcacaaacgcggccgcgcggggcgcaccaccgtggacgacgccatcgactcggtggtggagcaggcgcgcaactacaggcccgcggtctctaccgtggacgcggccatccagaccgtggtgcggggcgcgcggcggtacgccaagctgaagagccgccggaagcgcgtggcccgccgccaccgccgccgacccggggccgccgccaaacgcgccgccgcggccctgcttcgccgggccaagcgcacgggccgccgcgccgccatgagggccgcgcgccgcttggccgccggcatcaccgccgccaccatggccccccgtacccgaagacgcgcggccgccgccgccgccgccgccatcagtgacatggccagcaggcgccggggcaacgtgtactgggtgcgcgactcggtgaccggcacgcgcgtgcccgtgcgcttccgccccccgcggacttgagatgatgtgaaaaaacaacactgagtctcctgctgttgtgtgtatcccagcggcggcggcgcgcgcagcgtcatgtccaagcgcaaaatcaaagaagagatgctccaggtcgtcgcgccggagatctatgggcccccgaagaaggaagagcaggattcgaagccccgcaagataaagcgggtcaaaaagaaaaagaaagatgatgacgatgccgatggggaggtggagttcctgcgcgccacggcgcccaggcgcccggtgcagtggaagggccggcgcgtaaagcgcgtcctgcgccccggcaccgcggtggtcttcacgcccggcgagcgctccacccggactttcaagcgcgtctatgacgaggtgtacggcgacgaagacctgctggagcaggccaacgagcgcttcggagagtttgcttacgggaagcgtcagcgggcgctggggaaggaggacctgctggcgctgccgctggaccagggcaaccccacccccagtctgaagcccgtgaccctgcagcaggtgctgccgagcagcgcaccctccgaggcgaagcggggtctgaagcgcgagggcggcgacctggcgcccaccgtgcagctcatggtgcccaagcggcagaggctggaggatgtgctggagaaaatgaaagtagaccccggtctgcagccggacatcagggtccgccccatcaagcaggtggcgccgggcctcggcgtgcagaccgtggacgtggtcatccccaccggcaactcccccgccgccgccaccactaccgctgcctccacggacatggagacacagaccgatcccgccgcagccgcagccgcagccgccgccgcgacctcctcggcggaggtgcagacggacccctggctgccgccggcgatgtcagctccccgcgcgcgtcgcgggcgcaggaagtacggcgccgccaacgcgctcctgcccgagtacgccttgcatccttccatcgcgcccacccccggctaccgaggctatacctaccgcccgcgaagagccaagggttccacccgccgtccccgccgacgcgccgccgccaccacccgccgccgccgccgcagacgccagcccgcactggctccagtctccgtgaggaaagtggcgcgcgacggacacaccctggtgctgcccagggcgcgctaccaccccagcatcgtttaaaagcctgttgtggttcttgcagatatggccctcacttgccgcctccgtttcccggtgccgggataccgaggaggaagatcgcgccgcaggaggggtctggccggccgcggcctgagcggaggcagccgccgcgcgcaccggcggcgacgcgccaccagccgacgcatgcgcggcggggtgctgcccctgttaatccccctgatcgccgcggcgatcggcgccgtgcccgggatcgcctccgtggccttgcaagcgtcccagaggcattgacagacttgcaaacttgcaaatatggaaaaaaaaaccccaataaaaaagtctagactctcacgctcgcttggtcctgtgactattttgtagaatggaagacatcaactttgcgtcgctggccccgcgtcacggctcgcgcccgttcctgggacactggaacgatatcggcaccagcaacatgagcggtggcgccttcagttggggctctctgtggagcggcattaaaagtatcgggtctgccgttaaaaattacggctcccgggcctggaacagcagcacgggccagatgttgagagacaagttgaaagagcagaacttccagcagaaggtggtggagggcctggcctccggcatcaacggggtggtggacctggccaaccaggccgtgcagaataagatcaacagcagactggacccccggccgccggtggaggaggtgccgccggcgctggagacggtgtcccccgatgggcgtggcgagaagcgcccgcggcccgatagggaagagaccactctggtcacgcagaccgatgagccgcccccgtatgaggaggccctgaagcaaggtctgcccaccacgcggcccatcgcgcccatggccaccggggtggtgggccgccacacccccgccacgctggacttgcctccgcccgccgatgtgccgcagcagcagaaggcggcacagccgggcccgcccgcgaccgcctcccgttcctccgccggtcctctgcgccgcgcggccagcggcccccgcgggggggtcgcgaggcacggcaactggcagagcacgctgaacagcatcgtgggtctgggggtgcggtccgtgaagcgccgccgatgctactgaatagcttagctaacgtgttgtatgtgtgtatgcgccctatgtcgccgccagaggagctgctgagtcgccgccgttcgcgcgcccaccaccaccgccactccgcccctcaagatggcgaccccatcgatgatgccgcagtggtcgtacatgcacatctcgggccaggacgcctcggagtacctgagccccgggctggtgcagttcgcccgcgccaccgagagctacttcagcctgagtaacaagtttaggaaccccacggtggcgcccacgcacgatgtgaccaccgaccggtctcagcgcctgacgctgcggttcattcccgtggaccgcgaggacaccgcgtactcgtacaaggcgcggttcaccctggccgtgggcgacaaccgcgtgctggacatggcctccacctactttgacatccgcggggtgctggaccggggtcccactttcaagccctactctggcaccgcctacaactccctggcccccaagggcgctcccaactcctgcgagtgggagcaagaggaaactcaggcagttgaagaagcagcagaagaggaagaagaagatgctgacggtcaagctgaggaagagcaagcagctaccaaaaagactcatgtatatgctcaggctcccctttctggcgaaaaaattagtaaagatggtctgcaaataggaacggacgctacagctacagaacaaaaacctatttatgcagaccctacattccagcccgaaccccaaatcggggagtcccagtggaatgaggcagatgctacagtcgccggcggtagagtgctaaagaaatctactcccatgaaaccatgctatggttcctatgcaagacccacaaatgctaatggaggtcagggtgtactaacggcaaatgcccagggacagctagaatctcaggttgaaatgcaattcttttcaacttctgaaaacgcccgtaacgaggctaacaacattcagcccaaattggtgctgtatagtgaggatgtgcacatggagaccccggatacgcacctttcttacaagcccgcaaaaagcgatgacaattcaaaaatcatgctgggtcagcagtccatgcccaacagacctaattacatcggcttcagagacaactttatcggcctcatgtattacaatagcactggcaacatgggagtgcttgcaggtcaggcctctcagttgaatgcagtggtggacttgcaagacagaaacacagaactgtcctaccagctcttgcttgattccatgggtgacagaaccagatacttttccatgtggaatcaggcagtggacagttatgacccagatgttagaattattgaaaatcatggaactgaagacgagctccccaactattgtttccctctgggtggcataggggtaactgacacttaccaggctgttaaaaccaacaatggcaataacgggggccaggtgacttggacaaaagatgaaacttttgcagatcgcaatgaaataggggtgggaaacaatttcgctatggagatcaacctcagtgccaacctgtggagaaacttcctgtactccaacgtggcgctgtacctaccagacaagcttaagtacaacccctccaatgtggacatctctgacaaccccaacacctacgattacatgaacaagcgagtggtggccccggggctggtggactgctacatcaacctgggcgcgcgctggtcgctggactacatggacaacgtcaaccccttcaaccaccaccgcaatgcgggcctgcgctaccgctccatgctcctgggcaacgggcgctacgtgcccttccacatccaggtgccccagaagttctttgccatcaagaacctcctcctcctgccgggctcctacacctacgagtggaacttcaggaaggatgtcaacatggtcctccagagctctctgggtaacgatctcagggtggacggggccagcatcaagttcgagagcatctgcctctacgccaccttcttccccatggcccacaacacggcctccacgctcgaggccatgctcaggaacgacaccaacgaccagtccttcaatgactacctctccgccgccaacatgctctaccccatacccgccaacgccaccaacgtccccatctccatcccctcgcgcaactgggcggccttccgcggctgggccttcacccgcctcaagaccaaggagaccccctccctgggctcgggattcgacccctactacacctactcgggctccattccctacctggacggcaccttctacctcaaccacactttcaagaaggtctcggtcaccttcgactcctcggtcagctggccgggcaacgaccgtctgctcacccccaacgagttcgagatcaagcgctcggtcgacggggagggctacaacgtggcccagtgcaacatgaccaaggactggttcctggtccagatgctggccaactacaacatcggctaccagggcttctacatcccagagagctacaaggacaggatgtactccttcttcaggaacttccagcccatgagccggcaggtggtggaccagaccaagtacaaggactaccaggaggtgggcatcatccaccagcacaacaactcgggcttcgtgggctacctcgcccccaccatgcgcgagggacaggcctaccccgccaacttcccctatccgctcataggcaagaccgcggtcgacagcatcacccagaaaaagttcctctgcgaccgcaccctctggcgcatccccttctccagcaacttcatgtccatgggtgcgctctcggacctgggccagaacttgctctacgccaactccgcccacgccctcgacatgaccttcgaggtcgaccccatggacgagcccacccttctctatgttctgttcgaagtctttgacgtggtccgggtccaccagccgcaccgcggcgtcatcgagaccgtgtacctgcgtacgcccttctcggccggcaacgccaccacctaaagaagcaagccgcagtcatcgccgcctgcatgccgtcgggttccaccgagcaagagctcagggccatcgtcagagacctgggatgcgggccctattttttgggcaccttcgacaagcgcttccctggctttgtctccccacacaagctggcctgcgccatcgtcaacacggccggccgcgagaccgggggcgtgcactggctggccttcgcctggaacccgcgctccaaaacatgcttcctctttgaccccttcggcttttcggaccagcggctcaagcaaatctacgagttcgagtacgagggcttgctgcgtcgcagcgccatcgcctcctcgcccgaccgctgcgtcaccctcgaaaagtccacccagaccgtgcaggggcccgactcggccgcctgcggtctcttctgctgcatgtttctgcacgcctttgtgcactggcctcagagtcccatggaccgcaaccccaccatgaacttgctgacgggggtgcccaactccatgctccagagcccccaggtcgagcccaccctgcgccgcaaccaggagcagctctacagcttcctggagcgccactcgccttacttccgccgccacagcgcacagatcaggagggccacctccttctgccacttgcaagagatgcaagaagggtaataacgatgtacacactttttttctcaataaatggcatctttttatttatacaagctctctggggtattcatttcccaccaccacccgccgttgtcgccatctggctctatttagaaatcgaaagggttctgccgggagtcgccgtgcgccacgggcagggacacgttgcgatactggtagcgggtgccccacttgaactcgggcaccaccaggcgaggcagctcggggaagttttcgctccacaggctgcgggtcagcaccagcgcgttcatcaggtcgggcgccgagatcttgaagtcgcagttggggccgccgccctgcgcgcgcgagttgcggtacaccgggttgcagcactggaacaccaacagcgccgggtgcttcacgctggccagcacgctgcggtcggagatcagctcggcgtccaggtcctccgcgttgctcagcgcgaacggggtcatcttgggcacttgccgccccaggaagggcgcgtgccccggtttcgagttgcagtcgcagcgcagcgggatcagcaggtgcccgtgcccggactcggcgttggggtacagcgcgcgcatgaaggcctgcatctggcggaaggccatctgggccttggcgccctccgagaagaacatgccgcaggacttgcccgagaactggtttgcggggcagctggcgtcgtgcaggcagcagcgcgcgtcggtgttggcgatctgcaccacgttgcgcccccaccggttcttcacgatcttggccttggacgattgctccttcagcgcgcgctgcccgttctcgctggtcacatccatctcgatcacatgttccttgttcaccatgctgctgccgtgcagacacttcagctcgccctccgtctcggtgcagcggtgctgccacagcgcgcagcccgtgggctcgaaagacttgtaggtcacctccgcgaaggactgcaggtacccctgcaaaaagcggcccatcatggtcacgaaggtcttgttgctgctgaaggtcagctgcagcccgcggtgctcctcgttcagccaggtcttgcacacggccgccagcgcctccacctggtcgggcagcatcttgaagttcaccttcagctcattctccacgtggtacttgtccatcagcgtgcgcgccgcctccatgcccttctcccaggccgacaccagcggcaggctcacggggttcttcaccatcaccgtggccgccgcctccgccgcgctttcgctttccgccccgctgttctcttcctcttcctcctcttcctcgccgccgcccactcgcagcccccgcaccacggggtcgtcttcctgcaggcgctgcaccttgcgcttgccgttgcgcccctgcttgatgcgcacgggcgggttgctgaagcccaccatcaccagcgcggcctcttcttgctcgtcctcgctgtccagaatgacctccggggagggggggttggtcatcctcagtaccgaggcacgcttctttttcttcctgggggcgttcgccagctccgcggctgcggccgctgccgaggtcgaaggccgagggctgggcgtgcgcggcaccagcgcgtcctgcgagccgtcctcgtcctcctcggactcgagacggaggcgggcccgcttcttcgggggcgcgcggggcggcggaggcggcggcggcgacggagacggggacgagacatcgtccagggtgggtggacggcgggccgcgccgcgtccgcgctcgggggtggtctcgcgctggtcctcttcccgactggccatctcccactgctccttctcctataggcagaaagagatcatggagtctctcatgcgagtcgagaaggaggaggacagcctaaccgccccctctgagccctccaccaccgccgccaccaccgccaatgccgccgcggacgacgcgcccaccgagaccaccgccagtaccaccctccccagcgacgcacccccgctcgagaatgaagtgctgatcgagcaggacccgggttttgtgagcggagaggaggatgaggtggatgagaaggagaaggaggaggtcgccgcctcagtgccaaaagaggataaaaagcaagaccaggacgacgcagataaggatgagacagcagtcgggcgggggaacggaagccatgatgctgatgacggctacctagacgtgggagacgacgtgctgcttaagcacctgcaccgccagtgcgtcatcgtctgcgacgcgctgcaggagcgctgcgaagtgcccctggacgtggcggaggtcagccgcgcctacgagcggcacctcttcgcgccgcacgtgccccccaagcgccgggagaacggcacctgcgagcccaacccgcgtctcaacttctacccggtcttcgcggtacccgaggtgctggccacctaccacatctttttccaaaactgcaagatccccctctcctgccgcgccaaccgcacccgcgccgacaaaaccctgaccctgcggcagggcgcccacatacctgatatcgcctctctggaggaagtgcccaagatcttcgagggtctcggtcgcgacgagaaacgggcggcgaacgctctgcacggagacagcgaaaacgagagtcactcgggggtgctggtggagctcgagggcgacaacgcgcgcctggccgtactcaagcgcagcatagaggtcacccactttgcctacccggcgctcaacctgccccccaaggtcatgagtgtggtcatgggcgagctcatcatgcgccgcgcccagcccctggccgcggatgcaaacttgcaagagtcctccgaggaaggcctgcccgcggtcagcgacgagcagctggcgcgctggctggagacccgcgaccccgcgcagctggaggagcggcgcaagctcatgatggccgcggtgctggtcaccgtggagctcgagtgtctgcagcgcttcttcgcggaccccgagatgcagcgcaagctcgaggagaccctgcactacaccttccgccagggctacgtgcgccaggcctgcaagatctccaacgtggagctctgcaacctggtctcctacctgggcatcctgcacgagaaccgcctcgggcagaacgtcctgcactccaccctcaaaggggaggcgcgccgcgactacatccgcgactgcgcctacctcttcctctgctacacctggcagacggccatgggggtctggcagcagtgcctggaggagcgcaacctcaaggagctggaaaagctcctcaagcgcaccctcagggacctctggacgggcttcaacgagcgctcggtggccgccgcgctggcggacatcatctttcccgagcgcctgctcaagaccctgcagcagggcctgcccgacttcaccagccagagcatgctgcagaacttcaggactttcatcctggagcgctcgggcatcctgccggccacttgctgcgcgctgcccagcgacttcgtgcccatcaagtacagggagtgcccgccgccgctctggggccactgctacctcttccagctggccaactacctcgcctaccactcggacctcatggaagacgtgagcggcgagggcctgctcgagtgccactgccgctgcaacctctgcacgccccaccgctctctagtctgcaacccgcagctgctcagcgagagtcagattatcggtaccttcgagctgcagggtccctcgcctgacgagaagtccgcggctccagggctgaaactcactccggggctgtggacttccgcctacctacgcaaatttgtacctgaggactaccacgcccacgagatcaggttctacgaagaccaatcccgcccgcccaaggcggagctcaccgcctgcgtcatcacccaggggcacatcctgggccaattgcaagccatcaacaaagcccgccgagagttcttgctgaaaaagggtcggggggtgtacctggacccccagtccggcgaggagctaaacccgctacccccgccgccgccccagcagcgggaccttgcttcccaggatggcacccagaaagaagcagcagccgccgccgccgccgcagccatacatgcttctggaggaagaggaggaggactgggacagtcaggcagaggaggtttcggacgaggagcaggaggagatgatggaagactgggaggaggacagcagcctagacgaggaagcttcagaggccgaagaggtggcagacgcaacaccatcgccctcggtcgcagccccctcgccggggcccctgaaatcctccgaacccagcaccagcgctataacctccgctcctccggcgccggcgccacccgcccgcagacccaaccgtagatgggacaccacaggaaccggggtcggtaagtccaagtgcccgccgccgccaccgcagcagcagcagcagcagcgccagggctaccgctcgtggcgcgggcacaagaacgccatagtcgcctgcttgcaagactgcgggggcaacatctctttcgcccgccgcttcctgctattccaccacggggtcgcctttccccgcaatgtcctgcattactaccgtcatctctacagcccctactgcagcggcgacccagaggcggcagcggcagccacagcggcgaccaccacctaggaagatatcctccgcgggcaagacagcggcagcagcggccaggagacccgcggcagcagcggcgggagcggtgggcgcactgcgcctctcgcccaacgaacccctctcgacccgggagctcagacacaggatcttccccactttgtatgccatcttccaacagagcagaggccaggagcaggagctgaaaataaaaaacagatctctgcgctccctcacccgcagctgtctgtatcacaaaagcgaagatcagcttcggcgcacgctggaggacgcggaggcactcttcagcaaatactgcgcgctcactcttaaagactagctccgcgcccttctcgaatttaggcgggagaaaactacgtcatcgccggccgccgcccagcccgcccagccgagatgagcaaagagattcccacgccatacatgtggagctaccagccgcagatgggactcgcggcgggagcggcccaggactactccacccgcatgaactacatgagcgcgggaccccacatgatctcacaggtcaacgggatccgcgcccagcgaaaccaaatactgctggaacaggcggccatcaccgccacgccccgccataatctcaacccccgaaattggcccgccgccctcgtgtaccaggaaaccccctccgccaccaccgtactacttccgcgtgacgcccaggccgaagtccagatgactaactcaggggcgcagctcgcgggcggctttcgtcacggggcgcggccgctccgaccaggtataagacacctgatgatcagaggccgaggtatccagctcaacgacgagtcggtgagctcttcgctcggtctccgtccggacggaactttccagctcgccggatccggccgctcttcgttcacgccccgccaggcgtacctgactctgcagacctcgtcctcggagccccgctccggcggcatcggaaccctccagttcgtggaggagttcgtgccctcggtctacttcaaccccttctcgggacctcccggacgctaccccgaccagttcattccgaactttgacgcggtgaaggactcggcggacggctacgactgaatgtcaggtgtcgaggcagagcagcttcgcctgagacacctcgagcactgccgccgccacaagtgcttcgcccgcggttctggtgagttctgctactttcagctacccgaggagcataccgaggggccggcgcacggcgtccgcctgaccacccagggcgaggttacctgttccctcatccgggagtttaccctccgtcccctgctagtggagcgggagcggggtccctgtgtcctaactatcgcctgcaactgccctaaccctggattacatcaagatctttgctgtcatctctgtgctgagtttaataaacgctgagatcagaatctactgggatttagtcccctttaactaatcaaacactggaatcaataaaaagaatcacttacttaaaatcagacagcaggtctctgtccagtttattcagcagcacctccttcccctcctcccaactctggtactccaaacgccttctggcggcaaacttcctccacaccctgaagggaatgtcagattcttgctcctgtccctccgcacccactatcttcatgttgttgcagatgaagcgcaccaaaacgtctgacgagagcttcaaccccgtgtacccctatgacacggaaagcggccctccctccgtccctttcctcacccctcccttcgtgtctcccgatggattccaagaaagtccccccggggtcctgtctctgaacctggccgagcccctggtcacttcccacggcatgctcgccctgaaaatgggaagtggcctctccctggacgacgctggcaacctcacctctcaagatatcaccaccgctagccctcccctcaaaaaaaccaagaccaacctcagcctagaaacctcatcccccctaactgtgagcacctcaggcgccctcaccgtagcagccgccgctcccctggcggtggccggcacctccctcaccatgcaatcagaggcccccctgacagtacaggatgcaaaactcaccctggccaccaaaggccccctgaccgtgtctgaaggcaaactggccttgcaaacatcggccccgctgacggccgctgacagcagcaccctcacagtcagtgccacaccaccccttagcacaagcaatggcagcttgggtattgacatgcaagcccccatttacaccaccaatggaaaactaggacttaactttggcgctcccctgcatgtggtagacagcctaaatgcactgactgtagttactggccaaggtcttacgataaacggaacagccctacaaactagagtctcaggtgccctcaactatgacacatcaggaaacctagaattgagagctgcagggggtatgcgagttgatgcaaatggtcaacttatccttgatgtagcttacccatttgatgcacaaaacaatctcagccttaggcttggacagggacccctgtttgttaactctgcccacaacttggatgttaactacaacagaggcctctacctgttcacatctggaaataccaaaaagctagaagttaatatcaaaacagccaagggtctcatttatgatgacactgctatagcaatcaatgcgggtgatgggctacagtttgactcaggctcagatacaaatccattaaaaactaaacttggattaggactggattatgactccagcagagccataattgctaaactgggaactggcctaagctttgacaacacaggtgccatcacagtaggcaacaaaaatgatgacaagcttaccttgtggaccacaccagacccatcccctaactgtagaatctattcagagaaagatgctaaattcacacttgttttgactaaatgcggcagtcaggtgttggccagcgtttctgttttatctgtaaaaggtagccttgcgcccatcagtggcacagtaactagtgctcagattgtcctcagatttgatgaaaatggagttctactaagcaattcttcccttgaccctcaatactggaactacagaaaaggtgaccttacagagggcactgcatataccaacgcagtgggatttatgcccaacctcacagcatacccaaaaacacagagccaaactgctaaaagcaacattgtaagtcaggtttacttgaatggggacaaatccaaacccatgaccctcaccattaccctcaatggaactaatgaaacaggagatgccacagtaagcacttactccatgtcattctcatggaactggaatggaagtaattacattaatgaaacgttccaaaccaactccttcaccttctcctacatcgcccaagaataaaaagcatgacgctgttgatttgattcaatgtgtttctgttttattttcaagcacaacaaaatcattcaagtcattcttccatcttagcttaatagacacagtagcttaatagacccagtagtgcaaagccccattctagcttataactagtggagaagtactcgcctacatgggggtagagtcataatcgtgcatcaggatagggcggtggtgctgcagcagcgcgcgaataaactgctgccgccgccgctccgtcctgcaggaatacaacatggcagtggtctcctcagcgatgattcgcaccgcccgcagcataaggcgccttgtcctccgggcacagcagcgcaccctgatctcacttaaatcagcacagtaactgcagcacagcaccacaatattgttcaaaatcccacagtgcaaggcgctgtatccaaagctcatggcggggaccacagaacccacgtggccatcataccacaagcgcaggtagattaagtggcgacccctcataaacacgctggacataaacattacctcttttggcatgttgtaattcaccacctcccggtaccatataaacctctgattaaacatggcgccatccaccaccatcctaaaccagctggccaaaacctgcccgccggctatacactgcagggaaccgggactggaacaatgacagtggagagcccaggactcgtaaccatggatcatcatgctcgtcatgatatcaatgttggcacaacacaggcacacgtgcatacacttcctcaggattacaagctcctcccgcgttagaaccatatcccagggaacaacccattcctgaatcagcgtaaatcccacactgcagggaagacctcgcacgtaactcacgttgtgcattgtcaaagtgttacattcgggcagcagcggatgatcctccagtatggtagcgcgggtttctgtctcaaaaggaggtagacgatccctactgtacggagtgcgccgagacaaccgagatcgtgttggtcgtagtgtcatgccaaatggaacgccggacgtagtcatatttcctgaagtcttagatctctcaacgcagcaccagcaccaacacttcgcagtgtaaaaggccaagtgccgagagagtatatataggaataaaaagtgacgtaaacgggcaaagtccaaaaaacgcccagaaaaaccgcacgcgaacctacgccccgaaacgaaagccaaaaaacactagacactcccttccggcgtcaacttccgctttcccacgctacgtcacttgccccagtcaaacaaactacatatcccgaacttccaagtcgccacgcccaaaacaccgcctacacctccccgcccgccggcccgcccccaaacccgcctcccgccccgcgccccgccccgcgccgcccatctcattatcatattggcttcaatccaaaataaggtatattattgatgatggtttaaacggatcctctagagtcgacctgcaggcatgcaagcttgagtattctatagtgtcacctaaatagcttggcgtaatcatggtcatagctgtttcctgtgtgaaattgttatccgctcacaattccacacaacatacgagccggaagcataaagtgtaaagcctggggtgcctaatgagtgagctaactcacattaattgcgttgcgctcactgcccgctttccagtcgggaaacctgtcgtgccagctgcattaatgaatcggccaacgcgaaccccttgcggccgcccgggccgtcgaccaattctcatgtttgacagcttatcatcgaatttctgccattcatccgcttattatcacttattcagctcggtacccggggatcctcgtttaaacaggcgtagcaaccaggcgtttaagggcaccaataactgccttaaaaaaattacgccccgccctgccactcatcgcagtactgttgtaattcattaagcattctgccgacatggaagccatcacaaacggcatgatgaacctgaatcgccagcggcatcagcaccttgtcgccttgcgtataatatttgcccatggtgaaaacgggggcgaagaagttgtccatattggccacgtttaaatcaaaactggtgaaactcacccagggattggctgagacgaaaaacatattctcaataaaccctttagggaaataggccaggttttcaccgtaacacgccacatcttgcgaatatatgtgtagaaactgccggaaatcgtcgtggtattcactccagagcgatgaaaacgtttcagtttgctcatggaaaacggtgtaacaagggtgaacactatcccatatcaccagctcaccgtctttcattgccatacggaattccggatgagcattcatcaggcgggcaagaatgtgaataaaggccggataaaacttgtgcttatttttctttacggtctttaaaaaggccgtaatatccagctgaacggtctggttataggtacattgagcaactgactgaaatgcctcaaaatgttctttacgatgccattgggatatatcaacggtggtatatccagtgatttttttctccattttagcttccttagctcctgaaaatctcgataactcaaaaaatacgcccggtagtgatcttatttcattatggtgaaagttggaacctcttacgtgccgatcaacgtctcattttcgccaaaagttggcccagggcttcccggtatcaacagggacaccaggatttatttattctgcgaagtgatcttccgtcacaggtatttattcgcgataagctcatggagcggcgtaaccgtcgcacaggaaggacagagaaagcgcggatctgggaagtgacggacagaacggtcaggacctggattggggaggcggttgccgccgctgctgctgacggtgtgacgttctctgttccggtcacaccacatacgttccgccattcctatgcgatgcacatgctgtatgccggtataccgctgaaagttctgcaaagcctgatgggacataagtccatcagttcaacggaagtctacacgaaggtttttgcgctggatgtggctgcccggcaccgggtgcagtttgcgatgccggagtctgatgcggttgcgatgctgaaacaattatcctgagaataaatgccttggcctttatatggaaatgtggaactgagtggatatgctgtttttgtctgttaaacagagaagctggctgttatccactgagaagcgaacgaaacagtcgggaaaatctcccattatcgtagagatccgcattattaatctcaggagcctgtgtagcgtttataggaagtagtgttctgtcatgatgcctgcaagcggtaacgaaaacgatttgaatatgccttcaggaacaatagaaatcttcgtgcggtgttacgttgaagtggagcggattatgtcagcaatggacagaacaacctaatgaacacagaaccatgatgtggtctgtccttttacagccagtagtgctcgccgcagtcgagcgacagggcgaagccctcgagtgagcgaggaagcaccagggaacagcacttatatattctgcttacacacgatgcctgaaaaaacttcccttggggttatccacttatccacggggatatttttataattattttttttatagtttttagatcttcttttttagagcgccttgtaggcctttatccatgctggttctagagaaggtgttgtgacaaattgccctttcagtgtgacaaatcaccctcaaatgacagtcctgtctgtgacaaattgcccttaaccctgtgacaaattgccctcagaagaagctgttttttcacaaagttatccctgcttattgactcttttttatttagtgtgacaatctaaaaacttgtcacacttcacatggatctgtcatggcggaaacagcggttatcaatcacaagaaacgtaaaaatagcccgcgaatcgtccagtcaaacgacctcactgaggcggcatatagtctctcccgggatcaaaaacgtatgctgtatctgttcgttgaccagatcagaaaatctgatggcaccctacaggaacatgacggtatctgcgagatccatgttgctaaatatgctgaaatattcggattgacctctgcggaagccagtaaggatatacggcaggcattgaagagtttcgcggggaaggaagtggttttttatcgccctgaagaggatgccggcgatgaaaaaggctatgaatcttttccttggtttatcaaacgtgcgcacagtccatccagagggctttacagtgtacatatcaacccatatctcattcccttctttatcgggttacagaaccggtttacgcagtttcggcttagtgaaacaaaagaaatcaccaatccgtatgccatgcgtttatacgaatccctgtgtcagtatcgtaagccggatggctcaggcatcgtctctctgaaaatcgactggatcatagagcgttaccagctgcctcaaagttaccagcgtatgcctgacttccgccgccgcttcctgcaggtctgtgttaatgagatcaacagcagaactccaatgcgcctctcatacattgagaaaaagaaaggccgccagacgactcatatcgtattttccttccgcgatatcacttccatgacgacaggatagtctgagggttatctgtcacagatttgagggtggttcgtcacatttgttctgacctactgagggtaatttgtcacagttttgctgtttccttcagcctgcatggattttctcatactttttgaactgtaatttttaaggaagccaaatttgagggcagtttgtcacagttgatttccttctctttcccttcgtcatgtgacctgatatcgggggttagttcgtcatcattgatgagggttgattatcacagtttattactctgaattggctatccgcgtgtgtacctctacctggagtttttcccacggtggatatttcttcttgcgctgagcgtaagagctatctgacagaacagttcttctttgcttcctcgccagttcgctcgctatgctcggttacacggctgcggcgagcgctagtgataataagtgactgaggtatgtgctcttcttatctccttttgtagtgttgctcttattttaaacaactttgcggttttttgatgactttgcgattttgttgttgctttgcagtaaattgcaagatttaataaaaaaacgcaaagcaatgattaaaggatgttcagaatgaaactcatggaaacacttaaccagtgcataaacgctggtcatgaaatgacgaaggctatcgccattgcacagtttaatgatgacagcccggaagcgaggaaaataacccggcgctggagaataggtgaagcagcggatttagttggggtttcttctcaggctatcagagatgccgagaaagcagggcgactaccgcacccggatatggaaattcgaggacgggttgagcaacgtgttggttatacaattgaacaaattaatcatatgcgtgatgtgtttggtacgcgattgcgacgtgctgaagacgtatttccaccggtgatcggggttgctgcccataaaggtggcgtttacaaaacctcagtttctgttcatcttgctcaggatctggctctgaaggggctacgtgttttgctcgtggaaggtaacgacccccagggaacagcctcaatgtatcacggatgggtaccagatcttcatattcatgcagaagacactctcctgcctttctatcttggggaaaaggacgatgtcacttatgcaataaagcccacttgctggccggggcttgacattattccttcctgtctggctctgcaccgtattgaaactgagttaatgggcaaatttgatgaaggtaaactgcccaccgatccacacctgatgctccgactggccattgaaactgttgctcatgactatgatgtcatagttattgacagcgcgcctaacctgggtatcggcacgattaatgtcgtatgtgctgctgatgtgctgattgttcccacgcctgctgagttgtttgactacacctccgcactgcagtttttcgatatgcttcgtgatctgctcaagaacgttgatcttaaagggttcgagcctgatgtacgtattttgcttaccaaatacagcaatagtaatggctctcagtccccgtggatggaggagcaaattcgggatgcctggggaagcatggttctaaaaaatgttgtacgtgaaacggatgaagttggtaaaggtcagatccggatgagaactgtttttgaacaggccattgatcaacgctcttcaactggtgcctggagaaatgctctttctatttgggaacctgtctgcaatgaaattttcgatcgtctgattaaaccacgctgggagattagataatgaagcgtgcgcctgttattccaaaacatacgctcaatactcaaccggttgaagatacttcgttatcgacaccagctgccccgatggtggattcgttaattgcgcgcgtaggagtaatggctcgcggtaatgccattactttgcctgtatgtggtcgggatgtgaagtttactcttgaagtgctccggggtgatagtgttgagaagacctctcgggtatggtcaggtaatgaacgtgaccaggagctgcttactgaggacgcactggatgatctcatcccttcttttctactgactggtcaacagacaccggcgttcggtcgaagagtatctggtgtcatagaaattgccgatgggagtcgccgtcgtaaagctgctgcacttaccgaaagtgattatcgtgttctggttggcgagctggatgatgagcagatggctgcattatccagattgggtaacgattatcgcccaacaagtgcttatgaacgtggtcagcgttatgcaagccgattgcagaatgaatttgctggaaatatttctgcgctggctgatgcggaaaatatttcacgtaagattattacccgctgtatcaacaccgccaaattgcctaaatcagttgttgctcttttttctcaccccggtgaactatctgcccggtcaggtgatgcacttcaaaaagcctttacagataaagaggaattacttaagcagcaggcatctaaccttcatgagcagaaaaaagctggggtgatatttgaagctgaagaagttatcactcttttaacttctgtgcttaaaacgtcatctgcatcaagaactagtttaagctcacgacatcagtttgctcctggagcgacagtattgtataagggcgataaaatggtgcttaacctggacaggtctcgtgttccaactgagtgtatagagaaaattgaggccattcttaaggaacttgaaaagccagcaccctgatgcgaccacgttttagtctacgtttatctgtctttacttaatgtcctttgttacaggccagaaagcataactggcctgaatattctctctgggcccactgttccacttgtatcgtcggtctgataatcagactgggaccacggtcccactcgtatcgtcggtctgattattagtctgggaccacggtcccactcgtatcgtcggtctgattattagtctgggaccacggtcccactcgtatcgtcggtctgataatcagactgggaccacggtcccactcgtatcgtcggtctgattattagtctgggaccatggtcccactcgtatcgtcggtctgattattagtctgggaccacggtcccactcgtatcgtcggtctgattattagtctggaaccacggtcccactcgtatcgtcggtctgattattagtctgggaccacggtcccactcgtatcgtcggtctgattattagtctgggaccacgatcccactcgtgttgtcggtctgattatcggtctgggaccacggtcccacttgtattgtcgatcagactatcagcgtgagactacgattccatcaatgcctgtcaagggcaagtattgacatgtcgtcgtaacctgtagaacggagtaacctcggtgtgcggttgtatgcctgctgtggattgctgctgtgtcctgcttatccacaacattttgcgcacggttatgtggacaaaatacctggttacccaggccgtgccggcacgttaaccgggctgcatccgatgcaagtgtgtcgctgtcgacgagctcgcgagctcggacatgaggttgccccgtattcagtgtcgctgatttgtattgtctgaagttgtttttacgttaagttgatgcagatcaattaatacgatacctgcgtcataattgattatttgacgtggtttgatggcctccacgcacgttgtgatatgtagatgataatcattatcactttacgggtcctttccggtgatccgacaggttacggggcggcgacctcgcgggttttcgctatttatgaaaattttccggtttaaggcgtttccgttcttcttcgtcataacttaatgtttttatttaaaataccctctgaaaagaaaggaaacgacaggtgctgaaagcgagctttttggcctctgtcgtttcctttctctgtttttgtccgtggaatgaacaatggaagtccgagctcatcgctaataacttcgtatagcatacattatacgaagttatattcgatgcggccgcaaggggttcgcgtcagcgggtgttggcgggtgtcggggctggcttaactatgcggcatcagagcagattgtactgagagtgcaccatatgcggtgtgaaataccgcacagatgcgtaaggagaaaataccgcatcaggcgccattcgccattcaggctgcgcaactgttgggaagggcgatcggtgcgggcctcttcgctattacgccagctggcgaaagggggatgtgctgcaaggcgattaagttgggtaacgccagggttttcccagtcacgacgttgtaaaacgacggccagtgaattgtaatacgactcactatagggcgaattcgagctcggtacccggggatcctcgtttaaac